European Patent Specification EP 3 535 289 B1, published July 17, 2024. Title: An Engineered Multi-component System for Identification and Characterisation of T-cell receptors, T-cell antigens and their functional interaction. Applicant: Genovie AB. The sequence listing filed with the application follows.

SEQUENCE LISTING (134 sequences)

SEQ ID NO: 1 - protein, 4 aa, Homo sapiens
  HCMV Antigen
NLVP

SEQ ID NO: 2 - protein, 9 aa, Cytomegalovirus
  Analyte Antigenic Peptide
NLVPMVATV

SEQ ID NO: 3 - protein, 9 aa, Artificial Sequence
  Analyte Antigenic Peptide
VYALPLKML

SEQ ID NO: 4 - DNA, 6071 bp, Artificial Sequence
  pcDNA3.1_GFP vector V1.A.4
gacggatcgggagatctcccgatcccctatggtgcactctcagtacaatctgctctgatgccgcatagttaagccagtatctgctccctgcttgtgtgttggaggtcgctgagtagtgcgcgagcaaaatttaagctacaacaaggcaaggcttgaccgacaattgcatgaagaatctgcttagggttaggcgttttgcgctgcttcgcgatgtacgggccagatatacgcgttgacattgattattgactagttattaatagtaatcaattacggggtcattagttcatagcccatatatggagttccgcgttacataacttacggtaaatggcccgcctggctgaccgcccaacgacccccgcccattgacgtcaataatgacgtatgttcccatagtaacgccaatagggactttccattgacgtcaatgggtggagtatttacggtaaactgcccacttggcagtacatcaagtgtatcatatgccaagtacgccccctattgacgtcaatgacggtaaatggcccgcctggcattatgcccagtacatgaccttatgggactttcctacttggcagtacatctacgtattagtcatcgctattaccatggtgatgcggttttggcagtacatcaatgggcgtggatagcggtttgactcacggggatttccaagtctccaccccattgacgtcaatgggagtttgttttggcaccaaaatcaacgggactttccaaaatgtcgtaacaactccgccccattgacgcaaatgggcggtaggcgtgtacggtgggaggtctatataagcagagctctctggctaactagagaacccactgcttactggcttatcgaaattaatacgactcactatagggagacccaagctggctagcgtttaaacttaagcttggtaccgccaccatggaatccgatgagtctggcctgcccgccatggaaatcgagtgcagaatcaccggcaccctgaacggcgtggaatttgagctcgtgggcggaggcgagggcacacctgaacagggcagaatgaccaacaagatgaagtccaccaagggggccctgaccttcagcccctacctgctgtctcacgtgatgggctacggcttctaccacttcggcacctaccccagcggctacgagaaccctttcctgcacgccatcaacaacggcggctacaccaacacccggatcgagaagtacgaggacggcggcgtgctgcacgtgtccttcagctacagatacgaggccggcagagtgatcggcgacttcaaagtgatgggcaccggattccccgaggacagcgtgatcttcaccgacaagatcatccggtccaacgccaccgtggaacatctgcaccccatgggcgacaacgacctggacggcagcttcaccagaaccttctccctgcgggatggcggctactacagcagcgtggtggacagccacatgcacttcaagagcgccatccaccccagcatcctccagaacggcggacccatgttcgccttcagacgggtggaagaggaccacagcaacaccgagctgggcatcgtggaataccagcacgccttcaagacccccgatgccgatgccggcgaggaatgagtcgagtctagagggcccgtttaaacccgctgatcagcctcgactgtgccttctagttgccagccatctgttgtttgcccctcccccgtgccttccttgaccctggaaggtgccactcccactgtcctttcctaataaaatgaggaaattgcatcgcattgtctgagtaggtgtcattctattctggggggtggggtggggcaggacagcaagggggaggattgggaagacaatagcaggcatgctggggatgcggtgggctctatggcttctgaggcggaaagaaccagctggggctctagggggtatccccacgcgccctgtagcggcgcattaagcgcggcgggtgtggtggttacgcgcagcgtgaccgctacacttgccagcgccctagcgcccgctcctttcgctttcttcccttcctttctcgccacgttcgccggctttccccgtcaagctctaaatcgggggctccctttagggttccgatttagtgctttacggcacctcgaccccaaaaaacttgattagggtgatggttcacgtagtgggccatcgccctgatagacggtttttcgccctttgacgttggagtccacgttctttaatagtggactcttgttccaaactggaacaacactcaaccctatctcggtctattcttttgatttataagggattttgccgatttcggcctattggttaaaaaatgagctgatttaacaaaaatttaacgcgaattaattctgtggaatgtgtgtcagttagggtgtggaaagtccccaggctccccagcaggcagaagtatgcaaagcatgcatctcaattagtcagcaaccaggtgtggaaagtccccaggctccccagcaggcagaagtatgcaaagcatgcatctcaattagtcagcaaccatagtcccgcccctaactccgcccatcccgcccctaactccgcccagttccgcccattctccgccccatggctgactaattttttttatttatgcagaggccgaggccgcctctgcctctgagctattccagaagtagtgaggaggcttttttggaggcctaggcttttgcaaaaagctcccgggagcttgtatatccattttcggatctgatcaagagacaggatgaggatcgtttcgcatgattgaacaagatggattgcacgcaggttctccggccgcttgggtggagaggctattcggctatgactgggcacaacagacaatcggctgctctgatgccgccgtgttccggctgtcagcgcaggggcgcccggttctttttgtcaagaccgacctgtccggtgccctgaatgaactgcaggacgaggcagcgcggctatcgtggctggccacgacgggcgttccttgcgcagctgtgctcgacgttgtcactgaagcgggaagggactggctgctattgggcgaagtgccggggcaggatctcctgtcatctcaccttgctcctgccgagaaagtatccatcatggctgatgcaatgcggcggctgcatacgcttgatccggctacctgcccattcgaccaccaagcgaaacatcgcatcgagcgagcacgtactcggatggaagccggtcttgtcgatcaggatgatctggacgaagagcatcaggggctcgcgccagccgaactgttcgccaggctcaaggcgcgcatgcccgacggcgaggatctcgtcgtgacccatggcgatgcctgcttgccgaatatcatggtggaaaatggccgcttttctggattcatcgactgtggccggctgggtgtggcggaccgctatcaggacatagcgttggctacccgtgatattgctgaagagcttggcggcgaatgggctgaccgcttcctcgtgctttacggtatcgccgctcccgattcgcagcgcatcgccttctatcgccttcttgacgagttcttctgagcgggactctggggttcgaaatgaccgaccaagcgacgcccaacctgccatcacgagatttcgattccaccgccgccttctatgaaaggttgggcttcggaatcgttttccgggacgccggctggatgatcctccagcgcggggatctcatgctggagttcttcgcccaccccaacttgtttattgcagcttataatggttacaaataaagcaatagcatcacaaatttcacaaataaagcatttttttcactgcattctagttgtggtttgtccaaactcatcaatgtatcttatcatgtctgtataccgtcgacctctagctagagcttggcgtaatcatggtcatagctgtttcctgtgtgaaattgttatccgctcacaattccacacaacatacgagccggaagcataaagtgtaaagcctggggtgcctaatgagtgagctaactcacattaattgcgttgcgctcactgcccgctttccagtcgggaaacctgtcgtgccagctgcattaatgaatcggccaacgcgcggggagaggcggtttgcgtattgggcgctcttccgcttcctcgctcactgactcgctgcgctcggtcgttcggctgcggcgagcggtatcagctcactcaaaggcggtaatacggttatccacagaatcaggggataacgcaggaaagaacatgtgagcaaaaggccagcaaaaggccaggaaccgtaaaaaggccgcgttgctggcgtttttccataggctccgcccccctgacgagcatcacaaaaatcgacgctcaagtcagaggtggcgaaacccgacaggactataaagataccaggcgtttccccctggaagctccctcgtgcgctctcctgttccgaccctgccgcttaccggatacctgtccgcctttctcccttcgggaagcgtggcgctttctcatagctcacgctgtaggtatctcagttcggtgtaggtcgttcgctccaagctgggctgtgtgcacgaaccccccgttcagcccgaccgctgcgccttatccggtaactatcgtcttgagtccaacccggtaagacacgacttatcgccactggcagcagccactggtaacaggattagcagagcgaggtatgtaggcggtgctacagagttcttgaagtggtggcctaactacggctacactagaagaacagtatttggtatctgcgctctgctgaagccagttaccttcggaaaaagagttggtagctcttgatccggcaaacaaaccaccgctggtagcggtttttttgtttgcaagcagcagattacgcgcagaaaaaaaggatctcaagaagatcctttgatcttttctacggggtctgacgctcagtggaacgaaaactcacgttaagggattttggtcatgagattatcaaaaaggatcttcacctagatccttttaaattaaaaatgaagttttaaatcaatctaaagtatatatgagtaaacttggtctgacagttaccaatgcttaatcagtgaggcacctatctcagcgatctgtctatttcgttcatccatagttgcctgactccccgtcgtgtagataactacgatacgggagggcttaccatctggccccagtgctgcaatgataccgcgagacccacgctcaccggctccagatttatcagcaataaaccagccagccggaagggccgagcgcagaagtggtcctgcaactttatccgcctccatccagtctattaattgttgccgggaagctagagtaagtagttcgccagttaatagtttgcgcaacgttgttgccattgctacaggcatcgtggtgtcacgctcgtcgtttggtatggcttcattcagctccggttcccaacgatcaaggcgagttacatgatcccccatgttgtgcaaaaaagcggttagctccttcggtcctccgatcgttgtcagaagtaagttggccgcagtgttatcactcatggttatggcagcactgcataattctcttactgtcatgccatccgtaagatgcttttctgtgactggtgagtactcaaccaagtcattctgagaatagtgtatgcggcgaccgagttgctcttgcccggcgtcaatacgggataataccgcgccacatagcagaactttaaaagtgctcatcattggaaaacgttcttcggggcgaaaactctcaaggatcttaccgctgttgagatccagttcgatgtaacccactcgtgcacccaactgatcttcagcatcttttactttcaccagcgtttctgggtgagcaaaaacaggaaggcaaaatgccgcaaaaaagggaataagggcgacacggaaatgttgaatactcatactcttcctttttcaatattattgaagcatttatcagggttattgtctcatgagcggatacatatttgaatgtatttagaaaaataaacaaataggggttccgcgcacatttccccgaaaagtgccacctgacgtc

SEQ ID NO: 5 - DNA, 6068 bp, Artificial Sequence
  pcDNA3.1_RFP vector V1.A.6
gacggatcgggagatctcccgatcccctatggtgcactctcagtacaatctgctctgatgccgcatagttaagccagtatctgctccctgcttgtgtgttggaggtcgctgagtagtgcgcgagcaaaatttaagctacaacaaggcaaggcttgaccgacaattgcatgaagaatctgcttagggttaggcgttttgcgctgcttcgcgatgtacgggccagatatacgcgttgacattgattattgactagttattaatagtaatcaattacggggtcattagttcatagcccatatatggagttccgcgttacataacttacggtaaatggcccgcctggctgaccgcccaacgacccccgcccattgacgtcaataatgacgtatgttcccatagtaacgccaatagggactttccattgacgtcaatgggtggagtatttacggtaaactgcccacttggcagtacatcaagtgtatcatatgccaagtacgccccctattgacgtcaatgacggtaaatggcccgcctggcattatgcccagtacatgaccttatgggactttcctacttggcagtacatctacgtattagtcatcgctattaccatggtgatgcggttttggcagtacatcaatgggcgtggatagcggtttgactcacggggatttccaagtctccaccccattgacgtcaatgggagtttgttttggcaccaaaatcaacgggactttccaaaatgtcgtaacaactccgccccattgacgcaaatgggcggtaggcgtgtacggtgggaggtctatataagcagagctctctggctaactagagaacccactgcttactggcttatcgaaattaatacgactcactatagggagacccaagctggctagcgtttaaacttaagcttggtaccgccaccatgagcgagctgatcaaagaaaacatgcacatgaagctgtacatggaaggcaccgtgaacaaccaccacttcaagtgcaccagcgagggcgagggcaagccttacgagggcacccagaccatgaagatcaaggtggtggaaggcggccctctgcccttcgcctttgatatcctggccaccagctttatgtacggcagcaaggccttcatcaaccacacccagggcatccccgatttcttcaagcagagcttccccgagggcttcacctgggagcggatcaccacatacgaggacggcggagtgctgaccgccacccaggataccagcttccagaacggctgcatcatctacaacgtgaagattaacggcgtgaacttccccagcaacggccccgtgatgcagaagaaaaccagaggctgggaggccaacaccgagatgctgtaccctgccgatggcggcctgagaggccattctcagatggccctgaaactcgtgggcggaggctacctgcactgctccttcaagaccacctacagaagcaagaagcccgccaagaacctgaagatgcccggcttccacttcgtggaccaccggctggaacggatcaaagaggccgacaaagaaacctacgtggaacagcacgagatggccgtggccaagtactgcgacctgcctagcaagctgggccacagatgagtcgagtctagagggcccgtttaaacccgctgatcagcctcgactgtgccttctagttgccagccatctgttgtttgcccctcccccgtgccttccttgaccctggaaggtgccactcccactgtcctttcctaataaaatgaggaaattgcatcgcattgtctgagtaggtgtcattctattctggggggtggggtggggcaggacagcaagggggaggattgggaagacaatagcaggcatgctggggatgcggtgggctctatggcttctgaggcggaaagaaccagctggggctctagggggtatccccacgcgccctgtagcggcgcattaagcgcggcgggtgtggtggttacgcgcagcgtgaccgctacacttgccagcgccctagcgcccgctcctttcgctttcttcccttcctttctcgccacgttcgccggctttccccgtcaagctctaaatcgggggctccctttagggttccgatttagtgctttacggcacctcgaccccaaaaaacttgattagggtgatggttcacgtagtgggccatcgccctgatagacggtttttcgccctttgacgttggagtccacgttctttaatagtggactcttgttccaaactggaacaacactcaaccctatctcggtctattcttttgatttataagggattttgccgatttcggcctattggttaaaaaatgagctgatttaacaaaaatttaacgcgaattaattctgtggaatgtgtgtcagttagggtgtggaaagtccccaggctccccagcaggcagaagtatgcaaagcatgcatctcaattagtcagcaaccaggtgtggaaagtccccaggctccccagcaggcagaagtatgcaaagcatgcatctcaattagtcagcaaccatagtcccgcccctaactccgcccatcccgcccctaactccgcccagttccgcccattctccgccccatggctgactaattttttttatttatgcagaggccgaggccgcctctgcctctgagctattccagaagtagtgaggaggcttttttggaggcctaggcttttgcaaaaagctcccgggagcttgtatatccattttcggatctgatcaagagacaggatgaggatcgtttcgcatgattgaacaagatggattgcacgcaggttctccggccgcttgggtggagaggctattcggctatgactgggcacaacagacaatcggctgctctgatgccgccgtgttccggctgtcagcgcaggggcgcccggttctttttgtcaagaccgacctgtccggtgccctgaatgaactgcaggacgaggcagcgcggctatcgtggctggccacgacgggcgttccttgcgcagctgtgctcgacgttgtcactgaagcgggaagggactggctgctattgggcgaagtgccggggcaggatctcctgtcatctcaccttgctcctgccgagaaagtatccatcatggctgatgcaatgcggcggctgcatacgcttgatccggctacctgcccattcgaccaccaagcgaaacatcgcatcgagcgagcacgtactcggatggaagccggtcttgtcgatcaggatgatctggacgaagagcatcaggggctcgcgccagccgaactgttcgccaggctcaaggcgcgcatgcccgacggcgaggatctcgtcgtgacccatggcgatgcctgcttgccgaatatcatggtggaaaatggccgcttttctggattcatcgactgtggccggctgggtgtggcggaccgctatcaggacatagcgttggctacccgtgatattgctgaagagcttggcggcgaatgggctgaccgcttcctcgtgctttacggtatcgccgctcccgattcgcagcgcatcgccttctatcgccttcttgacgagttcttctgagcgggactctggggttcgaaatgaccgaccaagcgacgcccaacctgccatcacgagatttcgattccaccgccgccttctatgaaaggttgggcttcggaatcgttttccgggacgccggctggatgatcctccagcgcggggatctcatgctggagttcttcgcccaccccaacttgtttattgcagcttataatggttacaaataaagcaatagcatcacaaatttcacaaataaagcatttttttcactgcattctagttgtggtttgtccaaactcatcaatgtatcttatcatgtctgtataccgtcgacctctagctagagcttggcgtaatcatggtcatagctgtttcctgtgtgaaattgttatccgctcacaattccacacaacatacgagccggaagcataaagtgtaaagcctggggtgcctaatgagtgagctaactcacattaattgcgttgcgctcactgcccgctttccagtcgggaaacctgtcgtgccagctgcattaatgaatcggccaacgcgcggggagaggcggtttgcgtattgggcgctcttccgcttcctcgctcactgactcgctgcgctcggtcgttcggctgcggcgagcggtatcagctcactcaaaggcggtaatacggttatccacagaatcaggggataacgcaggaaagaacatgtgagcaaaaggccagcaaaaggccaggaaccgtaaaaaggccgcgttgctggcgtttttccataggctccgcccccctgacgagcatcacaaaaatcgacgctcaagtcagaggtggcgaaacccgacaggactataaagataccaggcgtttccccctggaagctccctcgtgcgctctcctgttccgaccctgccgcttaccggatacctgtccgcctttctcccttcgggaagcgtggcgctttctcatagctcacgctgtaggtatctcagttcggtgtaggtcgttcgctccaagctgggctgtgtgcacgaaccccccgttcagcccgaccgctgcgccttatccggtaactatcgtcttgagtccaacccggtaagacacgacttatcgccactggcagcagccactggtaacaggattagcagagcgaggtatgtaggcggtgctacagagttcttgaagtggtggcctaactacggctacactagaagaacagtatttggtatctgcgctctgctgaagccagttaccttcggaaaaagagttggtagctcttgatccggcaaacaaaccaccgctggtagcggtttttttgtttgcaagcagcagattacgcgcagaaaaaaaggatctcaagaagatcctttgatcttttctacggggtctgacgctcagtggaacgaaaactcacgttaagggattttggtcatgagattatcaaaaaggatcttcacctagatccttttaaattaaaaatgaagttttaaatcaatctaaagtatatatgagtaaacttggtctgacagttaccaatgcttaatcagtgaggcacctatctcagcgatctgtctatttcgttcatccatagttgcctgactccccgtcgtgtagataactacgatacgggagggcttaccatctggccccagtgctgcaatgataccgcgagacccacgctcaccggctccagatttatcagcaataaaccagccagccggaagggccgagcgcagaagtggtcctgcaactttatccgcctccatccagtctattaattgttgccgggaagctagagtaagtagttcgccagttaatagtttgcgcaacgttgttgccattgctacaggcatcgtggtgtcacgctcgtcgtttggtatggcttcattcagctccggttcccaacgatcaaggcgagttacatgatcccccatgttgtgcaaaaaagcggttagctccttcggtcctccgatcgttgtcagaagtaagttggccgcagtgttatcactcatggttatggcagcactgcataattctcttactgtcatgccatccgtaagatgcttttctgtgactggtgagtactcaaccaagtcattctgagaatagtgtatgcggcgaccgagttgctcttgcccggcgtcaatacgggataataccgcgccacatagcagaactttaaaagtgctcatcattggaaaacgttcttcggggcgaaaactctcaaggatcttaccgctgttgagatccagttcgatgtaacccactcgtgcacccaactgatcttcagcatcttttactttcaccagcgtttctgggtgagcaaaaacaggaaggcaaaatgccgcaaaaaagggaataagggcgacacggaaatgttgaatactcatactcttcctttttcaatattattgaagcatttatcagggttattgtctcatgagcggatacatatttgaatgtatttagaaaaataaacaaataggggttccgcgcacatttccccgaaaagtgccacctgacgtc

SEQ ID NO: 6 - DNA, 10428 bp, Artificial Sequence
  SpCas9-2A-GFP vector V1.A.8
gacggatcgggagatctcccgatcccctatggtgcactctcagtacaatctgctctgatgccgcatagttaagccagtatctgctccctgcttgtgtgttggaggtcgctgagtagtgcgcgagcaaaatttaagctacaacaaggcaaggcttgaccgacaattgcatgaagaatctgcttagggttaggcgttttgcgctgcttcgcgatgtacgggccagatatacgcgttgacattgattattgactagttattaatagtaatcaattacggggtcattagttcatagcccatatatggagttccgcgttacataacttacggtaaatggcccgcctggctgaccgcccaacgacccccgcccattgacgtcaataatgacgtatgttcccatagtaacgccaatagggactttccattgacgtcaatgggtggagtatttacggtaaactgcccacttggcagtacatcaagtgtatcatatgccaagtacgccccctattgacgtcaatgacggtaaatggcccgcctggcattatgcccagtacatgaccttatgggactttcctacttggcagtacatctacgtattagtcatcgctattaccatggtgatgcggttttggcagtacatcaatgggcgtggatagcggtttgactcacggggatttccaagtctccaccccattgacgtcaatgggagtttgttttggcaccaaaatcaacgggactttccaaaatgtcgtaacaactccgccccattgacgcaaatgggcggtaggcgtgtacggtgggaggtctatataagcagagctctctggctaactagagaacccactgcttactggcttatcgaaattaatacgactcactatagggagacccaagctggctagcgtttaaacttaagcttggtaccgccaccatggactataaggaccacgacggagactacaaggatcatgatattgattacaaagacgatgacgataagatggccccaaagaagaagcggaaggtcggtatccacggagtcccagcagccgacaagaagtacagcatcggcctggacatcggcaccaactctgtgggctgggccgtgatcaccgacgagtacaaggtgcccagcaagaaattcaaggtgctgggcaacaccgaccggcacagcatcaagaagaacctgatcggagccctgctgttcgacagcggcgaaacagccgaggccacccggctgaagagaaccgccagaagaagatacaccagacggaagaaccggatctgctatctgcaagagatcttcagcaacgagatggccaaggtggacgacagcttcttccacagactggaagagtccttcctggtggaagaggataagaagcacgagcggcaccccatcttcggcaacatcgtggacgaggtggcctaccacgagaagtaccccaccatctaccacctgagaaagaaactggtggacagcaccgacaaggccgacctgcggctgatctatctggccctggcccacatgatcaagttccggggccacttcctgatcgagggcgacctgaaccccgacaacagcgacgtggacaagctgttcatccagctggtgcagacctacaaccagctgttcgaggaaaaccccatcaacgccagcggcgtggacgccaaggccatcctgtctgccagactgagcaagagcagacggctggaaaatctgatcgcccagctgcccggcgagaagaagaatggcctgttcggaaacctgattgccctgagcctgggcctgacccccaacttcaagagcaacttcgacctggccgaggatgccaaactgcagctgagcaaggacacctacgacgacgacctggacaacctgctggcccagatcggcgaccagtacgccgacctgtttctggccgccaagaacctgtccgacgccatcctgctgagcgacatcctgagagtgaacaccgagatcaccaaggcccccctgagcgcctctatgatcaagagatacgacgagcaccaccaggacctgaccctgctgaaagctctcgtgcggcagcagctgcctgagaagtacaaagagattttcttcgaccagagcaagaacggctacgccggctacattgacggcggagccagccaggaagagttctacaagttcatcaagcccatcctggaaaagatggacggcaccgaggaactgctcgtgaagctgaacagagaggacctgctgcggaagcagcggaccttcgacaacggcagcatcccccaccagatccacctgggagagctgcacgccattctgcggcggcaggaagatttttacccattcctgaaggacaaccgggaaaagatcgagaagatcctgaccttccgcatcccctactacgtgggccctctggccaggggaaacagcagattcgcctggatgaccagaaagagcgaggaaaccatcaccccctggaacttcgaggaagtggtggacaagggcgcttccgcccagagcttcatcgagcggatgaccaacttcgataagaacctgcccaacgagaaggtgctgcccaagcacagcctgctgtacgagtacttcaccgtgtataacgagctgaccaaagtgaaatacgtgaccgagggaatgagaaagcccgccttcctgagcggcgagcagaaaaaggccatcgtggacctgctgttcaagaccaaccggaaagtgaccgtgaagcagctgaaagaggactacttcaagaaaatcgagtgcttcgactccgtggaaatctccggcgtggaagatcggttcaacgcctccctgggcacataccacgatctgctgaaaattatcaaggacaaggacttcctggacaatgaggaaaacgaggacattctggaagatatcgtgctgaccctgacactgtttgaggacagagagatgatcgaggaacggctgaaaacctatgcccacctgttcgacgacaaagtgatgaagcagctgaagcggcggagatacaccggctggggcaggctgagccggaagctgatcaacggcatccgggacaagcagtccggcaagacaatcctggatttcctgaagtccgacggcttcgccaacagaaacttcatgcagctgatccacgacgacagcctgacctttaaagaggacatccagaaagcccaggtgtccggccagggcgatagcctgcacgagcacattgccaatctggccggcagccccgccattaagaagggcatcctgcagacagtgaaggtggtggacgagctcgtgaaagtgatgggccggcacaagcccgagaacatcgtgatcgaaatggccagagagaaccagaccacccagaagggacagaagaacagccgcgagagaatgaagcggatcgaagagggcatcaaagagctgggcagccagatcctgaaagaacaccccgtggaaaacacccagctgcagaacgagaagctgtacctgtactacctgcagaatgggcgggatatgtacgtggaccaggaactggacatcaaccggctgtccgactacgatgtggaccatatcgtgcctcagagctttctgaaggacgactccatcgacaacaaggtgctgaccagaagcgacaagaaccggggcaagagcgacaacgtgccctccgaagaggtcgtgaagaagatgaagaactactggcggcagctgctgaacgccaagctgattacccagagaaagttcgacaatctgaccaaggccgagagaggcggcctgagcgaactggataaggccggcttcatcaagagacagctggtggaaacccggcagatcacaaagcacgtggcacagatcctggactcccggatgaacactaagtacgacgagaatgacaagctgatccgggaagtgaaagtgatcaccctgaagtccaagctggtgtccgatttccggaaggatttccagttttacaaagtgcgcgagatcaacaactaccaccacgcccacgacgcctacctgaacgccgtcgtgggaaccgccctgatcaaaaagtaccctaagctggaaagcgagttcgtgtacggcgactacaaggtgtacgacgtgcggaagatgatcgccaagagcgagcaggaaatcggcaaggctaccgccaagtacttcttctacagcaacatcatgaactttttcaagaccgagattaccctggccaacggcgagatccggaagcggcctctgatcgagacaaacggcgaaaccggggagatcgtgtgggataagggccgggattttgccaccgtgcggaaagtgctgagcatgccccaagtgaatatcgtgaaaaagaccgaggtgcagacaggcggcttcagcaaagagtctatcctgcccaagaggaacagcgataagctgatcgccagaaagaaggactgggaccctaagaagtacggcggcttcgacagccccaccgtggcctattctgtgctggtggtggccaaagtggaaaagggcaagtccaagaaactgaagagtgtgaaagagctgctggggatcaccatcatggaaagaagcagcttcgagaagaatcccatcgactttctggaagccaagggctacaaagaagtgaaaaaggacctgatcatcaagctgcctaagtactccctgttcgagctggaaaacggccggaagagaatgctggcctctgccggcgaactgcagaagggaaacgaactggccctgccctccaaatatgtgaacttcctgtacctggccagccactatgagaagctgaagggctcccccgaggataatgagcagaaacagctgtttgtggaacagcacaagcactacctggacgagatcatcgagcagatcagcgagttctccaagagagtgatcctggccgacgctaatctggacaaagtgctgtccgcctacaacaagcaccgggataagcccatcagagagcaggccgagaatatcatccacctgtttaccctgaccaatctgggagcccctgccgccttcaagtactttgacaccaccatcgaccggaagaggtacaccagcaccaaagaggtgctggacgccaccctgatccaccagagcatcaccggcctgtacgagacacggatcgacctgtctcagctgggaggcgacaaaaggccggcggccacgaaaaaggccggccaggcaaaaaagaaaaaggaattcggcagtggagagggcagaggaagtctgctaacatgcggtgacgtcgaggagaatcctggcccagtgagcaagggcgaggagctgttcaccggggtggtgcccatcctggtcgagctggacggcgacgtaaacggccacaagttcagcgtgtccggcgagggcgagggcgatgccacctacggcaagctgaccctgaagttcatctgcaccaccggcaagctgcccgtgccctggcccaccctcgtgaccaccctgacctacggcgtgcagtgcttcagccgctaccccgaccacatgaagcagcacgacttcttcaagtccgccatgcccgaaggctacgtccaggagcgcaccatcttcttcaaggacgacggcaactacaagacccgcgccgaggtgaagttcgagggcgacaccctggtgaaccgcatcgagctgaagggcatcgacttcaaggaggacggcaacatcctggggcacaagctggagtacaactacaacagccacaacgtctatatcatggccgacaagcagaagaacggcatcaaggtgaacttcaagatccgccacaacatcgaggacggcagcgtgcagctcgccgaccactaccagcagaacacccccatcggcgacggccccgtgctgctgcccgacaaccactacctgagcacccagtccgccctgagcaaagaccccaacgagaagcgcgatcacatggtcctgctggagttcgtgaccgccgccgggatcactctcggcatggacgagctgtacaaggaattctaacgctagagggcccgtttaaacccgctgatcagcctcgactgtgccttctagttgccagccatctgttgtttgcccctcccccgtgccttccttgaccctggaaggtgccactcccactgtcctttcctaataaaatgaggaaattgcatcgcattgtctgagtaggtgtcattctattctggggggtggggtggggcaggacagcaagggggaggattgggaagacaatagcaggcatgctggggatgcggtgggctctatggcttctgaggcggaaagaaccagctggggctctagggggtatccccacgcgccctgtagcggcgcattaagcgcggcgggtgtggtggttacgcgcagcgtgaccgctacacttgccagcgccctagcgcccgctcctttcgctttcttcccttcctttctcgccacgttcgccggctttccccgtcaagctctaaatcgggggctccctttagggttccgatttagtgctttacggcacctcgaccccaaaaaacttgattagggtgatggttcacgtagtgggccatcgccctgatagacggtttttcgccctttgacgttggagtccacgttctttaatagtggactcttgttccaaactggaacaacactcaaccctatctcggtctattcttttgatttataagggattttgccgatttcggcctattggttaaaaaatgagctgatttaacaaaaatttaacgcgaattaattctgtggaatgtgtgtcagttagggtgtggaaagtccccaggctccccagcaggcagaagtatgcaaagcatgcatctcaattagtcagcaaccaggtgtggaaagtccccaggctccccagcaggcagaagtatgcaaagcatgcatctcaattagtcagcaaccatagtcccgcccctaactccgcccatcccgcccctaactccgcccagttccgcccattctccgccccatggctgactaattttttttatttatgcagaggccgaggccgcctctgcctctgagctattccagaagtagtgaggaggcttttttggaggcctaggcttttgcaaaaagctcccgggagcttgtatatccattttcggatctgatcaagagacaggatgaggatcgtttcgcatgattgaacaagatggattgcacgcaggttctccggccgcttgggtggagaggctattcggctatgactgggcacaacagacaatcggctgctctgatgccgccgtgttccggctgtcagcgcaggggcgcccggttctttttgtcaagaccgacctgtccggtgccctgaatgaactgcaggacgaggcagcgcggctatcgtggctggccacgacgggcgttccttgcgcagctgtgctcgacgttgtcactgaagcgggaagggactggctgctattgggcgaagtgccggggcaggatctcctgtcatctcaccttgctcctgccgagaaagtatccatcatggctgatgcaatgcggcggctgcatacgcttgatccggctacctgcccattcgaccaccaagcgaaacatcgcatcgagcgagcacgtactcggatggaagccggtcttgtcgatcaggatgatctggacgaagagcatcaggggctcgcgccagccgaactgttcgccaggctcaaggcgcgcatgcccgacggcgaggatctcgtcgtgacccatggcgatgcctgcttgccgaatatcatggtggaaaatggccgcttttctggattcatcgactgtggccggctgggtgtggcggaccgctatcaggacatagcgttggctacccgtgatattgctgaagagcttggcggcgaatgggctgaccgcttcctcgtgctttacggtatcgccgctcccgattcgcagcgcatcgccttctatcgccttcttgacgagttcttctgagcgggactctggggttcgaaatgaccgaccaagcgacgcccaacctgccatcacgagatttcgattccaccgccgccttctatgaaaggttgggcttcggaatcgttttccgggacgccggctggatgatcctccagcgcggggatctcatgctggagttcttcgcccaccccaacttgtttattgcagcttataatggttacaaataaagcaatagcatcacaaatttcacaaataaagcatttttttcactgcattctagttgtggtttgtccaaactcatcaatgtatcttatcatgtctgtataccgtcgacctctagctagagcttggcgtaatcatggtcatagctgtttcctgtgtgaaattgttatccgctcacaattccacacaacatacgagccggaagcataaagtgtaaagcctggggtgcctaatgagtgagctaactcacattaattgcgttgcgctcactgcccgctttccagtcgggaaacctgtcgtgccagctgcattaatgaatcggccaacgcgcggggagaggcggtttgcgtattgggcgctcttccgcttcctcgctcactgactcgctgcgctcggtcgttcggctgcggcgagcggtatcagctcactcaaaggcggtaatacggttatccacagaatcaggggataacgcaggaaagaacatgtgagcaaaaggccagcaaaaggccaggaaccgtaaaaaggccgcgttgctggcgtttttccataggctccgcccccctgacgagcatcacaaaaatcgacgctcaagtcagaggtggcgaaacccgacaggactataaagataccaggcgtttccccctggaagctccctcgtgcgctctcctgttccgaccctgccgcttaccggatacctgtccgcctttctcccttcgggaagcgtggcgctttctcatagctcacgctgtaggtatctcagttcggtgtaggtcgttcgctccaagctgggctgtgtgcacgaaccccccgttcagcccgaccgctgcgccttatccggtaactatcgtcttgagtccaacccggtaagacacgacttatcgccactggcagcagccactggtaacaggattagcagagcgaggtatgtaggcggtgctacagagttcttgaagtggtggcctaactacggctacactagaagaacagtatttggtatctgcgctctgctgaagccagttaccttcggaaaaagagttggtagctcttgatccggcaaacaaaccaccgctggtagcggtttttttgtttgcaagcagcagattacgcgcagaaaaaaaggatctcaagaagatcctttgatcttttctacggggtctgacgctcagtggaacgaaaactcacgttaagggattttggtcatgagattatcaaaaaggatcttcacctagatccttttaaattaaaaatgaagttttaaatcaatctaaagtatatatgagtaaacttggtctgacagttaccaatgcttaatcagtgaggcacctatctcagcgatctgtctatttcgttcatccatagttgcctgactccccgtcgtgtagataactacgatacgggagggcttaccatctggccccagtgctgcaatgataccgcgagacccacgctcaccggctccagatttatcagcaataaaccagccagccggaagggccgagcgcagaagtggtcctgcaactttatccgcctccatccagtctattaattgttgccgggaagctagagtaagtagttcgccagttaatagtttgcgcaacgttgttgccattgctacaggcatcgtggtgtcacgctcgtcgtttggtatggcttcattcagctccggttcccaacgatcaaggcgagttacatgatcccccatgttgtgcaaaaaagcggttagctccttcggtcctccgatcgttgtcagaagtaagttggccgcagtgttatcactcatggttatggcagcactgcataattctcttactgtcatgccatccgtaagatgcttttctgtgactggtgagtactcaaccaagtcattctgagaatagtgtatgcggcgaccgagttgctcttgcccggcgtcaatacgggataataccgcgccacatagcagaactttaaaagtgctcatcattggaaaacgttcttcggggcgaaaactctcaaggatcttaccgctgttgagatccagttcgatgtaacccactcgtgcacccaactgatcttcagcatcttttactttcaccagcgtttctgggtgagcaaaaacaggaaggcaaaatgccgcaaaaaagggaataagggcgacacggaaatgttgaatactcatactcttcctttttcaatattattgaagcatttatcagggttattgtctcatgagcggatacatatttgaatgtatttagaaaaataaacaaataggggttccgcgcacatttccccgaaaagtgccacctgacgtc

SEQ ID NO: 7 - DNA, 2508 bp, Artificial Sequence
  pMA-SV40pA vector V1.C.2
ctaaattgtaagcgttaatattttgttaaaattcgcgttaaatttttgttaaatcagctcattttttaaccaataggccgaaatcggcaaaatcccttataaatcaaaagaatagaccgagatagggttgagtggccgctacagggcgctcccattcgccattcaggctgcgcaactgttgggaagggcgtttcggtgcgggcctcttcgctattacgccagctggcgaaagggggatgtgctgcaaggcgattaagttgggtaacgccagggttttcccagtcacgacgttgtaaaacgacggccagtgagcgcgacgtaatacgactcactatagggcgaattggcggaaggccgtcaaggccgcatgaattgttgttgttaacttgtttattgcagcttataatggttacaaataaagcaatagcatcacaaatttcacaaataaagcatttttttcactgcattctagttgtggtttgtccaaactcatcaatgtatcttatcatgtctggatctgcggatccaatctcgagctgggcctcatgggccttccgctcactgcccgctttccagtcgggaaacctgtcgtgccagctgcattaacatggtcatagctgtttccttgcgtattgggcgctctccgcttcctcgctcactgactcgctgcgctcggtcgttcgggtaaagcctggggtgcctaatgagcaaaaggccagcaaaaggccaggaaccgtaaaaaggccgcgttgctggcgtttttccataggctccgcccccctgacgagcatcacaaaaatcgacgctcaagtcagaggtggcgaaacccgacaggactataaagataccaggcgtttccccctggaagctccctcgtgcgctctcctgttccgaccctgccgcttaccggatacctgtccgcctttctcccttcgggaagcgtggcgctttctcatagctcacgctgtaggtatctcagttcggtgtaggtcgttcgctccaagctgggctgtgtgcacgaaccccccgttcagcccgaccgctgcgccttatccggtaactatcgtcttgagtccaacccggtaagacacgacttatcgccactggcagcagccactggtaacaggattagcagagcgaggtatgtaggcggtgctacagagttcttgaagtggtggcctaactacggctacactagaagaacagtatttggtatctgcgctctgctgaagccagttaccttcggaaaaagagttggtagctcttgatccggcaaacaaaccaccgctggtagcggtggtttttttgtttgcaagcagcagattacgcgcagaaaaaaaggatctcaagaagatcctttgatcttttctacggggtctgacgctcagtggaacgaaaactcacgttaagggattttggtcatgagattatcaaaaaggatcttcacctagatccttttaaattaaaaatgaagttttaaatcaatctaaagtatatatgagtaaacttggtctgacagttaccaatgcttaatcagtgaggcacctatctcagcgatctgtctatttcgttcatccatagttgcctgactccccgtcgtgtagataactacgatacgggagggcttaccatctggccccagtgctgcaatgataccgcgagaaccacgctcaccggctccagatttatcagcaataaaccagccagccggaagggccgagcgcagaagtggtcctgcaactttatccgcctccatccagtctattaattgttgccgggaagctagagtaagtagttcgccagttaatagtttgcgcaacgttgttgccattgctacaggcatcgtggtgtcacgctcgtcgtttggtatggcttcattcagctccggttcccaacgatcaaggcgagttacatgatcccccatgttgtgcaaaaaagcggttagctccttcggtcctccgatcgttgtcagaagtaagttggccgcagtgttatcactcatggttatggcagcactgcataattctcttactgtcatgccatccgtaagatgcttttctgtgactggtgagtactcaaccaagtcattctgagaatagtgtatgcggcgaccgagttgctcttgcccggcgtcaatacgggataataccgcgccacatagcagaactttaaaagtgctcatcattggaaaacgttcttcggggcgaaaactctcaaggatcttaccgctgttgagatccagttcgatgtaacccactcgtgcacccaactgatcttcagcatcttttactttcaccagcgtttctgggtgagcaaaaacaggaaggcaaaatgccgcaaaaaagggaataagggcgacacggaaatgttgaatactcatactcttcctttttcaatattattgaagcatttatcagggttattgtctcatgagcggatacatatttgaatgtatttagaaaaataaacaaataggggttccgcgcacatttccccgaaaagtgccac

SEQ ID NO: 8 - DNA, 4341 bp, Artificial Sequence
  HLA-A 02:01 6xHis + Exon2/3-HA-L+R vector V1.C.6
ctaaattgtaagcgttaatattttgttaaaattcgcgttaaatttttgttaaatcagctcattttttaaccaataggccgaaatcggcaaaatcccttataaatcaaaagaatagaccgagatagggttgagtggccgctacagggcgctcccattcgccattcaggctgcgcaactgttgggaagggcgtttcggtgcgggcctcttcgctattacgccagctggcgaaagggggatgtgctgcaaggcgattaagttgggtaacgccagggttttcccagtcacgacgttgtaaaacgacggccagtgagcgcgacgtaatacgactcactatagggcgaattggcggaaggccgtcaaggccgcatgaattcgctaccggtatagtaatcaattacggggtcattagttcatagcccatatatggagttccgcgttacataacttacggtaaatggcccgcctggctgaccgcccaacgacccccgcccattgacgtcaataatgacgtatgttcccatagtaacgccaatagggactttccattgacgtcaatgggtggagtatttacggtaaactgcccacttggcagtacatcaagtgtatcatatgccaagtacgccccctattgacgtcaatgacggtaaatggcccgcctggcattatgcccagtacatgaccttatgggactttcctacttggcagtacatctacgtattagtcatcgctattaccatggtgatgcggttttggcagtacatcaatgggcgtggatagcggtttgactcacggggatttccaagtctccaccccattgacgtcaatgggagtttgttttggcaccaaaatcaacgggactttccaaaatgtcgtaacaactccgccccattgacgcaaatgggcggtaggcgtgtacggtgggaggtctatataagcagagctggtttagtgaaccgtcagatcaggtaccatggccgtcatggcgccccgaaccctcgtcctgctactctcgggggctctggccctgacccagacctgggcgggctctcactccatgaggtatttcttcacatccgtgtctcggccaggacgcggagagccacgcttcatcgcagtgggctacgtggacgacacgcagttcgtgcggttcgacagcgacgccgcgagccagaggatggagccgcgggcgccgtggatagagcaggagggtccggagtattgggacggggagacacggaaagtgaaggcccactcacagactcaccgagtggacctggggaccctgcgcggctactacaaccagagcgaggccggttctcacaccgtccagaggatgtatggctgcgacgtggggtcggactggcgcttcctccgcggataccaccagtacgcctacgacggcaaggattacatcgccctgaaagaggacctgcgctcttggaccgcggcggacatggcagctcagaccaccaagcacaagtgggaggcggcccatgtggcggagcagttgagagcctacctggagggcacgtgcgtggagtggctccgcagatacctggagaacgggaaggagacgctgcagcgcacggacgcccccaaaacgcatatgactcaccacgctgtctctgaccatgaagccaccctgaggtgctgggccctgagcttctaccctgcggagatcacactgacctggcagcgggatggggaggaccagacccaggacacggagctcgtggagaccaggcctgcaggggatggaaccttccagaagtgggcggctgtggtggtgccttctggacaggagcagagatacacctgccatgtgcagcatgagggtttgcccaagcccctcaccctgagatgggagccgtcttcccagcccaccatccccatcgtgggcatcattgctggcctggttctctttggagctgtgatcactggagctgtggtcgctgctgtgatgtggaggaggaagagctcagatagaaaaggagggagctactctcaggctgcaagcagtgacagtgcccagggctctgatgtgtctctcacagcttgtaaagtgcccgggcatcatcaccatcaccactgactatagtcgtctagacctgatcataatcaagccatatcacatctgtagaggtttacttgctttaaaaaacctccacacctccccctgaacctgaaacataaaatgaatgcaattgttgttgttaacttgtttattgcagcttataatggttacaaataaagcaatagcatcacaaatttcacaaataaagcatttttttcactgcattctagttgtggtttgtccaaactcatcaatgtatcttatcatgtctggatctgcggatccaatctcgagctgggcctcatgggccttccgctcactgcccgctttccagtcgggaaacctgtcgtgccagctgcattaacatggtcatagctgtttccttgcgtattgggcgctctccgcttcctcgctcactgactcgctgcgctcggtcgttcgggtaaagcctggggtgcctaatgagcaaaaggccagcaaaaggccaggaaccgtaaaaaggccgcgttgctggcgtttttccataggctccgcccccctgacgagcatcacaaaaatcgacgctcaagtcagaggtggcgaaacccgacaggactataaagataccaggcgtttccccctggaagctccctcgtgcgctctcctgttccgaccctgccgcttaccggatacctgtccgcctttctcccttcgggaagcgtggcgctttctcatagctcacgctgtaggtatctcagttcggtgtaggtcgttcgctccaagctgggctgtgtgcacgaaccccccgttcagcccgaccgctgcgccttatccggtaactatcgtcttgagtccaacccggtaagacacgacttatcgccactggcagcagccactggtaacaggattagcagagcgaggtatgtaggcggtgctacagagttcttgaagtggtggcctaactacggctacactagaagaacagtatttggtatctgcgctctgctgaagccagttaccttcggaaaaagagttggtagctcttgatccggcaaacaaaccaccgctggtagcggtggtttttttgtttgcaagcagcagattacgcgcagaaaaaaaggatctcaagaagatcctttgatcttttctacggggtctgacgctcagtggaacgaaaactcacgttaagggattttggtcatgagattatcaaaaaggatcttcacctagatccttttaaattaaaaatgaagttttaaatcaatctaaagtatatatgagtaaacttggtctgacagttaccaatgcttaatcagtgaggcacctatctcagcgatctgtctatttcgttcatccatagttgcctgactccccgtcgtgtagataactacgatacgggagggcttaccatctggccccagtgctgcaatgataccgcgagaaccacgctcaccggctccagatttatcagcaataaaccagccagccggaagggccgagcgcagaagtggtcctgcaactttatccgcctccatccagtctattaattgttgccgggaagctagagtaagtagttcgccagttaatagtttgcgcaacgttgttgccattgctacaggcatcgtggtgtcacgctcgtcgtttggtatggcttcattcagctccggttcccaacgatcaaggcgagttacatgatcccccatgttgtgcaaaaaagcggttagctccttcggtcctccgatcgttgtcagaagtaagttggccgcagtgttatcactcatggttatggcagcactgcataattctcttactgtcatgccatccgtaagatgcttttctgtgactggtgagtactcaaccaagtcattctgagaatagtgtatgcggcgaccgagttgctcttgcccggcgtcaatacgggataataccgcgccacatagcagaactttaaaagtgctcatcattggaaaacgttcttcggggcgaaaactctcaaggatcttaccgctgttgagatccagttcgatgtaacccactcgtgcacccaactgatcttcagcatcttttactttcaccagcgtttctgggtgagcaaaaacaggaaggcaaaatgccgcaaaaaagggaataagggcgacacggaaatgttgaatactcatactcttcctttttcaatattattgaagcatttatcagggttattgtctcatgagcggatacatatttgaatgtatttagaaaaataaacaaataggggttccgcgcacatttccccgaaaagtgccac

SEQ ID NO: 9 - DNA, 4332 bp, Artificial Sequence
  HLA-B 35:01 6xHis + Exon2/3-HA-L+R vector V1.C.9
ctaaattgtaagcgttaatattttgttaaaattcgcgttaaatttttgttaaatcagctcattttttaaccaataggccgaaatcggcaaaatcccttataaatcaaaagaatagaccgagatagggttgagtggccgctacagggcgctcccattcgccattcaggctgcgcaactgttgggaagggcgtttcggtgcgggcctcttcgctattacgccagctggcgaaagggggatgtgctgcaaggcgattaagttgggtaacgccagggttttcccagtcacgacgttgtaaaacgacggccagtgagcgcgacgtaatacgactcactatagggcgaattggcggaaggccgtcaaggccgcatgaattcgctaccggtatagtaatcaattacggggtcattagttcatagcccatatatggagttccgcgttacataacttacggtaaatggcccgcctggctgaccgcccaacgacccccgcccattgacgtcaataatgacgtatgttcccatagtaacgccaatagggactttccattgacgtcaatgggtggagtatttacggtaaactgcccacttggcagtacatcaagtgtatcatatgccaagtacgccccctattgacgtcaatgacggtaaatggcccgcctggcattatgcccagtacatgaccttatgggactttcctacttggcagtacatctacgtattagtcatcgctattaccatggtgatgcggttttggcagtacatcaatgggcgtggatagcggtttgactcacggggatttccaagtctccaccccattgacgtcaatgggagtttgttttggcaccaaaatcaacgggactttccaaaatgtcgtaacaactccgccccattgacgcaaatgggcggtaggcgtgtacggtgggaggtctatataagcagagctggtttagtgaaccgtcagatcaggtaccatgcgggtcacggcgccccgaaccgtcctcctgctgctctggggggcagtggccctgaccgagacctgggccggctcccactccatgaggtatttctacaccgccatgtcccggccaggacgcggagagccacgcttcatcgcagtgggctacgtggacgacacccagttcgtgaggttcgacagcgacgccgcgagtccgaggacggagcctcgggcgccatggatagagcaggaggggccggagtattgggaccggaacacacagatcttcaagaccaacacacagacttaccgagagagcctgcggaacctgcgcggctactacaaccagagcgaggccgggtctcacatcatccagaggatgtatggctgcgacctggggcccgacgggcgcctcctccgcgggcatgaccagtccgcctacgacggcaaggattacatcgccctgaacgaggacctgagctcctggaccgcggcggacaccgcggctcagatcacccagcgcaagtgggaggcggcccgtgtggcggagcagctgagagcctacctggagggcctgtgcgtggagtggctccgcagatacctggagaacgggaaggagactcttcagcgcgcagatcctccaaagacacacgtgacccaccaccccgtctctgaccatgaggccaccctgaggtgctgggccctgggcttctaccctgcggagatcacactgacctggcagcgggatggcgaggaccaaactcaggacactgagcttgtggagaccagaccagcaggagatagaaccttccagaagtgggcagctgtggtggtgccttctggagaagagcagagatacacatgccatgtacagcatgaggggctgccgaagcccctcaccctgagatgggagccatcttcccagtccaccatccccatcgtgggcattgttgctggcctggctgtcctagcagttgtggtcatcggagctgtggtcgctactgtgatgtgtaggaggaagagctcaggtggaaaaggagggagctactctcaggctgcgtccagcgacagtgcccagggctctgatgtgtctctcacagctcccgggcatcatcaccatcaccactgactatagtcgtctagacctgatcataatcaagccatatcacatctgtagaggtttacttgctttaaaaaacctccacacctccccctgaacctgaaacataaaatgaatgcaattgttgttgttaacttgtttattgcagcttataatggttacaaataaagcaatagcatcacaaatttcacaaataaagcatttttttcactgcattctagttgtggtttgtccaaactcatcaatgtatcttatcatgtctggatctgcggatccaatctcgagctgggcctcatgggccttccgctcactgcccgctttccagtcgggaaacctgtcgtgccagctgcattaacatggtcatagctgtttccttgcgtattgggcgctctccgcttcctcgctcactgactcgctgcgctcggtcgttcgggtaaagcctggggtgcctaatgagcaaaaggccagcaaaaggccaggaaccgtaaaaaggccgcgttgctggcgtttttccataggctccgcccccctgacgagcatcacaaaaatcgacgctcaagtcagaggtggcgaaacccgacaggactataaagataccaggcgtttccccctggaagctccctcgtgcgctctcctgttccgaccctgccgcttaccggatacctgtccgcctttctcccttcgggaagcgtggcgctttctcatagctcacgctgtaggtatctcagttcggtgtaggtcgttcgctccaagctgggctgtgtgcacgaaccccccgttcagcccgaccgctgcgccttatccggtaactatcgtcttgagtccaacccggtaagacacgacttatcgccactggcagcagccactggtaacaggattagcagagcgaggtatgtaggcggtgctacagagttcttgaagtggtggcctaactacggctacactagaagaacagtatttggtatctgcgctctgctgaagccagttaccttcggaaaaagagttggtagctcttgatccggcaaacaaaccaccgctggtagcggtggtttttttgtttgcaagcagcagattacgcgcagaaaaaaaggatctcaagaagatcctttgatcttttctacggggtctgacgctcagtggaacgaaaactcacgttaagggattttggtcatgagattatcaaaaaggatcttcacctagatccttttaaattaaaaatgaagttttaaatcaatctaaagtatatatgagtaaacttggtctgacagttaccaatgcttaatcagtgaggcacctatctcagcgatctgtctatttcgttcatccatagttgcctgactccccgtcgtgtagataactacgatacgggagggcttaccatctggccccagtgctgcaatgataccgcgagaaccacgctcaccggctccagatttatcagcaataaaccagccagccggaagggccgagcgcagaagtggtcctgcaactttatccgcctccatccagtctattaattgttgccgggaagctagagtaagtagttcgccagttaatagtttgcgcaacgttgttgccattgctacaggcatcgtggtgtcacgctcgtcgtttggtatggcttcattcagctccggttcccaacgatcaaggcgagttacatgatcccccatgttgtgcaaaaaagcggttagctccttcggtcctccgatcgttgtcagaagtaagttggccgcagtgttatcactcatggttatggcagcactgcataattctcttactgtcatgccatccgtaagatgcttttctgtgactggtgagtactcaaccaagtcattctgagaatagtgtatgcggcgaccgagttgctcttgcccggcgtcaatacgggataataccgcgccacatagcagaactttaaaagtgctcatcattggaaaacgttcttcggggcgaaaactctcaaggatcttaccgctgttgagatccagttcgatgtaacccactcgtgcacccaactgatcttcagcatcttttactttcaccagcgtttctgggtgagcaaaaacaggaaggcaaaatgccgcaaaaaagggaataagggcgacacggaaatgttgaatactcatactcttcctttttcaatattattgaagcatttatcagggttattgtctcatgagcggatacatatttgaatgtatttagaaaaataaacaaataggggttccgcgcacatttccccgaaaagtgccac

SEQ ID NO: 10 - DNA, 5733 bp, Artificial Sequence
  AAVS1-L_B07_6xH vector V1.F.10
ctaaattgtaagcgttaatattttgttaaaattcgcgttaaatttttgttaaatcagctcattttttaaccaataggccgaaatcggcaaaatcccttataaatcaaaagaatagaccgagatagggttgagtggccgctacagggcgctcccattcgccattcaggctgcgcaactgttgggaagggcgtttcggtgcgggcctcttcgctattacgccagctggcgaaagggggatgtgctgcaaggcgattaagttgggtaacgccagggttttcccagtcacgacgttgtaaaacgacggccagtgagcgcgacgtaatacgactcactatagggcgaattggcggaaggccgtcaaggccgcatgaattgagctctactggcttctgcgccgcctctggcccactgtttccccttcccaggcaggtcctgctttctctgacctgcattctctcccctgggcctgtgccgctttctgtctgcagcttgtggcctgggtcacctctacggctggcccagatccttccctgccgcctccttcaggttccgtcttcctccactccctcttccccttgctctctgctgtgttgctgcccaaggatgctctttccggagcacttccttctcggcgctgcaccacgtgatgtcctctgagcggatcctccccgtgtctgggtcctctccgggcatctctcctccctcacccaaccccatgccgtcttcactcgctgggttcccttttccttctccttctggggcctgtgccatctctcgtttcttaggatggccttctccgacggatgtctcccttgcgtcccgcctccccttcttgtaggcctgcatcatcaccgtttttctggacaaccccaaagtaccccgtctccctggctttagccacctctccatcctcttgctttctttgcctggacaccccgttctcctgtggattcgggtcacctctcactcctttcatttgggcagctcccctaccccccttacctctctagtctgtgctagctcttccagccccctgtcatggcatcttccaggggtccgagagctcagctagtcttcttcctccaacccgggcccctatgtccacttcaggacagcatgtttgctgcctccagggatcctgtgtccccgagctgggaccaccttatattcccagggccggttaatgtggctctggttctgggtacttttatctgtcccctccaccggtatagtaatcaattacggggtcattagttcatagcccatatatggagttccgcgttacataacttacggtaaatggcccgcctggctgaccgcccaacgacccccgcccattgacgtcaataatgacgtatgttcccatagtaacgccaatagggactttccattgacgtcaatgggtggagtatttacggtaaactgcccacttggcagtacatcaagtgtatcatatgccaagtacgccccctattgacgtcaatgacggtaaatggcccgcctggcattatgcccagtacatgaccttatgggactttcctacttggcagtacatctacgtattagtcatcgctattaccatggtgatgcggttttggcagtacatcaatgggcgtggatagcggtttgactcacggggatttccaagtctccaccccattgacgtcaatgggagtttgttttggcaccaaaatcaacgggactttccaaaatgtcgtaacaactccgccccattgacgcaaatgggcggtaggcgtgtacggtgggaggtctatataagcagagctggtttagtgaaccgtcagatcaggtaccatgctggtcatggcgccccgaaccgtcctcctgctgctctcggcggccctggccctgaccgagacctgggccggctcccactccatgaggtatttctacacctccgtgtctcggccaggacgcggagagccacgcttcatctcagtgggctacgtggacgacacccagttcgtgaggttcgacagcgacgccgcgagtccgagagaggagccgcgggcgccgtggatagagcaggaggggccggagtattgggaccggaacacacagatctacaaggcccaggcacagactgaccgagagagcctgcggaacctgcgcggctactacaaccagagcgaggccgggtctcacaccctccagagcatgtacggctgcgacgtggggccggacgggcgcctcctccgcgggcatgaccagtacgcctacgacggcaaggattacatcgccctgaacgaggacctgcgctcctggaccgccgcggacacggcggctcagatcacccagcgcaagtgggaggcggcccgtgaggcggagcagcggagagcctacctggagggcgagtgcgtggagtggctccgcagatacctggagaacgggaaggacaaacttgagcgcgcagaccctccaaagacacacgtgacccaccaccccatctctgaccatgaggccaccctgaggtgctgggccctgggtttctaccctgcggagatcacactgacctggcagcgggatggcgaggaccaaactcaggacactgagcttgtggagaccagaccagcaggagatagaaccttccagaagtgggcagctgtggtggtgccttctggagaagagcagagatacacatgccatgtacagcatgaggggctgccgaagcccctcaccctgagatgggagccgtcttcccagtccaccgtccccatcgtgggcattgttgctggcctggctgtcctagcagttgtggtcatcggagctgtggtcgctgctgtgatgtgtaggaggaagagttcaggtggaaaaggagggagctactctcaggctgcgtgcagcgacagtgcccagggctctgatgtgtctctcacagctcccgggcatcatcaccatcaccactgactatagtcgtctagacctgatcataatcaagccatatcacatctgtagaggtttacttgctttaaaaaacctccacacctccccctgaacctgaaacataaaatgaatgcaattgttgttgttaacttgtttattgcagcttataatggttacaaataaagcaatagcatcacaaatttcacaaataaagcatttttttcactgcattctagttgtggtttgtccaaactcatcaatgtatcttatcatgtctggatctgcggatcaggattggtgacagaaaagccccatccttaggcctcctccttcctagtctcctgatattgggtctaacccccacctcctgttaggcagattccttatctggtgacacacccccatttcctggagccatctctctccttgccagaacctctaaggtttgcttacgatggagccagagaggatcctgggagggagagcttggcagggggtgggagggaagggggggatgcgtgacctgcccggttctcagtggccaccctgcgctaccctctcccagaacctgagctgctctgacgcggctgtctggtgcgtttcactgatcctggtgctgcagcttccttacacttcccaagaggagaagcagtttggaaaaacaaaatcagaataagttggtcctgagttctaactttggctcttcacctttctagtccccaatttatattgttcctccgtgcgtcagttttacctgtgagataaggccagtagccagccccgtcctggcagggctgtggtgaggaggggggtgtccgtgtggaaaactccctttgtgagaatggtgcgtcctcgagctgggcctcatgggccttccgctcactgcccgctttccagtcgggaaacctgtcgtgccagctgcattaacatggtcatagctgtttccttgcgtattgggcgctctccgcttcctcgctcactgactcgctgcgctcggtcgttcgggtaaagcctggggtgcctaatgagcaaaaggccagcaaaaggccaggaaccgtaaaaaggccgcgttgctggcgtttttccataggctccgcccccctgacgagcatcacaaaaatcgacgctcaagtcagaggtggcgaaacccgacaggactataaagataccaggcgtttccccctggaagctccctcgtgcgctctcctgttccgaccctgccgcttaccggatacctgtccgcctttctcccttcgggaagcgtggcgctttctcatagctcacgctgtaggtatctcagttcggtgtaggtcgttcgctccaagctgggctgtgtgcacgaaccccccgttcagcccgaccgctgcgccttatccggtaactatcgtcttgagtccaacccggtaagacacgacttatcgccactggcagcagccactggtaacaggattagcagagcgaggtatgtaggcggtgctacagagttcttgaagtggtggcctaactacggctacactagaagaacagtatttggtatctgcgctctgctgaagccagttaccttcggaaaaagagttggtagctcttgatccggcaaacaaaccaccgctggtagcggtggtttttttgtttgcaagcagcagattacgcgcagaaaaaaaggatctcaagaagatcctttgatcttttctacggggtctgacgctcagtggaacgaaaactcacgttaagggattttggtcatgagattatcaaaaaggatcttcacctagatccttttaaattaaaaatgaagttttaaatcaatctaaagtatatatgagtaaacttggtctgacagttaccaatgcttaatcagtgaggcacctatctcagcgatctgtctatttcgttcatccatagttgcctgactccccgtcgtgtagataactacgatacgggagggcttaccatctggccccagtgctgcaatgataccgcgagaaccacgctcaccggctccagatttatcagcaataaaccagccagccggaagggccgagcgcagaagtggtcctgcaactttatccgcctccatccagtctattaattgttgccgggaagctagagtaagtagttcgccagttaatagtttgcgcaacgttgttgccattgctacaggcatcgtggtgtcacgctcgtcgtttggtatggcttcattcagctccggttcccaacgatcaaggcgagttacatgatcccccatgttgtgcaaaaaagcggttagctccttcggtcctccgatcgttgtcagaagtaagttggccgcagtgttatcactcatggttatggcagcactgcataattctcttactgtcatgccatccgtaagatgcttttctgtgactggtgagtactcaaccaagtcattctgagaatagtgtatgcggcgaccgagttgctcttgcccggcgtcaatacgggataataccgcgccacatagcagaactttaaaagtgctcatcattggaaaacgttcttcggggcgaaaactctcaaggatcttaccgctgttgagatccagttcgatgtaacccactcgtgcacccaactgatcttcagcatcttttactttcaccagcgtttctgggtgagcaaaaacaggaaggcaaaatgccgcaaaaaagggaataagggcgacacggaaatgttgaatactcatactcttcctttttcaatattattgaagcatttatcagggttattgtctcatgagcggatacatatttgaatgtatttagaaaaataaacaaataggggttccgcgcacatttccccgaaaagtgccac

SEQ ID NO: 11 - DNA, 5520 bp, Artificial Sequence
  AAVS1-S_A24_6xH vector V1.F.8
ctaaattgtaagcgttaatattttgttaaaattcgcgttaaatttttgttaaatcagctcattttttaaccaataggccgaaatcggcaaaatcccttataaatcaaaagaatagaccgagatagggttgagtggccgctacagggcgctcccattcgccattcaggctgcgcaactgttgggaagggcgtttcggtgcgggcctcttcgctattacgccagctggcgaaagggggatgtgctgcaaggcgattaagttgggtaacgccagggttttcccagtcacgacgttgtaaaacgacggccagtgagcgcgacgtaatacgactcactatagggcgaattggcggaaggccgtcaaggccgcatgaattgctgcccaaggatgctctttccggagcacttccttctcggcgctgcaccacgtgatgtcctctgagcggatcctccccgtgtctgggtcctctccgggcatctctcctccctcacccaaccccatgccgtgttcactcgctgggttcccttttccttctccttctggggcctgtgccatctctcgtttcttaggatggccttctccgacggatgtctcccttgcgtcccgcctccccttcttgtaggcctgcatcatcaccgtttttctggacaaccccaaagtaccccgtctccctggcttagcacctctccatcctcttgctttctttgcctggacaccccgttctcctgtggattcgggtcacctctcactcctttcatttgggcagctcccctaccccccttacctctctagtctgtgctagctcttccagccccctgtcatggcatcttccaggggtccgagagctcagctagtcttcttcctccaacccgggccctatgtccacttcaggacagcatgtttgctgcctccagggatcctgtgtccccgagctgggaccaccttatattcccagggccggttaatgtggctctggttctgggtacttttatctgtcccctccaccggtatagtaatcaattacggggtcattagttcatagcccatatatggagttccgcgttacataacttacggtaaatggcccgcctggctgaccgcccaacgacccccgcccattgacgtcaataatgacgtatgttcccatagtaacgccaatagggactttccattgacgtcaatgggtggagtatttacggtaaactgcccacttggcagtacatcaagtgtatcatatgccaagtacgccccctattgacgtcaatgacggtaaatggcccgcctggcattatgcccagtacatgaccttatgggactttcctacttggcagtacatctacgtattagtcatcgctattaccatggtgatgcggttttggcagtacatcaatgggcgtggatagcggtttgactcacggggatttccaagtctccaccccattgacgtcaatgggagtttgttttggcaccaaaatcaacgggactttccaaaatgtcgtaacaactccgccccattgacgcaaatgggcggtaggcgtgtacggtgggaggtctatataagcagagctggtttagtgaaccgtcagatcaggtaccatggccgtcatggcgccccgaaccctcgtcctgctactctcgggggccctggccctgacccagacctgggcaggctcccactccatgaggtatttctccacatccgtgtctcggccaggacgcggagagccacgcttcatcgccgtgggctacgtggacgacacgcagttcgtgcggttcgacagcgacgccgcgagccagaggatggagccgcgggcgccgtggatagagcaggaggggccggagtattgggacgaggagacagggaaagtgaaggcccactcacagactgaccgagagaacctgcggatcgcgctccgctactacaaccagagcgaggccggttctcacaccctccagatgatgtttggctgcgacgtggggtcggacgggcgcttcctccgcggataccaccagtacgcctacgacggcaaggattacatcgccctgaaagaggacctgcgctcttggaccgcggcggacatggcggctcagatcaccaagcgcaagtgggaggcggcccatgtggcggagcagcagagagcctacctggagggcacgtgcgtggacgggctccgcagatacctggagaacgggaaggagacgctgcagcgcacggacccccccaagacacatatgacccaccaccccatctctgaccatgaggccactctgagatgctgggccctgggcttctaccctgcggagatcacactgacctggcagcgggatggggaggaccagacccaggacacggagcttgtggagaccaggcctgcaggggatggaaccttccagaagtgggcagctgtggtggttccttctggagaggagcagagatacacctgccatgtgcagcatgagggtctgcccaagcccctcaccctgagatgggagccatcttcccagcccaccgtccccatcgtgggcatcattgctggcctggttctccttggagctgtgatcactggagctgtggtcgctgctgtgatgtggaggaggaacagctcagatagaaaaggagggagctactctcaggctgcaagcagtgacagtgcccagggctctgatgtgtctctcacagcttgtaaagtgcccgggcatcatcaccatcaccactgactatagtcgtctagacctgatcataatcaagccatatcacatctgtagaggtttacttgctttaaaaaacctccacacctccccctgaacctgaaacataaaatgaatgcaattgttgttgttaacttgtttattgcagcttataatggttacaaataaagcaatagcatcacaaatttcacaaataaagcatttttttcactgcattctagttgtggtttgtccaaactcatcaatgtatcttatcatgtctggatctgcggatcaggattggtgacagaaaagcccccatccttaggcctcctccttcctagtctcctgatattcgtctaacccccacctcctgttaggcagattccttatctggtgacacacccccatttcctggagccatctctctccttgccagaacctctaaggtttgcttacgatggagccagagaggatcctgggagggagacttggcagggggtgggagggaagggggggatgcgtgacctgcccggttctcagtggccaccctgcgctaccctctcccagaacctgagctgctctgacgcggctgtctggtgcgtttcactgatcctggtgctgcagcttccttacacttcccaagaggagaagcagtttggaaaaacaaaatcagaataagttggtcctgagttctaactttggctcttcacctttctagcccccaatttatattgttcctccgtgcgtcagttttacctgtgagataaggccagtagccacccccgtcctggcagggctgtggtgaggaggggggtgtccgtgtggaaaactccctttgtgagaatggtgcgtcctcgagctgggcctcatgggccttccgctcactgcccgctttccagtcgggaaacctgtcgtgccagctgcattaacatggtcatagctgtttccttgcgtattgggcgctctccgcttcctcgctcactgactcgctgcgctcggtcgttcgggtaaagcctggggtgcctaatgagcaaaaggccagcaaaaggccaggaaccgtaaaaaggccgcgttgctggcgtttttccataggctccgcccccctgacgagcatcacaaaaatcgacgctcaagtcagaggtggcgaaacccgacaggactataaagataccaggcgtttccccctggaagctccctcgtgcgctctcctgttccgaccctgccgcttaccggatacctgtccgcctttctcccttcgggaagcgtggcgctttctcatagctcacgctgtaggtatctcagttcggtgtaggtcgttcgctccaagctgggctgtgtgcacgaaccccccgttcagcccgaccgctgcgccttatccggtaactatcgtcttgagtccaacccggtaagacacgacttatcgccactggcagcagccactggtaacaggattagcagagcgaggtatgtaggcggtgctacagagttcttgaagtggtggcctaactacggctacactagaagaacagtatttggtatctgcgctctgctgaagccagttaccttcggaaaaagagttggtagctcttgatccggcaaacaaaccaccgctggtagcggtggtttttttgtttgcaagcagcagattacgcgcagaaaaaaaggatctcaagaagatcctttgatcttttctacggggtctgacgctcagtggaacgaaaactcacgttaagggattttggtcatgagattatcaaaaaggatcttcacctagatccttttaaattaaaaatgaagttttaaatcaatctaaagtatatatgagtaaacttggtctgacagttaccaatgcttaatcagtgaggcacctatctcagcgatctgtctatttcgttcatccatagttgcctgactccccgtcgtgtagataactacgatacgggagggcttaccatctggccccagtgctgcaatgataccgcgagaaccacgctcaccggctccagatttatcagcaataaaccagccagccggaagggccgagcgcagaagtggtcctgcaactttatccgcctccatccagtctattaattgttgccgggaagctagagtaagtagttcgccagttaatagtttgcgcaacgttgttgccattgctacaggcatcgtggtgtcacgctcgtcgtttggtatggcttcattcagctccggttcccaacgatcaaggcgagttacatgatcccccatgttgtgcaaaaaagcggttagctccttcggtcctccgatcgttgtcagaagtaagttggccgcagtgttatcactcatggttatggcagcactgcataattctcttactgtcatgccatccgtaagatgcttttctgtgactggtgagtactcaaccaagtcattctgagaatagtgtatgcggcgaccgagttgctcttgcccggcgtcaatacgggataataccgcgccacatagcagaactttaaaagtgctcatcattggaaaacgttcttcggggcgaaaactctcaaggatcttaccgctgttgagatccagttcgatgtaacccactcgtgcacccaactgatcttcagcatcttttactttcaccagcgtttctgggtgagcaaaaacaggaaggcaaaatgccgcaaaaaagggaataagggcgacacggaaatgttgaatactcatactcttcctttttcaatattattgaagcatttatcagggttattgtctcatgagcggatacatatttgaatgtatttagaaaaataaacaaataggggttccgcgcacatttccccgaaaagtgccac

SEQ ID NO: 12 - DNA, 7062 bp, Artificial Sequence
  AAVS1-l_GFP_HCMVpp65 vector V1.G.10
ctaaattgtaagcgttaatattttgttaaaattcgcgttaaatttttgttaaatcagctcattttttaaccaataggccgaaatcggcaaaatcccttataaatcaaaagaatagaccgagatagggttgagtggccgctacagggcgctcccattcgccattcaggctgcgcaactgttgggaagggcgtttcggtgcgggcctcttcgctattacgccagctggcgaaagggggatgtgctgcaaggcgattaagttgggtaacgccagggttttcccagtcacgacgttgtaaaacgacggccagtgagcgcgacgtaatacgactcactatagggcgaattggcggaaggccgtcaaggccgcatgaattgagctctactggcttctgcgccgcctctggcccactgtttccccttcccaggcaggtcctgctttctctgacctgcattctctcccctgggcctgtgccgctttctgtctgcagcttgtggcctgggtcacctctacggctggcccagatccttccctgccgcctccttcaggttccgtcttcctccactccctcttccccttgctctctgctgtgttgctgcccaaggatgctctttccggagcacttccttctcggcgctgcaccacgtgatgtcctctgagcggatcctccccgtgtctgggtcctctccgggcatctctcctccctcacccaaccccatgccgtcttcactcgctgggttcccttttccttctccttctggggcctgtgccatctctcgtttcttaggatggccttctccgacggatgtctcccttgcgtcccgcctccccttcttgtaggcctgcatcatcaccgtttttctggacaaccccaaagtaccccgtctccctggctttagccacctctccatcctcttgctttctttgcctggacaccccgttctcctgtggattcgggtcacctctcactcctttcatttgggcagctcccctaccccccttacctctctagtctgtgctagctcttccagccccctgtcatggcatcttccaggggtccgagagctcagctagtcttcttcctccaacccgggcccctatgtccacttcaggacagcatgtttgctgcctccagggatcctgtgtccccgagctgggaccaccttatattcccagggccggttaatgtggctctggttctgggtacttttatctgtcccctccaccggtatagtaatcaattacggggtcattagttcatagcccatatatggagttccgcgttacataacttacggtaaatggcccgcctggctgaccgcccaacgacccccgcccattgacgtcaataatgacgtatgttcccatagtaacgccaatagggactttccattgacgtcaatgggtggagtatttacggtaaactgcccacttggcagtacatcaagtgtatcatatgccaagtacgccccctattgacgtcaatgacggtaaatggcccgcctggcattatgcccagtacatgaccttatgggactttcctacttggcagtacatctacgtattagtcatcgctattaccatggtgatgcggttttggcagtacatcaatgggcgtggatagcggtttgactcacggggatttccaagtctccaccccattgacgtcaatgggagtttgttttggcaccaaaatcaacgggactttccaaaatgtcgtaacaactccgccccattgacgcaaatgggcggtaggcgtgtacggtgggaggtctatataagcagagctggtttagtgaaccgtcagatcaggtaccgccaccatggaatccgatgagtctggcctgcccgccatggaaatcgagtgcagaatcaccggcaccctgaacggcgtggaatttgagctcgtgggcggaggcgagggcacacctgaacagggcagaatgaccaacaagatgaagtccaccaagggggccctgaccttcagcccctacctgctgtctcacgtgatgggctacggcttctaccacttcggcacctaccccagcggctacgagaaccctttcctgcacgccatcaacaacggcggctacaccaacacccggatcgagaagtacgaggacggcggcgtgctgcacgtgtccttcagctacagatacgaggccggcagagtgatcggcgacttcaaagtgatgggcaccggattccccgaggacagcgtgatcttcaccgacaagatcatccggtccaacgccaccgtggaacatctgcaccccatgggcgacaacgacctggacggcagcttcaccagaaccttctccctgcgggatggcggctactacagcagcgtggtggacagccacatgcacttcaagagcgccatccaccccagcatcctccagaacggcggacccatgttcgccttcagacgggtggaagaggaccacagcaacaccgagctgggcatcgtggaataccagcacgccttcaagacccccgatgccgatgccggcgaggaaggcagtggagagggcagaggaagtctgctaacatgtggtgacgtcgaggagaatcctggcccaatggagtcgcgcggtcgccgttgtcccgaaatgatatccgtactgggtcccatttcggggcacgtgctgaaagccgtgtttagtcgcggcgatacgccggtgctgccgcacgagacgcgactcctgcagacgggtatccacgtacgcgtgagccagccctcgctgatcttggtatcgcagtacacgcccgactcgacgccatgccaccgcggcgacaatcagctgcaggtgcagcacacgtactttacgggcagcgaggtggagaacgtgtcggtcaacgtgcacaaccccacgggccgaagcatctgccccagccaggagcccatgtcgatctatgtgtacgcgctgccgctcaagatgctgaacatccccagcatcaacgtgcaccactacccgtcggcggccgagcgcaaacaccgacacctgcccgtagctgacgctgtgattcacgcgtcgggcaagcagatgtggcaggcgcgtctcacggtctcgggactggcctggacgcgtcagcagaaccagtggaaagagcccgacgtctactacacgtcagcgttcgtgtttcccaccaaggacgtggcactgcggcacgtggtgtgcgcgcacgagctggtttgctccatggagaacacgcgcgcaaccaagatgcaggtgataggtgaccagtacgtcaaggtgtacctggagtccttctgcgaggacgtgccctccggcaagctctttatgcacgtcacgctgggctctgacgtggaagaggacctgacgatgacccgcaacccgcaacccttcatgcgcccccacgagcgcaacggctttacggtgttgtgtcccaaaaatatgataatcaaaccgggcaagatctcgcacatcatgctggatgtggcttttacctcacacgagcattttgggctgctgtgtcccaagagcatcccgggcctgagcatctcaggtaacctgttgatgaacgggcagcagatcttcctggaggtacaagccatacgcgagaccgtggaactgcgtcagtacgatcccgtggctgcgctcttctttttcgatatcgacttgctgctgcagcgcgggcctcagtacagcgagcaccccaccttcaccagccagtatcgcatccagggcaagcttgagtaccgacacacctgggaccggcacgacgagggtgccgcccagggcgacgacgacgtctggaccagcggatcggactccgacgaagaactcgtaaccaccgagcgcaagacgccccgcgtcaccggcggcggcgccatggcgggcgcctccacttccgcgggccgcaaacgcaaatcagcatcctcggcgacggcgtgcacgtcgggcgttatgacacgcggccgccttaaggccgagtccaccgtcgcgcccgaagaggacaccgacgaggattccgacaacgaaatccacaatccggccgtgttcacctggccgccctggcaggccggcatcctggcccgcaacctggtgcccatggtggctacggttcagggtcagaatctgaagtaccaggagttcttctgggacgccaacgacatctaccgcatcttcgccgaattggaaggcgtatggcagcccgctgcgcaacccaaacgtcgccgccaccggcaagacgccttgcccgggccatgcatcgcctcgacgcccaaaaagcaccgaggttgatctagacctgatcataatcaagccatatcacatctgtagaggtttacttgctttaaaaaacctccacacctccccctgaacctgaaacataaaatgaatgcaattgttgttgttaacttgtttattgcagcttataatggttacaaataaagcaatagcatcacaaatttcacaaataaagcatttttttcactgcattctagttgtggtttgtccaaactcatcaatgtatcttatcatgtctggatctgcggatcaggattggtgacagaaaagccccatccttaggcctcctccttcctagtctcctgatattgggtctaacccccacctcctgttaggcagattccttatctggtgacacacccccatttcctggagccatctctctccttgccagaacctctaaggtttgcttacgatggagccagagaggatcctgggagggagagcttggcagggggtgggagggaagggggggatgcgtgacctgcccggttctcagtggccaccctgcgctaccctctcccagaacctgagctgctctgacgcggctgtctggtgcgtttcactgatcctggtgctgcagcttccttacacttcccaagaggagaagcagtttggaaaaacaaaatcagaataagttggtcctgagttctaactttggctcttcacctttctagtccccaatttatattgttcctccgtgcgtcagttttacctgtgagataaggccagtagccagccccgtcctggcagggctgtggtgaggaggggggtgtccgtgtggaaaactccctttgtgagaatggtgcgtcctcgagctgggcctcatgggccttccgctcactgcccgctttccagtcgggaaacctgtcgtgccagctgcattaacatggtcatagctgtttccttgcgtattgggcgctctccgcttcctcgctcactgactcgctgcgctcggtcgttcgggtaaagcctggggtgcctaatgagcaaaaggccagcaaaaggccaggaaccgtaaaaaggccgcgttgctggcgtttttccataggctccgcccccctgacgagcatcacaaaaatcgacgctcaagtcagaggtggcgaaacccgacaggactataaagataccaggcgtttccccctggaagctccctcgtgcgctctcctgttccgaccctgccgcttaccggatacctgtccgcctttctcccttcgggaagcgtggcgctttctcatagctcacgctgtaggtatctcagttcggtgtaggtcgttcgctccaagctgggctgtgtgcacgaaccccccgttcagcccgaccgctgcgccttatccggtaactatcgtcttgagtccaacccggtaagacacgacttatcgccactggcagcagccactggtaacaggattagcagagcgaggtatgtaggcggtgctacagagttcttgaagtggtggcctaactacggctacactagaagaacagtatttggtatctgcgctctgctgaagccagttaccttcggaaaaagagttggtagctcttgatccggcaaacaaaccaccgctggtagcggtggtttttttgtttgcaagcagcagattacgcgcagaaaaaaaggatctcaagaagatcctttgatcttttctacggggtctgacgctcagtggaacgaaaactcacgttaagggattttggtcatgagattatcaaaaaggatcttcacctagatccttttaaattaaaaatgaagttttaaatcaatctaaagtatatatgagtaaacttggtctgacagttaccaatgcttaatcagtgaggcacctatctcagcgatctgtctatttcgttcatccatagttgcctgactccccgtcgtgtagataactacgatacgggagggcttaccatctggccccagtgctgcaatgataccgcgagaaccacgctcaccggctccagatttatcagcaataaaccagccagccggaagggccgagcgcagaagtggtcctgcaactttatccgcctccatccagtctattaattgttgccgggaagctagagtaagtagttcgccagttaatagtttgcgcaacgttgttgccattgctacaggcatcgtggtgtcacgctcgtcgtttggtatggcttcattcagctccggttcccaacgatcaaggcgagttacatgatcccccatgttgtgcaaaaaagcggttagctccttcggtcctccgatcgttgtcagaagtaagttggccgcagtgttatcactcatggttatggcagcactgcataattctcttactgtcatgccatccgtaagatgcttttctgtgactggtgagtactcaaccaagtcattctgagaatagtgtatgcggcgaccgagttgctcttgcccggcgtcaatacgggataataccgcgccacatagcagaactttaaaagtgctcatcattggaaaacgttcttcggggcgaaaactctcaaggatcttaccgctgttgagatccagttcgatgtaacccactcgtgcacccaactgatcttcagcatcttttactttcaccagcgtttctgggtgagcaaaaacaggaaggcaaaatgccgcaaaaaagggaataagggcgacacggaaatgttgaatactcatactcttcctttttcaatattattgaagcatttatcagggttattgtctcatgagcggatacatatttgaatgtatttagaaaaataaacaaataggggttccgcgcacatttccccgaaaagtgccac

SEQ ID NO: 13 - DNA, 7062 bp, Artificial Sequence
  AAVS1-l_GFP_HCMVpp65 ANET vector V1.G.9
ctaaattgtaagcgttaatattttgttaaaattcgcgttaaatttttgttaaatcagctcattttttaaccaataggccgaaatcggcaaaatcccttataaatcaaaagaatagaccgagatagggttgagtggccgctacagggcgctcccattcgccattcaggctgcgcaactgttgggaagggcgtttcggtgcgggcctcttcgctattacgccagctggcgaaagggggatgtgctgcaaggcgattaagttgggtaacgccagggttttcccagtcacgacgttgtaaaacgacggccagtgagcgcgacgtaatacgactcactatagggcgaattggcggaaggccgtcaaggccgcatgaattgagctctactggcttctgcgccgcctctggcccactgtttccccttcccaggcaggtcctgctttctctgacctgcattctctcccctgggcctgtgccgctttctgtctgcagcttgtggcctgggtcacctctacggctggcccagatccttccctgccgcctccttcaggttccgtcttcctccactccctcttccccttgctctctgctgtgttgctgcccaaggatgctctttccggagcacttccttctcggcgctgcaccacgtgatgtcctctgagcggatcctccccgtgtctgggtcctctccgggcatctctcctccctcacccaaccccatgccgtcttcactcgctgggttcccttttccttctccttctggggcctgtgccatctctcgtttcttaggatggccttctccgacggatgtctcccttgcgtcccgcctccccttcttgtaggcctgcatcatcaccgtttttctggacaaccccaaagtaccccgtctccctggctttagccacctctccatcctcttgctttctttgcctggacaccccgttctcctgtggattcgggtcacctctcactcctttcatttgggcagctcccctaccccccttacctctctagtctgtgctagctcttccagccccctgtcatggcatcttccaggggtccgagagctcagctagtcttcttcctccaacccgggcccctatgtccacttcaggacagcatgtttgctgcctccagggatcctgtgtccccgagctgggaccaccttatattcccagggccggttaatgtggctctggttctgggtacttttatctgtcccctccaccggtatagtaatcaattacggggtcattagttcatagcccatatatggagttccgcgttacataacttacggtaaatggcccgcctggctgaccgcccaacgacccccgcccattgacgtcaataatgacgtatgttcccatagtaacgccaatagggactttccattgacgtcaatgggtggagtatttacggtaaactgcccacttggcagtacatcaagtgtatcatatgccaagtacgccccctattgacgtcaatgacggtaaatggcccgcctggcattatgcccagtacatgaccttatgggactttcctacttggcagtacatctacgtattagtcatcgctattaccatggtgatgcggttttggcagtacatcaatgggcgtggatagcggtttgactcacggggatttccaagtctccaccccattgacgtcaatgggagtttgttttggcaccaaaatcaacgggactttccaaaatgtcgtaacaactccgccccattgacgcaaatgggcggtaggcgtgtacggtgggaggtctatataagcagagctggtttagtgaaccgtcagatcaggtaccgccaccatggaatccgatgagtctggcctgcccgccatggaaatcgagtgcagaatcaccggcaccctgaacggcgtggaatttgagctcgtgggcggaggcgagggcacacctgaacagggcagaatgaccaacaagatgaagtccaccaagggggccctgaccttcagcccctacctgctgtctcacgtgatgggctacggcttctaccacttcggcacctaccccagcggctacgagaaccctttcctgcacgccatcaacaacggcggctacaccaacacccggatcgagaagtacgaggacggcggcgtgctgcacgtgtccttcagctacagatacgaggccggcagagtgatcggcgacttcaaagtgatgggcaccggattccccgaggacagcgtgatcttcaccgacaagatcatccggtccaacgccaccgtggaacatctgcaccccatgggcgacaacgacctggacggcagcttcaccagaaccttctccctgcgggatggcggctactacagcagcgtggtggacagccacatgcacttcaagagcgccatccaccccagcatcctccagaacggcggacccatgttcgccttcagacgggtggaagaggaccacagcaacaccgagctgggcatcgtggaataccagcacgccttcaagacccccgatgccgatgccggcgaggaaggcagtggagagggcagaggaagtctgctaacatgtggtgacgtcgaggagaatcctggcccaatggagtcgcgcggtcgccgttgtcccgaaatgatatccgtactgggtcccatttcggggcacgtgctgaaagccgtgtttagtcgcggcgatacgccggtgctgccgcacgagacgcgactcctgcagacgggtatccacgtacgcgtgagccagccctcgctgatcttggtatcgcagtacacgcccgactcgacgccatgccaccgcggcgacaatcagctgcaggtgcagcacacgtactttacgggcagcgaggtggagaacgtgtcggtcaacgtgcacaaccccacgggccgaagcatctgccccagccaggagcccatgtcgatctatgtgtacgcgctgccgctcaagatgctgaacatccccagcgctaacgaaacccactacccgtcggcggccgagcgcaaacaccgacacctgcccgtagctgacgctgtgattcacgcgtcgggcaagcagatgtggcaggcgcgtctcacggtctcgggactggcctggacgcgtcagcagaaccagtggaaagagcccgacgtctactacacgtcagcgttcgtgtttcccaccaaggacgtggcactgcggcacgtggtgtgcgcgcacgagctggtttgctccatggagaacacgcgcgcaaccaagatgcaggtgataggtgaccagtacgtcaaggtgtacctggagtccttctgcgaggacgtgccctccggcaagctctttatgcacgtcacgctgggctctgacgtggaagaggacctgacgatgacccgcaacccgcaacccttcatgcgcccccacgagcgcaacggctttacggtgttgtgtcccaaaaatatgataatcaaaccgggcaagatctcgcacatcatgctggatgtggcttttacctcacacgagcattttgggctgctgtgtcccaagagcatcccgggcctgagcatctcaggtaacctgttgatgaacgggcagcagatcttcctggaggtacaagccatacgcgagaccgtggaactgcgtcagtacgatcccgtggctgcgctcttctttttcgatatcgacttgctgctgcagcgcgggcctcagtacagcgagcaccccaccttcaccagccagtatcgcatccagggcaagcttgagtaccgacacacctgggaccggcacgacgagggtgccgcccagggcgacgacgacgtctggaccagcggatcggactccgacgaagaactcgtaaccaccgagcgcaagacgccccgcgtcaccggcggcggcgccatggcgggcgcctccacttccgcgggccgcaaacgcaaatcagcatcctcggcgacggcgtgcacgtcgggcgttatgacacgcggccgccttaaggccgagtccaccgtcgcgcccgaagaggacaccgacgaggattccgacaacgaaatccacaatccggccgtgttcacctggccgccctggcaggccggcatcctggcccgcaacctggtgcccatggtggctacggttcagggtcagaatctgaagtaccaggagttcttctgggacgccaacgacatctaccgcatcttcgccgaattggaaggcgtatggcagcccgctgcgcaacccaaacgtcgccgccaccggcaagacgccttgcccgggccatgcatcgcctcgacgcccaaaaagcaccgaggttgatctagacctgatcataatcaagccatatcacatctgtagaggtttacttgctttaaaaaacctccacacctccccctgaacctgaaacataaaatgaatgcaattgttgttgttaacttgtttattgcagcttataatggttacaaataaagcaatagcatcacaaatttcacaaataaagcatttttttcactgcattctagttgtggtttgtccaaactcatcaatgtatcttatcatgtctggatctgcggatcaggattggtgacagaaaagccccatccttaggcctcctccttcctagtctcctgatattgggtctaacccccacctcctgttaggcagattccttatctggtgacacacccccatttcctggagccatctctctccttgccagaacctctaaggtttgcttacgatggagccagagaggatcctgggagggagagcttggcagggggtgggagggaagggggggatgcgtgacctgcccggttctcagtggccaccctgcgctaccctctcccagaacctgagctgctctgacgcggctgtctggtgcgtttcactgatcctggtgctgcagcttccttacacttcccaagaggagaagcagtttggaaaaacaaaatcagaataagttggtcctgagttctaactttggctcttcacctttctagtccccaatttatattgttcctccgtgcgtcagttttacctgtgagataaggccagtagccagccccgtcctggcagggctgtggtgaggaggggggtgtccgtgtggaaaactccctttgtgagaatggtgcgtcctcgagctgggcctcatgggccttccgctcactgcccgctttccagtcgggaaacctgtcgtgccagctgcattaacatggtcatagctgtttccttgcgtattgggcgctctccgcttcctcgctcactgactcgctgcgctcggtcgttcgggtaaagcctggggtgcctaatgagcaaaaggccagcaaaaggccaggaaccgtaaaaaggccgcgttgctggcgtttttccataggctccgcccccctgacgagcatcacaaaaatcgacgctcaagtcagaggtggcgaaacccgacaggactataaagataccaggcgtttccccctggaagctccctcgtgcgctctcctgttccgaccctgccgcttaccggatacctgtccgcctttctcccttcgggaagcgtggcgctttctcatagctcacgctgtaggtatctcagttcggtgtaggtcgttcgctccaagctgggctgtgtgcacgaaccccccgttcagcccgaccgctgcgccttatccggtaactatcgtcttgagtccaacccggtaagacacgacttatcgccactggcagcagccactggtaacaggattagcagagcgaggtatgtaggcggtgctacagagttcttgaagtggtggcctaactacggctacactagaagaacagtatttggtatctgcgctctgctgaagccagttaccttcggaaaaagagttggtagctcttgatccggcaaacaaaccaccgctggtagcggtggtttttttgtttgcaagcagcagattacgcgcagaaaaaaaggatctcaagaagatcctttgatcttttctacggggtctgacgctcagtggaacgaaaactcacgttaagggattttggtcatgagattatcaaaaaggatcttcacctagatccttttaaattaaaaatgaagttttaaatcaatctaaagtatatatgagtaaacttggtctgacagttaccaatgcttaatcagtgaggcacctatctcagcgatctgtctatttcgttcatccatagttgcctgactccccgtcgtgtagataactacgatacgggagggcttaccatctggccccagtgctgcaatgataccgcgagaaccacgctcaccggctccagatttatcagcaataaaccagccagccggaagggccgagcgcagaagtggtcctgcaactttatccgcctccatccagtctattaattgttgccgggaagctagagtaagtagttcgccagttaatagtttgcgcaacgttgttgccattgctacaggcatcgtggtgtcacgctcgtcgtttggtatggcttcattcagctccggttcccaacgatcaaggcgagttacatgatcccccatgttgtgcaaaaaagcggttagctccttcggtcctccgatcgttgtcagaagtaagttggccgcagtgttatcactcatggttatggcagcactgcataattctcttactgtcatgccatccgtaagatgcttttctgtgactggtgagtactcaaccaagtcattctgagaatagtgtatgcggcgaccgagttgctcttgcccggcgtcaatacgggataataccgcgccacatagcagaactttaaaagtgctcatcattggaaaacgttcttcggggcgaaaactctcaaggatcttaccgctgttgagatccagttcgatgtaacccactcgtgcacccaactgatcttcagcatcttttactttcaccagcgtttctgggtgagcaaaaacaggaaggcaaaatgccgcaaaaaagggaataagggcgacacggaaatgttgaatactcatactcttcctttttcaatattattgaagcatttatcagggttattgtctcatgagcggatacatatttgaatgtatttagaaaaataaacaaataggggttccgcgcacatttccccgaaaagtgccac

SEQ ID NO: 14 - DNA, 7062 bp, Artificial Sequence
  AAVS1-l_GFP_HCMVpp65 AIN vector V1.H.1
ctaaattgtaagcgttaatattttgttaaaattcgcgttaaatttttgttaaatcagctcattttttaaccaataggccgaaatcggcaaaatcccttataaatcaaaagaatagaccgagatagggttgagtggccgctacagggcgctcccattcgccattcaggctgcgcaactgttgggaagggcgtttcggtgcgggcctcttcgctattacgccagctggcgaaagggggatgtgctgcaaggcgattaagttgggtaacgccagggttttcccagtcacgacgttgtaaaacgacggccagtgagcgcgacgtaatacgactcactatagggcgaattggcggaaggccgtcaaggccgcatgaattgagctctactggcttctgcgccgcctctggcccactgtttccccttcccaggcaggtcctgctttctctgacctgcattctctcccctgggcctgtgccgctttctgtctgcagcttgtggcctgggtcacctctacggctggcccagatccttccctgccgcctccttcaggttccgtcttcctccactccctcttccccttgctctctgctgtgttgctgcccaaggatgctctttccggagcacttccttctcggcgctgcaccacgtgatgtcctctgagcggatcctccccgtgtctgggtcctctccgggcatctctcctccctcacccaaccccatgccgtcttcactcgctgggttcccttttccttctccttctggggcctgtgccatctctcgtttcttaggatggccttctccgacggatgtctcccttgcgtcccgcctccccttcttgtaggcctgcatcatcaccgtttttctggacaaccccaaagtaccccgtctccctggctttagccacctctccatcctcttgctttctttgcctggacaccccgttctcctgtggattcgggtcacctctcactcctttcatttgggcagctcccctaccccccttacctctctagtctgtgctagctcttccagccccctgtcatggcatcttccaggggtccgagagctcagctagtcttcttcctccaacccgggcccctatgtccacttcaggacagcatgtttgctgcctccagggatcctgtgtccccgagctgggaccaccttatattcccagggccggttaatgtggctctggttctgggtacttttatctgtcccctccaccggtatagtaatcaattacggggtcattagttcatagcccatatatggagttccgcgttacataacttacggtaaatggcccgcctggctgaccgcccaacgacccccgcccattgacgtcaataatgacgtatgttcccatagtaacgccaatagggactttccattgacgtcaatgggtggagtatttacggtaaactgcccacttggcagtacatcaagtgtatcatatgccaagtacgccccctattgacgtcaatgacggtaaatggcccgcctggcattatgcccagtacatgaccttatgggactttcctacttggcagtacatctacgtattagtcatcgctattaccatggtgatgcggttttggcagtacatcaatgggcgtggatagcggtttgactcacggggatttccaagtctccaccccattgacgtcaatgggagtttgttttggcaccaaaatcaacgggactttccaaaatgtcgtaacaactccgccccattgacgcaaatgggcggtaggcgtgtacggtgggaggtctatataagcagagctggtttagtgaaccgtcagatcaggtaccgccaccatggaatccgatgagtctggcctgcccgccatggaaatcgagtgcagaatcaccggcaccctgaacggcgtggaatttgagctcgtgggcggaggcgagggcacacctgaacagggcagaatgaccaacaagatgaagtccaccaagggggccctgaccttcagcccctacctgctgtctcacgtgatgggctacggcttctaccacttcggcacctaccccagcggctacgagaaccctttcctgcacgccatcaacaacggcggctacaccaacacccggatcgagaagtacgaggacggcggcgtgctgcacgtgtccttcagctacagatacgaggccggcagagtgatcggcgacttcaaagtgatgggcaccggattccccgaggacagcgtgatcttcaccgacaagatcatccggtccaacgccaccgtggaacatctgcaccccatgggcgacaacgacctggacggcagcttcaccagaaccttctccctgcgggatggcggctactacagcagcgtggtggacagccacatgcacttcaagagcgccatccaccccagcatcctccagaacggcggacccatgttcgccttcagacgggtggaagaggaccacagcaacaccgagctgggcatcgtggaataccagcacgccttcaagacccccgatgccgatgccggcgaggaaggcagtggagagggcagaggaagtctgctaacatgtggtgacgtcgaggagaatcctggcccaatggagtcgcgcggtcgccgttgtcccgaaatgatatccgtactgggtcccatttcggggcacgtgctgaaagccgtgtttagtcgcggcgatacgccggtgctgccgcacgagacgcgactcctgcagacgggtatccacgtacgcgtgagccagccctcgctgatcttggtatcgcagtacacgcccgactcgacgccatgccaccgcggcgacaatcagctgcaggtgcagcacacgtactttacgggcagcgaggtggagaacgtgtcggtcaacgtgcacaaccccacgggccgaagcatctgccccagccaggagcccatgtcgatctatgtgtacgcgctgccgctcaagatgctgaacatccccagcatcaacgtgcaccactacccgtcggcggccgagcgcaaacaccgacacctgcccgtagctgacgctgtgattcacgcgtcgggcaagcagatgtggcaggcgcgtctcacggtctcgggactggcctggacgcgtcagcagaaccagtggaaagagcccgacgtctactacacgtcagcgttcgtgtttcccaccaaggacgtggcactgcggcacgtggtgtgcgcgcacgagctggtttgctccatggagaacacgcgcgcaaccaagatgcaggtgataggtgaccagtacgtcaaggtgtacctggagtccttctgcgaggacgtgccctccggcaagctctttatgcacgtcacgctgggctctgacgtggaagaggacctgacgatgacccgcaacccgcaacccttcatgcgcccccacgagcgcaacggctttacggtgttgtgtcccaaaaatatgataatcaaaccgggcaagatctcgcacatcatgctggatgtggcttttacctcacacgagcattttgggctgctgtgtcccaagagcatcccgggcctgagcatctcaggtaacctgttgatgaacgggcagcagatcttcctggaggtacaagccatacgcgagaccgtggaactgcgtcagtacgatcccgtggctgcgctcttctttttcgatatcgacttgctgctgcagcgcgggcctcagtacagcgagcaccccaccttcaccagccagtatcgcatccagggcaagcttgagtaccgacacacctgggaccggcacgacgagggtgccgcccagggcgacgacgacgtctggaccagcggatcggactccgacgaagaactcgtaaccaccgagcgcaagacgccccgcgtcaccggcggcggcgccatggcgggcgcctccacttccgcgggccgcaaacgcaaatcagcatcctcggcgacggcgtgcacgtcgggcgttatgacacgcggccgccttaaggccgagtccaccgtcgcgcccgaagaggacaccgacgaggattccgacaacgaaatccacaatccggccgtgttcacctggccgccctggcaggccggcatcctggcccgcaacctggtggcaattaatgctacggttcagggtcagaatctgaagtaccaggagttcttctgggacgccaacgacatctaccgcatcttcgccgaattggaaggcgtatggcagcccgctgcgcaacccaaacgtcgccgccaccggcaagacgccttgcccgggccatgcatcgcctcgacgcccaaaaagcaccgaggttgatctagacctgatcataatcaagccatatcacatctgtagaggtttacttgctttaaaaaacctccacacctccccctgaacctgaaacataaaatgaatgcaattgttgttgttaacttgtttattgcagcttataatggttacaaataaagcaatagcatcacaaatttcacaaataaagcatttttttcactgcattctagttgtggtttgtccaaactcatcaatgtatcttatcatgtctggatctgcggatcaggattggtgacagaaaagccccatccttaggcctcctccttcctagtctcctgatattgggtctaacccccacctcctgttaggcagattccttatctggtgacacacccccatttcctggagccatctctctccttgccagaacctctaaggtttgcttacgatggagccagagaggatcctgggagggagagcttggcagggggtgggagggaagggggggatgcgtgacctgcccggttctcagtggccaccctgcgctaccctctcccagaacctgagctgctctgacgcggctgtctggtgcgtttcactgatcctggtgctgcagcttccttacacttcccaagaggagaagcagtttggaaaaacaaaatcagaataagttggtcctgagttctaactttggctcttcacctttctagtccccaatttatattgttcctccgtgcgtcagttttacctgtgagataaggccagtagccagccccgtcctggcagggctgtggtgaggaggggggtgtccgtgtggaaaactccctttgtgagaatggtgcgtcctcgagctgggcctcatgggccttccgctcactgcccgctttccagtcgggaaacctgtcgtgccagctgcattaacatggtcatagctgtttccttgcgtattgggcgctctccgcttcctcgctcactgactcgctgcgctcggtcgttcgggtaaagcctggggtgcctaatgagcaaaaggccagcaaaaggccaggaaccgtaaaaaggccgcgttgctggcgtttttccataggctccgcccccctgacgagcatcacaaaaatcgacgctcaagtcagaggtggcgaaacccgacaggactataaagataccaggcgtttccccctggaagctccctcgtgcgctctcctgttccgaccctgccgcttaccggatacctgtccgcctttctcccttcgggaagcgtggcgctttctcatagctcacgctgtaggtatctcagttcggtgtaggtcgttcgctccaagctgggctgtgtgcacgaaccccccgttcagcccgaccgctgcgccttatccggtaactatcgtcttgagtccaacccggtaagacacgacttatcgccactggcagcagccactggtaacaggattagcagagcgaggtatgtaggcggtgctacagagttcttgaagtggtggcctaactacggctacactagaagaacagtatttggtatctgcgctctgctgaagccagttaccttcggaaaaagagttggtagctcttgatccggcaaacaaaccaccgctggtagcggtggtttttttgtttgcaagcagcagattacgcgcagaaaaaaaggatctcaagaagatcctttgatcttttctacggggtctgacgctcagtggaacgaaaactcacgttaagggattttggtcatgagattatcaaaaaggatcttcacctagatccttttaaattaaaaatgaagttttaaatcaatctaaagtatatatgagtaaacttggtctgacagttaccaatgcttaatcagtgaggcacctatctcagcgatctgtctatttcgttcatccatagttgcctgactccccgtcgtgtagataactacgatacgggagggcttaccatctggccccagtgctgcaatgataccgcgagaaccacgctcaccggctccagatttatcagcaataaaccagccagccggaagggccgagcgcagaagtggtcctgcaactttatccgcctccatccagtctattaattgttgccgggaagctagagtaagtagttcgccagttaatagtttgcgcaacgttgttgccattgctacaggcatcgtggtgtcacgctcgtcgtttggtatggcttcattcagctccggttcccaacgatcaaggcgagttacatgatcccccatgttgtgcaaaaaagcggttagctccttcggtcctccgatcgttgtcagaagtaagttggccgcagtgttatcactcatggttatggcagcactgcataattctcttactgtcatgccatccgtaagatgcttttctgtgactggtgagtactcaaccaagtcattctgagaatagtgtatgcggcgaccgagttgctcttgcccggcgtcaatacgggataataccgcgccacatagcagaactttaaaagtgctcatcattggaaaacgttcttcggggcgaaaactctcaaggatcttaccgctgttgagatccagttcgatgtaacccactcgtgcacccaactgatcttcagcatcttttactttcaccagcgtttctgggtgagcaaaaacaggaaggcaaaatgccgcaaaaaagggaataagggcgacacggaaatgttgaatactcatactcttcctttttcaatattattgaagcatttatcagggttattgtctcatgagcggatacatatttgaatgtatttagaaaaataaacaaataggggttccgcgcacatttccccgaaaagtgccac

SEQ ID NO: 15 - DNA, 6348 bp, Artificial Sequence
  AAVS1_DRA_Flag-DRB1_6xHis vector V1.I.5
ctaaattgtaagcgttaatattttgttaaaattcgcgttaaatttttgttaaatcagctcattttttaaccaataggccgaaatcggcaaaatcccttataaatcaaaagaatagaccgagatagggttgagtggccgctacagggcgctcccattcgccattcaggctgcgcaactgttgggaagggcgtttcggtgcgggcctcttcgctattacgccagctggcgaaagggggatgtgctgcaaggcgattaagttgggtaacgccagggttttcccagtcacgacgttgtaaaacgacggccagtgagcgcgacgtaatacgactcactatagggcgaattggcggaaggccgtcaaggccgcatgaattgagctctactggcttctgcgccgcctctggcccactgtttccccttcccaggcaggtcctgctttctctgacctgcattctctcccctgggcctgtgccgctttctgtctgcagcttgtggcctgggtcacctctacggctggcccagatccttccctgccgcctccttcaggttccgtcttcctccactccctcttccccttgctctctgctgtgttgctgcccaaggatgctctttccggagcacttccttctcggcgctgcaccacgtgatgtcctctgagcggatcctccccgtgtctgggtcctctccgggcatctctcctccctcacccaaccccatgccgtcttcactcgctgggttcccttttccttctccttctggggcctgtgccatctctcgtttcttaggatggccttctccgacggatgtctcccttgcgtcccgcctccccttcttgtaggcctgcatcatcaccgtttttctggacaaccccaaagtaccccgtctccctggctttagccacctctccatcctcttgctttctttgcctggacaccccgttctcctgtggattcgggtcacctctcactcctttcatttgggcagctcccctaccccccttacctctctagtctgtgctagctcttccagccccctgtcatggcatcttccaggggtccgagagctcagctagtcttcttcctccaacccgggcccctatgtccacttcaggacagcatgtttgctgcctccagggatcctgtgtccccgagctgggaccaccttatattcccagggccggttaatgtggctctggttctgggtacttttatctgtcccctccaccggtatagtaatcaattacggggtcattagttcatagcccatatatggagttccgcgttacataacttacggtaaatggcccgcctggctgaccgcccaacgacccccgcccattgacgtcaataatgacgtatgttcccatagtaacgccaatagggactttccattgacgtcaatgggtggagtatttacggtaaactgcccacttggcagtacatcaagtgtatcatatgccaagtacgccccctattgacgtcaatgacggtaaatggcccgcctggcattatgcccagtacatgaccttatgggactttcctacttggcagtacatctacgtattagtcatcgctattaccatggtgatgcggttttggcagtacatcaatgggcgtggatagcggtttgactcacggggatttccaagtctccaccccattgacgtcaatgggagtttgttttggcaccaaaatcaacgggactttccaaaatgtcgtaacaactccgccccattgacgcaaatgggcggtaggcgtgtacggtgggaggtctatataagcagagctggtttagtgaaccgtcagatcaggtaccatggccataagtggagtccctgtgctaggatttttcatcatagctgtgctgatgagcgctcaggaatcatgggctatcaaagaagaacatgtgatcatccaggccgagttctatctgaatcctgaccaatcaggcgagtttatgtttgactttgatggtgatgagattttccatgtggatatggcaaagaaggagacggtctggcggcttgaagaatttggacgatttgccagctttgaggctcaaggtgcattggccaacatagctgtggacaaagccaacctggaaatcatgacaaagcgctccaactatactccgatcaccaatgtacctccagaggtaactgtgctcacgaacagccctgtggaactgagagagcccaacgtcctcatctgtttcatcgacaagttcaccccaccagtggtcaatgtcacgtggcttcgaaatggaaaacctgtcaccacaggagtgtcagagacagtctttctgcccagggaagatcaccttttccgcaagttccactatctccccttcctgccctcaactgaggacgtttacgactgcagggtggagcactggggcttggatgagcctcttctcaagcactgggagtttgatgctccaagccctctcccagagactacagagaacgtggtgtgtgccctgggcctgactgtgggtctggtgggcatcattattgggaccatcttcatcatcaagggagtgcgcaaaagcaatgcagcagaacgcagaggacctctgcccgggatggactataaggaccacgacggagactacaaggatcatgatattgattacaaagacgatgacgataagggatccggagccacgaacttctctctgttaaagcaagcaggagacgtggaagagaaccctggtcctatggtgtgtctgaagctccctggaggctcctgcatgacagcgctgacagtgacactgatggtgctgagctccccactggctttggctggggacacccgaccacgtttcttgtggcagcttaagttcgaatgtcatttcttcaatgggacggagagagtgcggttgctggaaagatgcatctataaccaagaggagtccgtgcgcttcgacagcgacgtgggggagtaccgggctgtgacggagctgggaaggcctgatgccgagtactggaacagccagaaggacctcctggagcagaggagagccgctgtggacacctactgcagacacaactacggggttggtgagagcttcacagtgcagcggcgagttgagcctaaggtgactgtgtatccttcaaagacccagcccctgcagcaccacaacctcctggtctgctctgtgagtggtttctatccaggcagcattgaagtcaggtggttccggaacggccaggaagagaaggctggggtggtgtccacaggcctgatccagaatggagattggaccttccagaccctggtgatgctggaaacagttcctcggagtggagaggtttacacctgccaagtggagcacccaagtgtgacgagccctctcacagtggaatggagagcacggtctgaatctgcacagagcaagatgctgagtggagtcgggggcttcgtgctgggcctgctcttccttggggccgggctgttcatctacttcaggaatcagaaaggacactctggacttcagccaacaggattcctgagccccgggcatcatcaccatcaccactgactatagtcgtctagacctgatcataatcaagccatatcacatctgtagaggtttacttgctttaaaaaacctccacacctccccctgaacctgaaacataaaatgaatgcaattgttgttgttaacttgtttattgcagcttataatggttacaaataaagcaatagcatcacaaatttcacaaataaagcatttttttcactgcattctagttgtggtttgtccaaactcatcaatgtatcttatcatgtctggatctgcggatcaggattggtgacagaaaagccccatccttaggcctcctccttcctagtctcctgatattgggtctaacccccacctcctgttaggcagattccttatctggtgacacacccccatttcctggagccatctctctccttgccagaacctctaaggtttgcttacgatggagccagagaggatcctgggagggagagcttggcagggggtgggagggaagggggggatgcgtgacctgcccggttctcagtggccaccctgcgctaccctctcccagaacctgagctgctctgacgcggctgtctggtgcgtttcactgatcctggtgctgcagcttccttacacttcccaagaggagaagcagtttggaaaaacaaaatcagaataagttggtcctgagttctaactttggctcttcacctttctagtccccaatttatattgttcctccgtgcgtcagttttacctgtgagataaggccagtagccagccccgtcctggcagggctgtggtgaggaggggggtgtccgtgtggaaaactccctttgtgagaatggtgcgtcctcgagctgggcctcatgggccttccgctcactgcccgctttccagtcgggaaacctgtcgtgccagctgcattaacatggtcatagctgtttccttgcgtattgggcgctctccgcttcctcgctcactgactcgctgcgctcggtcgttcgggtaaagcctggggtgcctaatgagcaaaaggccagcaaaaggccaggaaccgtaaaaaggccgcgttgctggcgtttttccataggctccgcccccctgacgagcatcacaaaaatcgacgctcaagtcagaggtggcgaaacccgacaggactataaagataccaggcgtttccccctggaagctccctcgtgcgctctcctgttccgaccctgccgcttaccggatacctgtccgcctttctcccttcgggaagcgtggcgctttctcatagctcacgctgtaggtatctcagttcggtgtaggtcgttcgctccaagctgggctgtgtgcacgaaccccccgttcagcccgaccgctgcgccttatccggtaactatcgtcttgagtccaacccggtaagacacgacttatcgccactggcagcagccactggtaacaggattagcagagcgaggtatgtaggcggtgctacagagttcttgaagtggtggcctaactacggctacactagaagaacagtatttggtatctgcgctctgctgaagccagttaccttcggaaaaagagttggtagctcttgatccggcaaacaaaccaccgctggtagcggtggtttttttgtttgcaagcagcagattacgcgcagaaaaaaaggatctcaagaagatcctttgatcttttctacggggtctgacgctcagtggaacgaaaactcacgttaagggattttggtcatgagattatcaaaaaggatcttcacctagatccttttaaattaaaaatgaagttttaaatcaatctaaagtatatatgagtaaacttggtctgacagttaccaatgcttaatcagtgaggcacctatctcagcgatctgtctatttcgttcatccatagttgcctgactccccgtcgtgtagataactacgatacgggagggcttaccatctggccccagtgctgcaatgataccgcgagaaccacgctcaccggctccagatttatcagcaataaaccagccagccggaagggccgagcgcagaagtggtcctgcaactttatccgcctccatccagtctattaattgttgccgggaagctagagtaagtagttcgccagttaatagtttgcgcaacgttgttgccattgctacaggcatcgtggtgtcacgctcgtcgtttggtatggcttcattcagctccggttcccaacgatcaaggcgagttacatgatcccccatgttgtgcaaaaaagcggttagctccttcggtcctccgatcgttgtcagaagtaagttggccgcagtgttatcactcatggttatggcagcactgcataattctcttactgtcatgccatccgtaagatgcttttctgtgactggtgagtactcaaccaagtcattctgagaatagtgtatgcggcgaccgagttgctcttgcccggcgtcaatacgggataataccgcgccacatagcagaactttaaaagtgctcatcattggaaaacgttcttcggggcgaaaactctcaaggatcttaccgctgttgagatccagttcgatgtaacccactcgtgcacccaactgatcttcagcatcttttactttcaccagcgtttctgggtgagcaaaaacaggaaggcaaaatgccgcaaaaaagggaataagggcgacacggaaatgttgaatactcatactcttcctttttcaatattattgaagcatttatcagggttattgtctcatgagcggatacatatttgaatgtatttagaaaaataaacaaataggggttccgcgcacatttccccgaaaagtgccac

SEQ ID NO: 16 - DNA, 6342 bp, Artificial Sequence
  AAVS1_DPA1_Flag-DPB1_6xHis vector V1.I.7
ctaaattgtaagcgttaatattttgttaaaattcgcgttaaatttttgttaaatcagctcattttttaaccaataggccgaaatcggcaaaatcccttataaatcaaaagaatagaccgagatagggttgagtggccgctacagggcgctcccattcgccattcaggctgcgcaactgttgggaagggcgtttcggtgcgggcctcttcgctattacgccagctggcgaaagggggatgtgctgcaaggcgattaagttgggtaacgccagggttttcccagtcacgacgttgtaaaacgacggccagtgagcgcgacgtaatacgactcactatagggcgaattggcggaaggccgtcaaggccgcatgaattgagctctactggcttctgcgccgcctctggcccactgtttccccttcccaggcaggtcctgctttctctgacctgcattctctcccctgggcctgtgccgctttctgtctgcagcttgtggcctgggtcacctctacggctggcccagatccttccctgccgcctccttcaggttccgtcttcctccactccctcttccccttgctctctgctgtgttgctgcccaaggatgctctttccggagcacttccttctcggcgctgcaccacgtgatgtcctctgagcggatcctccccgtgtctgggtcctctccgggcatctctcctccctcacccaaccccatgccgtcttcactcgctgggttcccttttccttctccttctggggcctgtgccatctctcgtttcttaggatggccttctccgacggatgtctcccttgcgtcccgcctccccttcttgtaggcctgcatcatcaccgtttttctggacaaccccaaagtaccccgtctccctggctttagccacctctccatcctcttgctttctttgcctggacaccccgttctcctgtggattcgggtcacctctcactcctttcatttgggcagctcccctaccccccttacctctctagtctgtgctagctcttccagccccctgtcatggcatcttccaggggtccgagagctcagctagtcttcttcctccaacccgggcccctatgtccacttcaggacagcatgtttgctgcctccagggatcctgtgtccccgagctgggaccaccttatattcccagggccggttaatgtggctctggttctgggtacttttatctgtcccctccaccggtatagtaatcaattacggggtcattagttcatagcccatatatggagttccgcgttacataacttacggtaaatggcccgcctggctgaccgcccaacgacccccgcccattgacgtcaataatgacgtatgttcccatagtaacgccaatagggactttccattgacgtcaatgggtggagtatttacggtaaactgcccacttggcagtacatcaagtgtatcatatgccaagtacgccccctattgacgtcaatgacggtaaatggcccgcctggcattatgcccagtacatgaccttatgggactttcctacttggcagtacatctacgtattagtcatcgctattaccatggtgatgcggttttggcagtacatcaatgggcgtggatagcggtttgactcacggggatttccaagtctccaccccattgacgtcaatgggagtttgttttggcaccaaaatcaacgggactttccaaaatgtcgtaacaactccgccccattgacgcaaatgggcggtaggcgtgtacggtgggaggtctatataagcagagctggtttagtgaaccgtcagatcaggtaccatgcgccctgaggacagaatgttccatatcagagctgtgatcttgagagccctctccttggctttcctgctgagtctccgaggagctggggccatcaaggcggaccatgtgtcaacttatgccgcgtttgtacagacgcatagaccaacaggggagtttatgtttgaatttgatgaagatgagatgttctatgtggatctggacaagaaggagaccgtctggcatctggaggagtttggccaagccttttcctttgaggctcagggcgggctggctaacattgctatattgaacaacaacttgaataccttgatccagcgttccaaccacactcaggccaccaacgatccccctgaggtgaccgtgtttcccaaggagcctgtggagctgggccagcccaacaccctcatctgccacattgacaagttcttcccaccagtgctcaacgtcacgtggctgtgcaacggggagctggtcactgagggtgtcgctgagagcctcttcctgcccagaacagattacagcttccacaagttccattacctgacctttgtgccctcagcagaggacttctatgactgcagggtggagcactggggcttggaccagccgctcctcaagcactgggaggcccaagagccaatccagatgcctgagacaacggagactgtgctctgtgccctgggcctggtgctgggcctagtcggcatcatcgtgggcaccgtcctcatcataaagtctctgcgttctggccatgaccctagagcccagggaaccctgcccgggatggactataaggaccacgacggagactacaaggatcatgatattgattacaaagacgatgacgataagggatccggagccacgaacttctctctgttaaagcaagcaggagacgtggaagagaaccctggtcctatgatggttctgcaggtttctgcggccccccggacagtggctctgacggcgttactgatggtgctgctcacatctgtggtccagggcagggccactccagagaattaccttttccagggacggcaggaatgctacgcgtttaatgggacacagcgcttcctggagagatacatctacaaccgggaggagttcgcgcgcttcgacagcgacgtgggggagttccgggcggtgacggagctggggcggcctgctgcggagtactggaacagccagaaggacatcctggaggagaagcgggcagtgccggacaggatgtgcagacacaactacgagctgggcgggcccatgaccctgcagcgccgagtccagcctagggtgaatgtttccccctccaagaaggggcccttgcagcaccacaacctgcttgtctgccacgtgacggatttctacccaggcagcattcaagtccgatggttcctgaatggacaggaggaaacagctggggtcgtgtccaccaacctgatccgtaatggagactggaccttccagatcctggtgatgctggaaatgaccccccagcagggagatgtctacacctgccaagtggagcacaccagcctggatagtcctgtcaccgtggagtggaaggcacagtctgattctgcccggagtaagacattgacgggagctgggggcttcgtgctggggctcatcatctgtggagtgggcatcttcatgcacaggaggagcaagaaagttcaacgaggatctgcacccgggcatcatcaccatcaccactgactatagtcgtctagacctgatcataatcaagccatatcacatctgtagaggtttacttgctttaaaaaacctccacacctccccctgaacctgaaacataaaatgaatgcaattgttgttgttaacttgtttattgcagcttataatggttacaaataaagcaatagcatcacaaatttcacaaataaagcatttttttcactgcattctagttgtggtttgtccaaactcatcaatgtatcttatcatgtctggatctgcggatcaggattggtgacagaaaagccccatccttaggcctcctccttcctagtctcctgatattgggtctaacccccacctcctgttaggcagattccttatctggtgacacacccccatttcctggagccatctctctccttgccagaacctctaaggtttgcttacgatggagccagagaggatcctgggagggagagcttggcagggggtgggagggaagggggggatgcgtgacctgcccggttctcagtggccaccctgcgctaccctctcccagaacctgagctgctctgacgcggctgtctggtgcgtttcactgatcctggtgctgcagcttccttacacttcccaagaggagaagcagtttggaaaaacaaaatcagaataagttggtcctgagttctaactttggctcttcacctttctagtccccaatttatattgttcctccgtgcgtcagttttacctgtgagataaggccagtagccagccccgtcctggcagggctgtggtgaggaggggggtgtccgtgtggaaaactccctttgtgagaatggtgcgtcctcgagctgggcctcatgggccttccgctcactgcccgctttccagtcgggaaacctgtcgtgccagctgcattaacatggtcatagctgtttccttgcgtattgggcgctctccgcttcctcgctcactgactcgctgcgctcggtcgttcgggtaaagcctggggtgcctaatgagcaaaaggccagcaaaaggccaggaaccgtaaaaaggccgcgttgctggcgtttttccataggctccgcccccctgacgagcatcacaaaaatcgacgctcaagtcagaggtggcgaaacccgacaggactataaagataccaggcgtttccccctggaagctccctcgtgcgctctcctgttccgaccctgccgcttaccggatacctgtccgcctttctcccttcgggaagcgtggcgctttctcatagctcacgctgtaggtatctcagttcggtgtaggtcgttcgctccaagctgggctgtgtgcacgaaccccccgttcagcccgaccgctgcgccttatccggtaactatcgtcttgagtccaacccggtaagacacgacttatcgccactggcagcagccactggtaacaggattagcagagcgaggtatgtaggcggtgctacagagttcttgaagtggtggcctaactacggctacactagaagaacagtatttggtatctgcgctctgctgaagccagttaccttcggaaaaagagttggtagctcttgatccggcaaacaaaccaccgctggtagcggtggtttttttgtttgcaagcagcagattacgcgcagaaaaaaaggatctcaagaagatcctttgatcttttctacggggtctgacgctcagtggaacgaaaactcacgttaagggattttggtcatgagattatcaaaaaggatcttcacctagatccttttaaattaaaaatgaagttttaaatcaatctaaagtatatatgagtaaacttggtctgacagttaccaatgcttaatcagtgaggcacctatctcagcgatctgtctatttcgttcatccatagttgcctgactccccgtcgtgtagataactacgatacgggagggcttaccatctggccccagtgctgcaatgataccgcgagaaccacgctcaccggctccagatttatcagcaataaaccagccagccggaagggccgagcgcagaagtggtcctgcaactttatccgcctccatccagtctattaattgttgccgggaagctagagtaagtagttcgccagttaatagtttgcgcaacgttgttgccattgctacaggcatcgtggtgtcacgctcgtcgtttggtatggcttcattcagctccggttcccaacgatcaaggcgagttacatgatcccccatgttgtgcaaaaaagcggttagctccttcggtcctccgatcgttgtcagaagtaagttggccgcagtgttatcactcatggttatggcagcactgcataattctcttactgtcatgccatccgtaagatgcttttctgtgactggtgagtactcaaccaagtcattctgagaatagtgtatgcggcgaccgagttgctcttgcccggcgtcaatacgggataataccgcgccacatagcagaactttaaaagtgctcatcattggaaaacgttcttcggggcgaaaactctcaaggatcttaccgctgttgagatccagttcgatgtaacccactcgtgcacccaactgatcttcagcatcttttactttcaccagcgtttctgggtgagcaaaaacaggaaggcaaaatgccgcaaaaaagggaataagggcgacacggaaatgttgaatactcatactcttcctttttcaatattattgaagcatttatcagggttattgtctcatgagcggatacatatttgaatgtatttagaaaaataaacaaataggggttccgcgcacatttccccgaaaagtgccac

SEQ ID NO: 17 - DNA, 2762 bp, Artificial Sequence
  HLA-A-sg-sp-opti1 vector V2.A.1
ctaaattgtaagcgttaatattttgttaaaattcgcgttaaatttttgttaaatcagctcattttttaaccaataggccgaaatcggcaaaatcccttataaatcaaaagaatagaccgagatagggttgagtggccgctacagggcgctcccattcgccattcaggctgcgcaactgttgggaagggcgtttcggtgcgggcctcttcgctattacgccagctggcgaaagggggatgtgctgcaaggcgattaagttgggtaacgccagggttttcccagtcacgacgttgtaaaacgacggccagtgagcgcgacgtaatacgactcactatagggcgaattggcggaaggccgtcaaggccgcatggatccaaggtcgggcaggaagagggcctatttcccatgattccttcatatttgcatatacgatacaaggctgttagagagataattagaattaatttgactgtaaacacaaagatattagtacaaaatacgtgacgtagaaagtaataatttcttgggtagtttgcagttttaaaattatgttttaaaatggactatcatatgcttaccgtaacttgaaagtatttcgatttcttggctttatatatcttgtggaaaggacgaaacaccgagggttcggggcgccatgagtttaagagctatgctggaaacagcatagcaagtttaaataaggctagtccgttatcaacttgaaaaagtggcaccgagtcggtgctttttttcagacatccatagatctagctcgagttttttttctagactgggcctcatgggccttccgctcactgcccgctttccagtcgggaaacctgtcgtgccagctgcattaacatggtcatagctgtttccttgcgtattgggcgctctccgcttcctcgctcactgactcgctgcgctcggtcgttcgggtaaagcctggggtgcctaatgagcaaaaggccagcaaaaggccaggaaccgtaaaaaggccgcgttgctggcgtttttccataggctccgcccccctgacgagcatcacaaaaatcgacgctcaagtcagaggtggcgaaacccgacaggactataaagataccaggcgtttccccctggaagctccctcgtgcgctctcctgttccgaccctgccgcttaccggatacctgtccgcctttctcccttcgggaagcgtggcgctttctcatagctcacgctgtaggtatctcagttcggtgtaggtcgttcgctccaagctgggctgtgtgcacgaaccccccgttcagcccgaccgctgcgccttatccggtaactatcgtcttgagtccaacccggtaagacacgacttatcgccactggcagcagccactggtaacaggattagcagagcgaggtatgtaggcggtgctacagagttcttgaagtggtggcctaactacggctacactagaagaacagtatttggtatctgcgctctgctgaagccagttaccttcggaaaaagagttggtagctcttgatccggcaaacaaaccaccgctggtagcggtggtttttttgtttgcaagcagcagattacgcgcagaaaaaaaggatctcaagaagatcctttgatcttttctacggggtctgacgctcagtggaacgaaaactcacgttaagggattttggtcatgagattatcaaaaaggatcttcacctagatccttttaaattaaaaatgaagttttaaatcaatctaaagtatatatgagtaaacttggtctgacagttaccaatgcttaatcagtgaggcacctatctcagcgatctgtctatttcgttcatccatagttgcctgactccccgtcgtgtagataactacgatacgggagggcttaccatctggccccagtgctgcaatgataccgcgagaaccacgctcaccggctccagatttatcagcaataaaccagccagccggaagggccgagcgcagaagtggtcctgcaactttatccgcctccatccagtctattaattgttgccgggaagctagagtaagtagttcgccagttaatagtttgcgcaacgttgttgccattgctacaggcatcgtggtgtcacgctcgtcgtttggtatggcttcattcagctccggttcccaacgatcaaggcgagttacatgatcccccatgttgtgcaaaaaagcggttagctccttcggtcctccgatcgttgtcagaagtaagttggccgcagtgttatcactcatggttatggcagcactgcataattctcttactgtcatgccatccgtaagatgcttttctgtgactggtgagtactcaaccaagtcattctgagaatagtgtatgcggcgaccgagttgctcttgcccggcgtcaatacgggataataccgcgccacatagcagaactttaaaagtgctcatcattggaaaacgttcttcggggcgaaaactctcaaggatcttaccgctgttgagatccagttcgatgtaacccactcgtgcacccaactgatcttcagcatcttttactttcaccagcgtttctgggtgagcaaaaacaggaaggcaaaatgccgcaaaaaagggaataagggcgacacggaaatgttgaatactcatactcttcctttttcaatattattgaagcatttatcagggttattgtctcatgagcggatacatatttgaatgtatttagaaaaataaacaaataggggttccgcgcacatttccccgaaaagtgccac

SEQ ID NO: 18 - DNA, 2762 bp, Artificial Sequence
  HLA-B-sg-sp-3 vector V2.A.7
ctaaattgtaagcgttaatattttgttaaaattcgcgttaaatttttgttaaatcagctcattttttaaccaataggccgaaatcggcaaaatcccttataaatcaaaagaatagaccgagatagggttgagtggccgctacagggcgctcccattcgccattcaggctgcgcaactgttgggaagggcgtttcggtgcgggcctcttcgctattacgccagctggcgaaagggggatgtgctgcaaggcgattaagttgggtaacgccagggttttcccagtcacgacgttgtaaaacgacggccagtgagcgcgacgtaatacgactcactatagggcgaattggcggaaggccgtcaaggccgcatggatccaaggtcgggcaggaagagggcctatttcccatgattccttcatatttgcatatacgatacaaggctgttagagagataattagaattaatttgactgtaaacacaaagatattagtacaaaatacgtgacgtagaaagtaataatttcttgggtagtttgcagttttaaaattatgttttaaaatggactatcatatgcttaccgtaacttgaaagtatttcgatttcttggctttatatatcttgtggaaaggacgaaacaccgtagaaatacctcatggagtgtttaagagctatgctggaaacagcatagcaagtttaaataaggctagtccgttatcaacttgaaaaagtggcaccgagtcggtgctttttttcagacatccatagatctagctcgagttttttttctagactgggcctcatgggccttccgctcactgcccgctttccagtcgggaaacctgtcgtgccagctgcattaacatggtcatagctgtttccttgcgtattgggcgctctccgcttcctcgctcactgactcgctgcgctcggtcgttcgggtaaagcctggggtgcctaatgagcaaaaggccagcaaaaggccaggaaccgtaaaaaggccgcgttgctggcgtttttccataggctccgcccccctgacgagcatcacaaaaatcgacgctcaagtcagaggtggcgaaacccgacaggactataaagataccaggcgtttccccctggaagctccctcgtgcgctctcctgttccgaccctgccgcttaccggatacctgtccgcctttctcccttcgggaagcgtggcgctttctcatagctcacgctgtaggtatctcagttcggtgtaggtcgttcgctccaagctgggctgtgtgcacgaaccccccgttcagcccgaccgctgcgccttatccggtaactatcgtcttgagtccaacccggtaagacacgacttatcgccactggcagcagccactggtaacaggattagcagagcgaggtatgtaggcggtgctacagagttcttgaagtggtggcctaactacggctacactagaagaacagtatttggtatctgcgctctgctgaagccagttaccttcggaaaaagagttggtagctcttgatccggcaaacaaaccaccgctggtagcggtggtttttttgtttgcaagcagcagattacgcgcagaaaaaaaggatctcaagaagatcctttgatcttttctacggggtctgacgctcagtggaacgaaaactcacgttaagggattttggtcatgagattatcaaaaaggatcttcacctagatccttttaaattaaaaatgaagttttaaatcaatctaaagtatatatgagtaaacttggtctgacagttaccaatgcttaatcagtgaggcacctatctcagcgatctgtctatttcgttcatccatagttgcctgactccccgtcgtgtagataactacgatacgggagggcttaccatctggccccagtgctgcaatgataccgcgagaaccacgctcaccggctccagatttatcagcaataaaccagccagccggaagggccgagcgcagaagtggtcctgcaactttatccgcctccatccagtctattaattgttgccgggaagctagagtaagtagttcgccagttaatagtttgcgcaacgttgttgccattgctacaggcatcgtggtgtcacgctcgtcgtttggtatggcttcattcagctccggttcccaacgatcaaggcgagttacatgatcccccatgttgtgcaaaaaagcggttagctccttcggtcctccgatcgttgtcagaagtaagttggccgcagtgttatcactcatggttatggcagcactgcataattctcttactgtcatgccatccgtaagatgcttttctgtgactggtgagtactcaaccaagtcattctgagaatagtgtatgcggcgaccgagttgctcttgcccggcgtcaatacgggataataccgcgccacatagcagaactttaaaagtgctcatcattggaaaacgttcttcggggcgaaaactctcaaggatcttaccgctgttgagatccagttcgatgtaacccactcgtgcacccaactgatcttcagcatcttttactttcaccagcgtttctgggtgagcaaaaacaggaaggcaaaatgccgcaaaaaagggaataagggcgacacggaaatgttgaatactcatactcttcctttttcaatattattgaagcatttatcagggttattgtctcatgagcggatacatatttgaatgtatttagaaaaataaacaaataggggttccgcgcacatttccccgaaaagtgccac

SEQ ID NO: 19 - DNA, 2762 bp, Artificial Sequence
  HLA-C-sg-sp-4 vector V2.B.3
ctaaattgtaagcgttaatattttgttaaaattcgcgttaaatttttgttaaatcagctcattttttaaccaataggccgaaatcggcaaaatcccttataaatcaaaagaatagaccgagatagggttgagtggccgctacagggcgctcccattcgccattcaggctgcgcaactgttgggaagggcgtttcggtgcgggcctcttcgctattacgccagctggcgaaagggggatgtgctgcaaggcgattaagttgggtaacgccagggttttcccagtcacgacgttgtaaaacgacggccagtgagcgcgacgtaatacgactcactatagggcgaattggcggaaggccgtcaaggccgcatggatccaaggtcgggcaggaagagggcctatttcccatgattccttcatatttgcatatacgatacaaggctgttagagagataattagaattaatttgactgtaaacacaaagatattagtacaaaatacgtgacgtagaaagtaataatttcttgggtagtttgcagttttaaaattatgttttaaaatggactatcatatgcttaccgtaacttgaaagtatttcgatttcttggctttatatatcttgtggaaaggacgaaacaccggggccggagtattgggaccgtttaagagctatgctggaaacagcatagcaagtttaaataaggctagtccgttatcaacttgaaaaagtggcaccgagtcggtgctttttttcagacatccatagatctagctcgagttttttttctagactgggcctcatgggccttccgctcactgcccgctttccagtcgggaaacctgtcgtgccagctgcattaacatggtcatagctgtttccttgcgtattgggcgctctccgcttcctcgctcactgactcgctgcgctcggtcgttcgggtaaagcctggggtgcctaatgagcaaaaggccagcaaaaggccaggaaccgtaaaaaggccgcgttgctggcgtttttccataggctccgcccccctgacgagcatcacaaaaatcgacgctcaagtcagaggtggcgaaacccgacaggactataaagataccaggcgtttccccctggaagctccctcgtgcgctctcctgttccgaccctgccgcttaccggatacctgtccgcctttctcccttcgggaagcgtggcgctttctcatagctcacgctgtaggtatctcagttcggtgtaggtcgttcgctccaagctgggctgtgtgcacgaaccccccgttcagcccgaccgctgcgccttatccggtaactatcgtcttgagtccaacccggtaagacacgacttatcgccactggcagcagccactggtaacaggattagcagagcgaggtatgtaggcggtgctacagagttcttgaagtggtggcctaactacggctacactagaagaacagtatttggtatctgcgctctgctgaagccagttaccttcggaaaaagagttggtagctcttgatccggcaaacaaaccaccgctggtagcggtggtttttttgtttgcaagcagcagattacgcgcagaaaaaaaggatctcaagaagatcctttgatcttttctacggggtctgacgctcagtggaacgaaaactcacgttaagggattttggtcatgagattatcaaaaaggatcttcacctagatccttttaaattaaaaatgaagttttaaatcaatctaaagtatatatgagtaaacttggtctgacagttaccaatgcttaatcagtgaggcacctatctcagcgatctgtctatttcgttcatccatagttgcctgactccccgtcgtgtagataactacgatacgggagggcttaccatctggccccagtgctgcaatgataccgcgagaaccacgctcaccggctccagatttatcagcaataaaccagccagccggaagggccgagcgcagaagtggtcctgcaactttatccgcctccatccagtctattaattgttgccgggaagctagagtaagtagttcgccagttaatagtttgcgcaacgttgttgccattgctacaggcatcgtggtgtcacgctcgtcgtttggtatggcttcattcagctccggttcccaacgatcaaggcgagttacatgatcccccatgttgtgcaaaaaagcggttagctccttcggtcctccgatcgttgtcagaagtaagttggccgcagtgttatcactcatggttatggcagcactgcataattctcttactgtcatgccatccgtaagatgcttttctgtgactggtgagtactcaaccaagtcattctgagaatagtgtatgcggcgaccgagttgctcttgcccggcgtcaatacgggataataccgcgccacatagcagaactttaaaagtgctcatcattggaaaacgttcttcggggcgaaaactctcaaggatcttaccgctgttgagatccagttcgatgtaacccactcgtgcacccaactgatcttcagcatcttttactttcaccagcgtttctgggtgagcaaaaacaggaaggcaaaatgccgcaaaaaagggaataagggcgacacggaaatgttgaatactcatactcttcctttttcaatattattgaagcatttatcagggttattgtctcatgagcggatacatatttgaatgtatttagaaaaataaacaaataggggttccgcgcacatttccccgaaaagtgccac

SEQ ID NO: 20 - DNA, 2762 bp, Artificial Sequence
  HLA-A-ex2-3_sg-sp-opti_1 vector V2.I.10
ctaaattgtaagcgttaatattttgttaaaattcgcgttaaatttttgttaaatcagctcattttttaaccaataggccgaaatcggcaaaatcccttataaatcaaaagaatagaccgagatagggttgagtggccgctacagggcgctcccattcgccattcaggctgcgcaactgttgggaagggcgtttcggtgcgggcctcttcgctattacgccagctggcgaaagggggatgtgctgcaaggcgattaagttgggtaacgccagggttttcccagtcacgacgttgtaaaacgacggccagtgagcgcgacgtaatacgactcactatagggcgaattggcggaaggccgtcaaggccgcatggatccaaggtcgggcaggaagagggcctatttcccatgattccttcatatttgcatatacgatacaaggctgttagagagataattagaattaatttgactgtaaacacaaagatattagtacaaaatacgtgacgtagaaagtaataatttcttgggtagtttgcagttttaaaattatgttttaaaatggactatcatatgcttaccgtaacttgaaagtatttcgatttcttggctttatatatcttgtggaaaggacgaaacaccgtccccaggctctcactgaagtttaagagctatgctggaaacagcatagcaagtttaaataaggctagtccgttatcaacttgaaaaagtggcaccgagtcggtgctttttttcagacatccatagatctagctcgagttttttttctagactgggcctcatgggccttccgctcactgcccgctttccagtcgggaaacctgtcgtgccagctgcattaacatggtcatagctgtttccttgcgtattgggcgctctccgcttcctcgctcactgactcgctgcgctcggtcgttcgggtaaagcctggggtgcctaatgagcaaaaggccagcaaaaggccaggaaccgtaaaaaggccgcgttgctggcgtttttccataggctccgcccccctgacgagcatcacaaaaatcgacgctcaagtcagaggtggcgaaacccgacaggactataaagataccaggcgtttccccctggaagctccctcgtgcgctctcctgttccgaccctgccgcttaccggatacctgtccgcctttctcccttcgggaagcgtggcgctttctcatagctcacgctgtaggtatctcagttcggtgtaggtcgttcgctccaagctgggctgtgtgcacgaaccccccgttcagcccgaccgctgcgccttatccggtaactatcgtcttgagtccaacccggtaagacacgacttatcgccactggcagcagccactggtaacaggattagcagagcgaggtatgtaggcggtgctacagagttcttgaagtggtggcctaactacggctacactagaagaacagtatttggtatctgcgctctgctgaagccagttaccttcggaaaaagagttggtagctcttgatccggcaaacaaaccaccgctggtagcggtggtttttttgtttgcaagcagcagattacgcgcagaaaaaaaggatctcaagaagatcctttgatcttttctacggggtctgacgctcagtggaacgaaaactcacgttaagggattttggtcatgagattatcaaaaaggatcttcacctagatccttttaaattaaaaatgaagttttaaatcaatctaaagtatatatgagtaaacttggtctgacagttaccaatgcttaatcagtgaggcacctatctcagcgatctgtctatttcgttcatccatagttgcctgactccccgtcgtgtagataactacgatacgggagggcttaccatctggccccagtgctgcaatgataccgcgagaaccacgctcaccggctccagatttatcagcaataaaccagccagccggaagggccgagcgcagaagtggtcctgcaactttatccgcctccatccagtctattaattgttgccgggaagctagagtaagtagttcgccagttaatagtttgcgcaacgttgttgccattgctacaggcatcgtggtgtcacgctcgtcgtttggtatggcttcattcagctccggttcccaacgatcaaggcgagttacatgatcccccatgttgtgcaaaaaagcggttagctccttcggtcctccgatcgttgtcagaagtaagttggccgcagtgttatcactcatggttatggcagcactgcataattctcttactgtcatgccatccgtaagatgcttttctgtgactggtgagtactcaaccaagtcattctgagaatagtgtatgcggcgaccgagttgctcttgcccggcgtcaatacgggataataccgcgccacatagcagaactttaaaagtgctcatcattggaaaacgttcttcggggcgaaaactctcaaggatcttaccgctgttgagatccagttcgatgtaacccactcgtgcacccaactgatcttcagcatcttttactttcaccagcgtttctgggtgagcaaaaacaggaaggcaaaatgccgcaaaaaagggaataagggcgacacggaaatgttgaatactcatactcttcctttttcaatattattgaagcatttatcagggttattgtctcatgagcggatacatatttgaatgtatttagaaaaataaacaaataggggttccgcgcacatttccccgaaaagtgccac

SEQ ID NO: 21 - DNA, 2763 bp, Artificial Sequence
  HLA-A-ex2-3_sg-sp-opti_2 vector V2.J.1
ctaaattgtaagcgttaatattttgttaaaattcgcgttaaatttttgttaaatcagctcattttttaaccaataggccgaaatcggcaaaatcccttataaatcaaaagaatagaccgagatagggttgagtggccgctacagggcgctcccattcgccattcaggctgcgcaactgttgggaagggcgtttcggtgcgggcctcttcgctattacgccagctggcgaaagggggatgtgctgcaaggcgattaagttgggtaacgccagggttttcccagtcacgacgttgtaaaacgacggccagtgagcgcgacgtaatacgactcactatagggcgaattggcggaaggccgtcaaggccgcatggatccaaggtcgggcaggaagagggcctatttcccatgattccttcatatttgcatatacgatacaaggctgttagagagataattagaattaatttgactgtaaacacaaagatattagtacaaaatacgtgacgtagaaagtaataatttcttgggtagtttgcagttttaaaattatgttttaaaatggactatcatatgcttaccgtaacttgaaagtatttcgatttcttggctttatatatcttgtggaaaggacgaaacaccgcaggctctcactgaacgggagtttaagagctatgctggaaacagcatagcaagtttaaataaggctagtccgttatcaacttgaaaaagtggcaccgagtcggtgctttttttcagacatccatagatctagctcgagttttttttctagactgggcctcatgggccttccgctcactgcccgctttccagtcgggaaacctgtcgtgccagctgcattaacatggtcatagctgtttccttgcgtattgggcgctctccgcttcctcgctcactgactcgctgcgctcggtcgttcgggtaaagcctggggtgcctaatgagcaaaaggccagcaaaaggccaggaaccgtaaaaaggccgcgttgctggcgtttttccataggctccgcccccctgacgagcatcacaaaaatcgacgctcaagtcagaggtggcgaaacccgacaggactataaagataccaggcgtttccccctggaagctccctcgtgcgctctcctgttccgaccctgccgcttaccggatacctgtccgcctttctcccttcgggaagcgtggcgctttctcatagctcacgctgtaggtatctcagttcggtgtaggtcgttcgctccaagctgggctgtgtgcacgaaccccccgttcagcccgaccgctgcgccttatccggtaactatcgtcttgagtccaacccggtaagacacgacttatcgccactggcagcagccactggtaacaggattagcagagcgaggtatgtaggcggtgctacagagttcttgaagtggtggcctaactacggctacactagaagaacagtatttggtatctgcgctctgctgaagccagttaccttcggaaaaagagttggtagctcttgatccggcaaacaaaccaccgctggtagcggtggtttttttgtttgcaagcagcagattacgcgcagaaaaaaaggatctcaagaagatcctttgatcttttctacggggtctgacgctcagtggaacgaaaactcacgttaagggattttggtcatgagattatcaaaaaggatcttcacctagatccttttaaattaaaaatgaagttttaaatcaatctaaagtatatatgagtaaacttggtctgacagttaccaatgcttaatcagtgaggcacctatctcagcgatctgtctatttcgttcatccatagttgcctgactccccgtcgtgtagataactacgatacgggagggcttaccatctggccccagtgctgcaatgataccgcgagaaccacgctcaccggctccagatttatcagcaataaaccagccagccggaagggccgagcgcagaagtggtcctgcaactttatccgcctccatccagtctattaattgttgccgggaagctagagtaagtagttcgccagttaatagtttgcgcaacgttgttgccattgctacaggcatcgtggtgtcacgctcgtcgtttggtatggcttcattcagctccggttcccaacgatcaaggcgagttacatgatcccccatgttgtgcaaaaaagcggttagctccttcggtcctccgatcgttgtcagaagtaagttggccgcagtgttatcactcatggttatggcagcactgcataattctcttactgtcatgccatccgtaagatgcttttctgtgactggtgagtactcaaccaagtcattctgagaatagtgtatgcggcgaccgagttgctcttgcccggcgtcaatacgggataataccgcgccacatagcagaactttaaaagtgctcatcattggaaaacgttcttcggggcgaaaactctcaaggatcttaccgctgttgagatccagttcgatgtaacccactcgtgcacccaactgatcttcagcatcttttactttcaccagcgtttctgggtgagcaaaaacaggaaggcaaaatgccgcaaaaaagggaataagggcgacacggaaatgttgaatactcatactcttcctttttcaatattattgaagcatttatcagggttattgtctcatgagcggatacatatttgaatgtatttagaaaaataaacaaataggggttccgcgcacatttccccgaaaagtgccac

SEQ ID NO: 22 - DNA, 2762 bp, Artificial Sequence
  AAVSI_sg-sp-opti_3 vector V2.J.6
ctaaattgtaagcgttaatattttgttaaaattcgcgttaaatttttgttaaatcagctcattttttaaccaataggccgaaatcggcaaaatcccttataaatcaaaagaatagaccgagatagggttgagtggccgctacagggcgctcccattcgccattcaggctgcgcaactgttgggaagggcgtttcggtgcgggcctcttcgctattacgccagctggcgaaagggggatgtgctgcaaggcgattaagttgggtaacgccagggttttcccagtcacgacgttgtaaaacgacggccagtgagcgcgacgtaatacgactcactatagggcgaattggcggaaggccgtcaaggccgcatggatccaaggtcgggcaggaagagggcctatttcccatgattccttcatatttgcatatacgatacaaggctgttagagagataattagaattaatttgactgtaaacacaaagatattagtacaaaatacgtgacgtagaaagtaataatttcttgggtagtttgcagttttaaaattatgttttaaaatggactatcatatgcttaccgtaacttgaaagtatttcgatttcttggctttatatatcttgtggaaaggacgaaacaccgtcaccaatcctgtccctaggtttaagagctatgctggaaacagcatagcaagtttaaataaggctagtccgttatcaacttgaaaaagtggcaccgagtcggtgctttttttcagacatccatagatctagctcgagttttttttctagactgggcctcatgggccttccgctcactgcccgctttccagtcgggaaacctgtcgtgccagctgcattaacatggtcatagctgtttccttgcgtattgggcgctctccgcttcctcgctcactgactcgctgcgctcggtcgttcgggtaaagcctggggtgcctaatgagcaaaaggccagcaaaaggccaggaaccgtaaaaaggccgcgttgctggcgtttttccataggctccgcccccctgacgagcatcacaaaaatcgacgctcaagtcagaggtggcgaaacccgacaggactataaagataccaggcgtttccccctggaagctccctcgtgcgctctcctgttccgaccctgccgcttaccggatacctgtccgcctttctcccttcgggaagcgtggcgctttctcatagctcacgctgtaggtatctcagttcggtgtaggtcgttcgctccaagctgggctgtgtgcacgaaccccccgttcagcccgaccgctgcgccttatccggtaactatcgtcttgagtccaacccggtaagacacgacttatcgccactggcagcagccactggtaacaggattagcagagcgaggtatgtaggcggtgctacagagttcttgaagtggtggcctaactacggctacactagaagaacagtatttggtatctgcgctctgctgaagccagttaccttcggaaaaagagttggtagctcttgatccggcaaacaaaccaccgctggtagcggtggtttttttgtttgcaagcagcagattacgcgcagaaaaaaaggatctcaagaagatcctttgatcttttctacggggtctgacgctcagtggaacgaaaactcacgttaagggattttggtcatgagattatcaaaaaggatcttcacctagatccttttaaattaaaaatgaagttttaaatcaatctaaagtatatatgagtaaacttggtctgacagttaccaatgcttaatcagtgaggcacctatctcagcgatctgtctatttcgttcatccatagttgcctgactccccgtcgtgtagataactacgatacgggagggcttaccatctggccccagtgctgcaatgataccgcgagaaccacgctcaccggctccagatttatcagcaataaaccagccagccggaagggccgagcgcagaagtggtcctgcaactttatccgcctccatccagtctattaattgttgccgggaagctagagtaagtagttcgccagttaatagtttgcgcaacgttgttgccattgctacaggcatcgtggtgtcacgctcgtcgtttggtatggcttcattcagctccggttcccaacgatcaaggcgagttacatgatcccccatgttgtgcaaaaaagcggttagctccttcggtcctccgatcgttgtcagaagtaagttggccgcagtgttatcactcatggttatggcagcactgcataattctcttactgtcatgccatccgtaagatgcttttctgtgactggtgagtactcaaccaagtcattctgagaatagtgtatgcggcgaccgagttgctcttgcccggcgtcaatacgggataataccgcgccacatagcagaactttaaaagtgctcatcattggaaaacgttcttcggggcgaaaactctcaaggatcttaccgctgttgagatccagttcgatgtaacccactcgtgcacccaactgatcttcagcatcttttactttcaccagcgtttctgggtgagcaaaaacaggaaggcaaaatgccgcaaaaaagggaataagggcgacacggaaatgttgaatactcatactcttcctttttcaatattattgaagcatttatcagggttattgtctcatgagcggatacatatttgaatgtatttagaaaaataaacaaataggggttccgcgcacatttccccgaaaagtgccac

SEQ ID NO: 23 - DNA, 6275 bp, Artificial Sequence
  pMA-CS-JG9-TCRbeta vector V3.C.5
gacggatcgggagatctcccgatcccctatggtgcactctcagtacaatctgctctgatgccgcatagttaagccagtatctgctccctgcttgtgtgttggaggtcgctgagtagtgcgcgagcaaaatttaagctacaacaaggcaaggcttgaccgacaattgcatgaagaatctgcttagggttaggcgttttgcgctgcttcgcgatgtacgggccagatatacgcgttgacattgattattgactagttattaatagtaatcaattacggggtcattagttcatagcccatatatggagttccgcgttacataacttacggtaaatggcccgcctggctgaccgcccaacgacccccgcccattgacgtcaataatgacgtatgttcccatagtaacgccaatagggactttccattgacgtcaatgggtggagtatttacggtaaactgcccacttggcagtacatcaagtgtatcatatgccaagtacgccccctattgacgtcaatgacggtaaatggcccgcctggcattatgcccagtacatgaccttatgggactttcctacttggcagtacatctacgtattagtcatcgctattaccatggtgatgcggttttggcagtacatcaatgggcgtggatagcggtttgactcacggggatttccaagtctccaccccattgacgtcaatgggagtttgttttggcaccaaaatcaacgggactttccaaaatgtcgtaacaactccgccccattgacgcaaatgggcggtaggcgtgtacggtgggaggtctatataagcagagctctctggctaactagagaacccactgcttactggcttatcgaaattaatacgactcactatagggagacccaagctggctagcgtttaaacttaagcttggtaccgagctcggatccaccatggactcctggaccttctgctgtgtgtccctttgcatcctggtagcaaagcacacagatgctggagttatccagtcaccccggcacgaggtgacagagatgggacaagaagtgactctgagatgtaaaccaatttcaggacacgactaccttttctggtacagacagaccatgatgcggggactggagttgctcatttactttaacaacaacgttccgatagatgattcagggatgcccgaggatcgattctcagctaagatgcctaatgcatcattctccactctgaagatccagccctcagaacccagggactcagctgtgtacttctgtgccagcagttcggcaaactatggctacaccttcggttcggggaccaggttaaccgttgtagaggacctgaacaaggtgttcccacccgaggtcgctgtgtttgagccatcagaagcagagatctcccacacccaaaaggccacactggtgtgcctggccacaggcttcttccctgaccacgtggagctgagctggtgggtgaatgggaaggaggtgcacagtggggtcagcacggacccgcagcccctcaaggagcagcccgccctcaatgactccagatactgcctgagcagccgcctgagggtctcggccaccttctggcagaacccccgcaaccacttccgctgtcaagtccagttctacgggctctcggagaatgacgagtggacccaggatagggccaaacccgtcacccagatcgtcagcgccgaggcctggggtagagcagactgtggctttacctcggtgtcctaccagcaaggggtcctgtctgccaccatcctctatgagatcctgctagggaaggccaccctgtatgctgtgctggtcagcgcccttgtgttgatggccatggtcaagagaaaggatttctgattctagacgactgtgccttctagttgccagccatctgttgtttgcccctcccccgtgccttccttgaccctggaaggtgccactcccactgtcctttcctaataaaatgaggaaattgcatcgcattgtctgagtaggtgtcattctattctggggggtggggtggggcaggacagcaagggggaggattgggaagacaatagcaggcatgctggggatgcggtgggctctatggcttctgaggcggaaagaaccagctggggctctagggggtatccccacgcgccctgtagcggcgcattaagcgcggcgggtgtggtggttacgcgcagcgtgaccgctacacttgccagcgccctagcgcccgctcctttcgctttcttcccttcctttctcgccacgttcgccggctttccccgtcaagctctaaatcgggggctccctttagggttccgatttagtgctttacggcacctcgaccccaaaaaacttgattagggtgatggttcacgtagtgggccatcgccctgatagacggtttttcgccctttgacgttggagtccacgttctttaatagtggactcttgttccaaactggaacaacactcaaccctatctcggtctattcttttgatttataagggattttgccgatttcggcctattggttaaaaaatgagctgatttaacaaaaatttaacgcgaattaattctgtggaatgtgtgtcagttagggtgtggaaagtccccaggctccccagcaggcagaagtatgcaaagcatgcatctcaattagtcagcaaccaggtgtggaaagtccccaggctccccagcaggcagaagtatgcaaagcatgcatctcaattagtcagcaaccatagtcccgcccctaactccgcccatcccgcccctaactccgcccagttccgcccattctccgccccatggctgactaattttttttatttatgcagaggccgaggccgcctctgcctctgagctattccagaagtagtgaggaggcttttttggaggcctaggcttttgcaaaaagctcccgggagcttgtatatccattttcggatctgatcaagagacaggatgaggatcgtttcgcatgattgaacaagatggattgcacgcaggttctccggccgcttgggtggagaggctattcggctatgactgggcacaacagacaatcggctgctctgatgccgccgtgttccggctgtcagcgcaggggcgcccggttctttttgtcaagaccgacctgtccggtgccctgaatgaactgcaggacgaggcagcgcggctatcgtggctggccacgacgggcgttccttgcgcagctgtgctcgacgttgtcactgaagcgggaagggactggctgctattgggcgaagtgccggggcaggatctcctgtcatctcaccttgctcctgccgagaaagtatccatcatggctgatgcaatgcggcggctgcatacgcttgatccggctacctgcccattcgaccaccaagcgaaacatcgcatcgagcgagcacgtactcggatggaagccggtcttgtcgatcaggatgatctggacgaagagcatcaggggctcgcgccagccgaactgttcgccaggctcaaggcgcgcatgcccgacggcgaggatctcgtcgtgacccatggcgatgcctgcttgccgaatatcatggtggaaaatggccgcttttctggattcatcgactgtggccggctgggtgtggcggaccgctatcaggacatagcgttggctacccgtgatattgctgaagagcttggcggcgaatgggctgaccgcttcctcgtgctttacggtatcgccgctcccgattcgcagcgcatcgccttctatcgccttcttgacgagttcttctgagcgggactctggggttcgaaatgaccgaccaagcgacgcccaacctgccatcacgagatttcgattccaccgccgccttctatgaaaggttgggcttcggaatcgttttccgggacgccggctggatgatcctccagcgcggggatctcatgctggagttcttcgcccaccccaacttgtttattgcagcttataatggttacaaataaagcaatagcatcacaaatttcacaaataaagcatttttttcactgcattctagttgtggtttgtccaaactcatcaatgtatcttatcatgtctgtataccgtcgacctctagctagagcttggcgtaatcatggtcatagctgtttcctgtgtgaaattgttatccgctcacaattccacacaacatacgagccggaagcataaagtgtaaagcctggggtgcctaatgagtgagctaactcacattaattgcgttgcgctcactgcccgctttccagtcgggaaacctgtcgtgccagctgcattaatgaatcggccaacgcgcggggagaggcggtttgcgtattgggcgctcttccgcttcctcgctcactgactcgctgcgctcggtcgttcggctgcggcgagcggtatcagctcactcaaaggcggtaatacggttatccacagaatcaggggataacgcaggaaagaacatgtgagcaaaaggccagcaaaaggccaggaaccgtaaaaaggccgcgttgctggcgtttttccataggctccgcccccctgacgagcatcacaaaaatcgacgctcaagtcagaggtggcgaaacccgacaggactataaagataccaggcgtttccccctggaagctccctcgtgcgctctcctgttccgaccctgccgcttaccggatacctgtccgcctttctcccttcgggaagcgtggcgctttctcatagctcacgctgtaggtatctcagttcggtgtaggtcgttcgctccaagctgggctgtgtgcacgaaccccccgttcagcccgaccgctgcgccttatccggtaactatcgtcttgagtccaacccggtaagacacgacttatcgccactggcagcagccactggtaacaggattagcagagcgaggtatgtaggcggtgctacagagttcttgaagtggtggcctaactacggctacactagaagaacagtatttggtatctgcgctctgctgaagccagttaccttcggaaaaagagttggtagctcttgatccggcaaacaaaccaccgctggtagcggtttttttgtttgcaagcagcagattacgcgcagaaaaaaaggatctcaagaagatcctttgatcttttctacggggtctgacgctcagtggaacgaaaactcacgttaagggattttggtcatgagattatcaaaaaggatcttcacctagatccttttaaattaaaaatgaagttttaaatcaatctaaagtatatatgagtaaacttggtctgacagttaccaatgcttaatcagtgaggcacctatctcagcgatctgtctatttcgttcatccatagttgcctgactccccgtcgtgtagataactacgatacgggagggcttaccatctggccccagtgctgcaatgataccgcgagacccacgctcaccggctccagatttatcagcaataaaccagccagccggaagggccgagcgcagaagtggtcctgcaactttatccgcctccatccagtctattaattgttgccgggaagctagagtaagtagttcgccagttaatagtttgcgcaacgttgttgccattgctacaggcatcgtggtgtcacgctcgtcgtttggtatggcttcattcagctccggttcccaacgatcaaggcgagttacatgatcccccatgttgtgcaaaaaagcggttagctccttcggtcctccgatcgttgtcagaagtaagttggccgcagtgttatcactcatggttatggcagcactgcataattctcttactgtcatgccatccgtaagatgcttttctgtgactggtgagtactcaaccaagtcattctgagaatagtgtatgcggcgaccgagttgctcttgcccggcgtcaatacgggataataccgcgccacatagcagaactttaaaagtgctcatcattggaaaacgttcttcggggcgaaaactctcaaggatcttaccgctgttgagatccagttcgatgtaacccactcgtgcacccaactgatcttcagcatcttttactttcaccagcgtttctgggtgagcaaaaacaggaaggcaaaatgccgcaaaaaagggaataagggcgacacggaaatgttgaatactcatactcttcctttttcaatattattgaagcatttatcagggttattgtctcatgagcggatacatatttgaatgtatttagaaaaataaacaaataggggttccgcgcacatttccccgaaaagtgccacctgacgtc

SEQ ID NO: 24 - DNA, 6125 bp, Artificial Sequence
  AAVS_Efla-intron_F14_RFPnls_F15 vector V4.B.2
ctaaattgtaagcgttaatattttgttaaaattcgcgttaaatttttgttaaatcagctcattttttaaccaataggccgaaatcggcaaaatcccttataaatcaaaagaatagaccgagatagggttgagtggccgctacagggcgctcccattcgccattcaggctgcgcaactgttgggaagggcgtttcggtgcgggcctcttcgctattacgccagctggcgaaagggggatgtgctgcaaggcgattaagttgggtaacgccagggttttcccagtcacgacgttgtaaaacgacggccagtgagcgcgacgtaatacgactcactatagggcgaattggcggaaggccgtcaaggccgcatgaattgagctctactggcttctgcgccgcctctggcccactgtttccccttcccaggcaggtcctgctttctctgacctgcattctctcccctgggcctgtgccgctttctgtctgcagcttgtggcctgggtcacctctacggctggcccagatccttccctgccgcctccttcaggttccgtcttcctccactccctcttccccttgctctctgctgtgttgctgcccaaggatgctctttccggagcacttccttctcggcgctgcaccacgtgatgtcctctgagcggatcctccccgtgtctgggtcctctccgggcatctctcctccctcacccaaccccatgccgtcttcactcgctgggttcccttttccttctccttctggggcctgtgccatctctcgtttcttaggatggccttctccgacggatgtctcccttgcgtcccgcctccccttcttgtaggcctgcatcatcaccgtttttctggacaaccccaaagtaccccgtctccctggctttagccacctctccatcctcttgctttctttgcctggacaccccgttctcctgtggattcgggtcacctctcactcctttcatttgggcagctcccctaccccccttacctctctagtctgtgctagctcttccagccccctgtcatggcatcttccaggggtccgagagctcagctagtcttcttcctccaacccgggcccctatgtccacttcaggacagcatgtttgctgcctccagggatcctgtgtccccgagctgggaccaccttatattcccagggccggttaatgtggctctggttctgggtacttttatctgtcccctccaccgggtggctccggtgcccgtcagtgggcagagcgcacatcgcccacagtccccgagaagttggggggaggggtcggcaattgaaccggtgcctagagaaggtggcgcggggtaaactgggaaagtgatgtcgtgtactggctccgcctttttcccgagggtgggggagaaccgtatataagtgcagtagtcgccgtgaacgttctttttcgcaacgggtttgccgccagaacacaggtaagtgccgtgtgtggttcccgcgggcctggcctctttacgggttatggcccttgcgtgccttgaattacttccactggctgcagtacgtgattcttgatcccgagcttcgggttggaagtgggtgggagagttcgaggccttgcgcttaaggagccccttcgcctcgtgcttgagttgaggcctggcctgggcgctggggccgccgcgtgcgaatctggtggcaccttcgcgcctgtctcgctgctttcgataagtctctagccatttaaaatttttgatgacctgctgcgacgctttttttctggcaagatagtcttgtaaatgcgggccaagatctgcacactggtatttcggtttttggggccgcgggcggcgacggggcccgtgcgtcccagcgcacatgttcggcgaggcggggcctgcgagcgcggccaccgagaatcggacgggggtagtctcaagctggccggcctgctctggtgcctggcctcgcgccgccgtgtatcgccccgccctgggcggcaaggctggcccggtcggcaccagttgcgtgagcggaaagatggccgcttcccggccctgctgcagggagctcaaaatggaggacgcggcgctcgggagagcgggcgggtgagtcacccacacaaaggaaaagggcctttccgtcctcagccgtcgcttcatgtgactccacggagtaccgggcgccgtccaggcacctcgattagttctcgagcttttggagtacgtcgtctttaggttggggggaggggttttatgcgatggagtttccccacactgagtgggtggagactgaagttaggccagcttggcacttgatgtaattctccttggaatttgccctttttgagtttggatcttggttcattctcaagcctcagacagtggttcaaagtttttttcttccatttcaggtgtcgtgactggtaccggaagttcctattccgaagttcctattctatcagaagtataggaacttcgtaccgagaccatggccccaaagaagaagcggaaggtcggtatccacggagtcccagcagccatgagcgagctgatcaaagaaaacatgcacatgaagctgtacatggaaggcaccgtgaacaaccaccacttcaagtgcaccagcgagggcgagggcaagccttacgagggcacccagaccatgaagatcaaggtggtggaaggcggccctctgcccttcgcctttgatatcctggccaccagctttatgtacggcagcaaggccttcatcaaccacacccagggcatccccgatttcttcaagcagagcttccccgagggcttcacctgggagcggatcaccacatacgaggacggcggagtgctgaccgccacccaggataccagcttccagaacggctgcatcatctacaacgtgaagattaacggcgtgaatttccccagcaacggccccgtgatgcagaagaaaaccagaggctgggaggccaacaccgagatgctgtaccctgccgatggcggcctgagaggccattctcagatggccctgaaactcgtgggcggaggctacctgcactgctccttcaagaccacctacagaagcaagaagcccgccaagaacctgaagatgcccggcttccacttcgtggaccaccggctggaacggatcaaagaggccgacaaagaaacctacgtggaacagcacgagatggccgtggccaagtactgcgacctgcctagcaagctgggccacagaaaaaggccggcggccacgaaaaaggccggccaggcaaaaaagaaaaagtgaggtctctctaggaagttcctattccgaagttcctattcttataggagtataggaacttctctagacctgatcataatcaagccatatcacatctgtagaggtttacttgctttaaaaaacctccacacctccccctgaacctgaaacataaaatgaatgcaattgttgttgttaacttgtttattgcagcttataatggttacaaataaagcaatagcatcacaaatttcacaaataaagcatttttttcactgcattctagttgtggtttgtccaaactcatcaatgtatcttatcatgtctggatctgcggatcaggattggtgacagaaaagccccatccttaggcctcctccttcctagtctcctgatattgggtctaacccccacctcctgttaggcagattccttatctggtgacacacccccatttcctggagccatctctctccttgccagaacctctaaggtttgcttacgatggagccagagaggatcctgggagggagagcttggcagggggtgggagggaagggggggatgcgtgacctgcccggttctcagtggccaccctgcgctaccctctcccagaacctgagctgctctgacgcggctgtctggtgcgtttcactgatcctggtgctgcagcttccttacacttcccaagaggagaagcagtttggaaaaacaaaatcagaataagttggtcctgagttctaactttggctcttcacctttctagtccccaatttatattgttcctccgtgcgtcagttttacctgtgagataaggccagtagccagccccgtcctggcagggctgtggtgaggaggggggtgtccgtgtggaaaactccctttgtgagaatggtgcgtcctcgagctgggcctcatgggccttccgctcactgcccgctttccagtcgggaaacctgtcgtgccagctgcattaacatggtcatagctgtttccttgcgtattgggcgctctccgcttcctcgctcactgactcgctgcgctcggtcgttcgggtaaagcctggggtgcctaatgagcaaaaggccagcaaaaggccaggaaccgtaaaaaggccgcgttgctggcgtttttccataggctccgcccccctgacgagcatcacaaaaatcgacgctcaagtcagaggtggcgaaacccgacaggactataaagataccaggcgtttccccctggaagctccctcgtgcgctctcctgttccgaccctgccgcttaccggatacctgtccgcctttctcccttcgggaagcgtggcgctttctcatagctcacgctgtaggtatctcagttcggtgtaggtcgttcgctccaagctgggctgtgtgcacgaaccccccgttcagcccgaccgctgcgccttatccggtaactatcgtcttgagtccaacccggtaagacacgacttatcgccactggcagcagccactggtaacaggattagcagagcgaggtatgtaggcggtgctacagagttcttgaagtggtggcctaactacggctacactagaagaacagtatttggtatctgcgctctgctgaagccagttaccttcggaaaaagagttggtagctcttgatccggcaaacaaaccaccgctggtagcggtggtttttttgtttgcaagcagcagattacgcgcagaaaaaaaggatctcaagaagatcctttgatcttttctacggggtctgacgctcagtggaacgaaaactcacgttaagggattttggtcatgagattatcaaaaaggatcttcacctagatccttttaaattaaaaatgaagttttaaatcaatctaaagtatatatgagtaaacttggtctgacagttaccaatgcttaatcagtgaggcacctatctcagcgatctgtctatttcgttcatccatagttgcctgactccccgtcgtgtagataactacgatacgggagggcttaccatctggccccagtgctgcaatgataccgcgagaaccacgctcaccggctccagatttatcagcaataaaccagccagccggaagggccgagcgcagaagtggtcctgcaactttatccgcctccatccagtctattaattgttgccgggaagctagagtaagtagttcgccagttaatagtttgcgcaacgttgttgccattgctacaggcatcgtggtgtcacgctcgtcgtttggtatggcttcattcagctccggttcccaacgatcaaggcgagttacatgatcccccatgttgtgcaaaaaagcggttagctccttcggtcctccgatcgttgtcagaagtaagttggccgcagtgttatcactcatggttatggcagcactgcataattctcttactgtcatgccatccgtaagatgcttttctgtgactggtgagtactcaaccaagtcattctgagaatagtgtatgcggcgaccgagttgctcttgcccggcgtcaatacgggataataccgcgccacatagcagaactttaaaagtgctcatcattggaaaacgttcttcggggcgaaaactctcaaggatcttaccgctgttgagatccagttcgatgtaacccactcgtgcacccaactgatcttcagcatcttttactttcaccagcgtttctgggtgagcaaaaacaggaaggcaaaatgccgcaaaaaagggaataagggcgacacggaaatgttgaatactcatactcttcctttttcaatattattgaagcatttatcagggttattgtctcatgagcggatacatatttgaatgtatttagaaaaataaacaaataggggttccgcgcacatttccccgaaaagtgccac

SEQ ID NO: 25 - DNA, 6131 bp, Artificial Sequence
  AAVS_Efla-intron_FRT_BFPnls_F3 vector V4.B.3
ctaaattgtaagcgttaatattttgttaaaattcgcgttaaatttttgttaaatcagctcattttttaaccaataggccgaaatcggcaaaatcccttataaatcaaaagaatagaccgagatagggttgagtggccgctacagggcgctcccattcgccattcaggctgcgcaactgttgggaagggcgtttcggtgcgggcctcttcgctattacgccagctggcgaaagggggatgtgctgcaaggcgattaagttgggtaacgccagggttttcccagtcacgacgttgtaaaacgacggccagtgagcgcgacgtaatacgactcactatagggcgaattggcggaaggccgtcaaggccgcatgaattgagctctactggcttctgcgccgcctctggcccactgtttccccttcccaggcaggtcctgctttctctgacctgcattctctcccctgggcctgtgccgctttctgtctgcagcttgtggcctgggtcacctctacggctggcccagatccttccctgccgcctccttcaggttccgtcttcctccactccctcttccccttgctctctgctgtgttgctgcccaaggatgctctttccggagcacttccttctcggcgctgcaccacgtgatgtcctctgagcggatcctccccgtgtctgggtcctctccgggcatctctcctccctcacccaaccccatgccgtcttcactcgctgggttcccttttccttctccttctggggcctgtgccatctctcgtttcttaggatggccttctccgacggatgtctcccttgcgtcccgcctccccttcttgtaggcctgcatcatcaccgtttttctggacaaccccaaagtaccccgtctccctggctttagccacctctccatcctcttgctttctttgcctggacaccccgttctcctgtggattcgggtcacctctcactcctttcatttgggcagctcccctaccccccttacctctctagtctgtgctagctcttccagccccctgtcatggcatcttccaggggtccgagagctcagctagtcttcttcctccaacccgggcccctatgtccacttcaggacagcatgtttgctgcctccagggatcctgtgtccccgagctgggaccaccttatattcccagggccggttaatgtggctctggttctgggtacttttatctgtcccctccaccgggtggctccggtgcccgtcagtgggcagagcgcacatcgcccacagtccccgagaagttggggggaggggtcggcaattgaaccggtgcctagagaaggtggcgcggggtaaactgggaaagtgatgtcgtgtactggctccgcctttttcccgagggtgggggagaaccgtatataagtgcagtagtcgccgtgaacgttctttttcgcaacgggtttgccgccagaacacaggtaagtgccgtgtgtggttcccgcgggcctggcctctttacgggttatggcccttgcgtgccttgaattacttccactggctgcagtacgtgattcttgatcccgagcttcgggttggaagtgggtgggagagttcgaggccttgcgcttaaggagccccttcgcctcgtgcttgagttgaggcctggcctgggcgctggggccgccgcgtgcgaatctggtggcaccttcgcgcctgtctcgctgctttcgataagtctctagccatttaaaatttttgatgacctgctgcgacgctttttttctggcaagatagtcttgtaaatgcgggccaagatctgcacactggtatttcggtttttggggccgcgggcggcgacggggcccgtgcgtcccagcgcacatgttcggcgaggcggggcctgcgagcgcggccaccgagaatcggacgggggtagtctcaagctggccggcctgctctggtgcctggcctcgcgccgccgtgtatcgccccgccctgggcggcaaggctggcccggtcggcaccagttgcgtgagcggaaagatggccgcttcccggccctgctgcagggagctcaaaatggaggacgcggcgctcgggagagcgggcgggtgagtcacccacacaaaggaaaagggcctttccgtcctcagccgtcgcttcatgtgactccacggagtaccgggcgccgtccaggcacctcgattagttctcgagcttttggagtacgtcgtctttaggttggggggaggggttttatgcgatggagtttccccacactgagtgggtggagactgaagttaggccagcttggcacttgatgtaattctccttggaatttgccctttttgagtttggatcttggttcattctcaagcctcagacagtggttcaaagtttttttcttccatttcaggtgtcgtgactggtaccggaagttcctattccgaagttcctattctctagaaagtataggaacttcgtaccgagaccatggccccaaagaagaagcggaaggtcggtatccacggagtcccagcagccatgagcgagctgattaaggagaacatgcacatgaagctgtacatggagggcaccgtggacaaccatcacttcaagtgcacatccgagggcgaaggcaagccctacgagggcacccagaccatgagaatcaaggtggtcgagggcggccctctccccttcgccttcgacatcctggctactagcttcctctacggcagcaagaccttcatcaaccacacccagggcatccccgacttcttcaagcagtccttccctgagggcttcacatgggagagagtcaccacatacgaggacgggggcgtgctgaccgctacccaggacaccagcctccaggacggctgcctcatctacaacgtcaagatcagaggggtgaatttcacatccaacggccctgtgatgcagaagaaaacactcggctgggaggccttcaccgagacgctgtaccccgctgacggcggcctggaaggcagaaacgacatggccctgaagctcgtgggcgggagccatctgatcgcaaacatcaagaccacatatagatccaagaaacccgctaagaacctcaagatgcctggcgtctactatgtggactacagactggaaagaatcaaggaggccaacaacgagacatacgtcgagcagcacgaggtggcagtggccagatactgcgacctccctagcaaactggggcacaagcttaataaaaggccggcggccacgaaaaaggccggccaggcaaaaaagaaaaagtaaggtctctctaggaagttcctattccgaagttcctattcttcaaatagtataggaacttctctagacctgatcataatcaagccatatcacatctgtagaggtttacttgctttaaaaaacctccacacctccccctgaacctgaaacataaaatgaatgcaattgttgttgttaacttgtttattgcagcttataatggttacaaataaagcaatagcatcacaaatttcacaaataaagcatttttttcactgcattctagttgtggtttgtccaaactcatcaatgtatcttatcatgtctggatctgcggatcaggattggtgacagaaaagccccatccttaggcctcctccttcctagtctcctgatattgggtctaacccccacctcctgttaggcagattccttatctggtgacacacccccatttcctggagccatctctctccttgccagaacctctaaggtttgcttacgatggagccagagaggatcctgggagggagagcttggcagggggtgggagggaagggggggatgcgtgacctgcccggttctcagtggccaccctgcgctaccctctcccagaacctgagctgctctgacgcggctgtctggtgcgtttcactgatcctggtgctgcagcttccttacacttcccaagaggagaagcagtttggaaaaacaaaatcagaataagttggtcctgagttctaactttggctcttcacctttctagtccccaatttatattgttcctccgtgcgtcagttttacctgtgagataaggccagtagccagccccgtcctggcagggctgtggtgaggaggggggtgtccgtgtggaaaactccctttgtgagaatggtgcgtcctcgagctgggcctcatgggccttccgctcactgcccgctttccagtcgggaaacctgtcgtgccagctgcattaacatggtcatagctgtttccttgcgtattgggcgctctccgcttcctcgctcactgactcgctgcgctcggtcgttcgggtaaagcctggggtgcctaatgagcaaaaggccagcaaaaggccaggaaccgtaaaaaggccgcgttgctggcgtttttccataggctccgcccccctgacgagcatcacaaaaatcgacgctcaagtcagaggtggcgaaacccgacaggactataaagataccaggcgtttccccctggaagctccctcgtgcgctctcctgttccgaccctgccgcttaccggatacctgtccgcctttctcccttcgggaagcgtggcgctttctcatagctcacgctgtaggtatctcagttcggtgtaggtcgttcgctccaagctgggctgtgtgcacgaaccccccgttcagcccgaccgctgcgccttatccggtaactatcgtcttgagtccaacccggtaagacacgacttatcgccactggcagcagccactggtaacaggattagcagagcgaggtatgtaggcggtgctacagagttcttgaagtggtggcctaactacggctacactagaagaacagtatttggtatctgcgctctgctgaagccagttaccttcggaaaaagagttggtagctcttgatccggcaaacaaaccaccgctggtagcggtggtttttttgtttgcaagcagcagattacgcgcagaaaaaaaggatctcaagaagatcctttgatcttttctacggggtctgacgctcagtggaacgaaaactcacgttaagggattttggtcatgagattatcaaaaaggatcttcacctagatccttttaaattaaaaatgaagttttaaatcaatctaaagtatatatgagtaaacttggtctgacagttaccaatgcttaatcagtgaggcacctatctcagcgatctgtctatttcgttcatccatagttgcctgactccccgtcgtgtagataactacgatacgggagggcttaccatctggccccagtgctgcaatgataccgcgagaaccacgctcaccggctccagatttatcagcaataaaccagccagccggaagggccgagcgcagaagtggtcctgcaactttatccgcctccatccagtctattaattgttgccgggaagctagagtaagtagttcgccagttaatagtttgcgcaacgttgttgccattgctacaggcatcgtggtgtcacgctcgtcgtttggtatggcttcattcagctccggttcccaacgatcaaggcgagttacatgatcccccatgttgtgcaaaaaagcggttagctccttcggtcctccgatcgttgtcagaagtaagttggccgcagtgttatcactcatggttatggcagcactgcataattctcttactgtcatgccatccgtaagatgcttttctgtgactggtgagtactcaaccaagtcattctgagaatagtgtatgcggcgaccgagttgctcttgcccggcgtcaatacgggataataccgcgccacatagcagaactttaaaagtgctcatcattggaaaacgttcttcggggcgaaaactctcaaggatcttaccgctgttgagatccagttcgatgtaacccactcgtgcacccaactgatcttcagcatcttttactttcaccagcgtttctgggtgagcaaaaacaggaaggcaaaatgccgcaaaaaagggaataagggcgacacggaaatgttgaatactcatactcttcctttttcaatattattgaagcatttatcagggttattgtctcatgagcggatacatatttgaatgtatttagaaaaataaacaaataggggttccgcgcacatttccccgaaaagtgccac

SEQ ID NO: 26 - DNA, 3602 bp, Artificial Sequence
  pMA_FRT_HLA-A*02:01-6xHis_F3 vector V4.D.2
ctaaattgtaagcgttaatattttgttaaaattcgcgttaaatttttgttaaatcagctcattttttaaccaataggccgaaatcggcaaaatcccttataaatcaaaagaatagaccgagatagggttgagtggccgctacagggcgctcccattcgccattcaggctgcgcaactgttgggaagggcgtttcggtgcgggcctcttcgctattacgccagctggcgaaagggggatgtgctgcaaggcgattaagttgggtaacgccagggttttcccagtcacgacgttgtaaaacgacggccagtgagcgcgacgtaatacgactcactatagggcgaattggcggaaggccgtcaaggccgcatgaattcgctaccgggaagttcctattccgaagttcctattctctagaaagtataggaacttcaggtaccatggccgtcatggcgccccgaaccctcgtcctgctactctcgggggctctggccctgacccagacctgggcgggctctcactccatgaggtatttcttcacatccgtgtctcggccaggacgcggagagccacgcttcatcgcagtgggctacgtggacgacacgcagttcgtgcggttcgacagcgacgccgcgagccagaggatggagccgcgggcgccgtggatagagcaggagggtccggagtattgggacggggagacacggaaagtgaaggcccactcacagactcaccgagtggacctggggaccctgcgcggctactacaaccagagcgaggccggttctcacaccgtccagaggatgtatggctgcgacgtggggtcggactggcgcttcctccgcggataccaccagtacgcctacgacggcaaggattacatcgccctgaaagaggacctgcgctcttggaccgcggcggacatggcagctcagaccaccaagcacaagtgggaggcggcccatgtggcggagcagttgagagcctacctggagggcacgtgcgtggagtggctccgcagatacctggagaacgggaaggagacgctgcagcgcacggacgcccccaaaacgcatatgactcaccacgctgtctctgaccatgaagccaccctgaggtgctgggccctgagcttctaccctgcggagatcacactgacctggcagcgggatggggaggaccagacccaggacacggagctcgtggagaccaggcctgcaggggatggaaccttccagaagtgggcggctgtggtggtgccttctggacaggagcagagatacacctgccatgtgcagcatgagggtttgcccaagcccctcaccctgagatgggagccgtcttcccagcccaccatccccatcgtgggcatcattgctggcctggttctctttggagctgtgatcactggagctgtggtcgctgctgtgatgtggaggaggaagagctcagatagaaaaggagggagctactctcaggctgcaagcagtgacagtgcccagggctctgatgtgtctctcacagcttgtaaagtgcccgggcatcatcaccatcaccactgactatagtcgtctagacgaagttcctattccgaagttcctattcttcaaatagtataggaacttcctcgagctgggcctcatgggccttccgctcactgcccgctttccagtcgggaaacctgtcgtgccagctgcattaacatggtcatagctgtttccttgcgtattgggcgctctccgcttcctcgctcactgactcgctgcgctcggtcgttcgggtaaagcctggggtgcctaatgagcaaaaggccagcaaaaggccaggaaccgtaaaaaggccgcgttgctggcgtttttccataggctccgcccccctgacgagcatcacaaaaatcgacgctcaagtcagaggtggcgaaacccgacaggactataaagataccaggcgtttccccctggaagctccctcgtgcgctctcctgttccgaccctgccgcttaccggatacctgtccgcctttctcccttcgggaagcgtggcgctttctcatagctcacgctgtaggtatctcagttcggtgtaggtcgttcgctccaagctgggctgtgtgcacgaaccccccgttcagcccgaccgctgcgccttatccggtaactatcgtcttgagtccaacccggtaagacacgacttatcgccactggcagcagccactggtaacaggattagcagagcgaggtatgtaggcggtgctacagagttcttgaagtggtggcctaactacggctacactagaagaacagtatttggtatctgcgctctgctgaagccagttaccttcggaaaaagagttggtagctcttgatccggcaaacaaaccaccgctggtagcggtggtttttttgtttgcaagcagcagattacgcgcagaaaaaaaggatctcaagaagatcctttgatcttttctacggggtctgacgctcagtggaacgaaaactcacgttaagggattttggtcatgagattatcaaaaaggatcttcacctagatccttttaaattaaaaatgaagttttaaatcaatctaaagtatatatgagtaaacttggtctgacagttaccaatgcttaatcagtgaggcacctatctcagcgatctgtctatttcgttcatccatagttgcctgactccccgtcgtgtagataactacgatacgggagggcttaccatctggccccagtgctgcaatgataccgcgagaaccacgctcaccggctccagatttatcagcaataaaccagccagccggaagggccgagcgcagaagtggtcctgcaactttatccgcctccatccagtctattaattgttgccgggaagctagagtaagtagttcgccagttaatagtttgcgcaacgttgttgccattgctacaggcatcgtggtgtcacgctcgtcgtttggtatggcttcattcagctccggttcccaacgatcaaggcgagttacatgatcccccatgttgtgcaaaaaagcggttagctccttcggtcctccgatcgttgtcagaagtaagttggccgcagtgttatcactcatggttatggcagcactgcataattctcttactgtcatgccatccgtaagatgcttttctgtgactggtgagtactcaaccaagtcattctgagaatagtgtatgcggcgaccgagttgctcttgcccggcgtcaatacgggataataccgcgccacatagcagaactttaaaagtgctcatcattggaaaacgttcttcggggcgaaaactctcaaggatcttaccgctgttgagatccagttcgatgtaacccactcgtgcacccaactgatcttcagcatcttttactttcaccagcgtttctgggtgagcaaaaacaggaaggcaaaatgccgcaaaaaagggaataagggcgacacggaaatgttgaatactcatactcttcctttttcaatattattgaagcatttatcagggttattgtctcatgagcggatacatatttgaatgtatttagaaaaataaacaaataggggttccgcgcacatttccccgaaaagtgccac

SEQ ID NO: 27 - DNA, 3182 bp, Artificial Sequence
  pMA-F14-GFP-F15 vector V4.H9
ctaaattgtaagcgttaatattttgttaaaattcgcgttaaatttttgttaaatcagctcattttttaaccaataggccgaaatcggcaaaatcccttataaatcaaaagaatagaccgagatagggttgagtggccgctacagggcgctcccattcgccattcaggctgcgcaactgttgggaagggcgtttcggtgcgggcctcttcgctattacgccagctggcgaaagggggatgtgctgcaaggcgattaagttgggtaacgccagggttttcccagtcacgacgttgtaaaacgacggccagtgagcgcgacgtaatacgactcactatagggcgaattggcggaaggccgtcaaggccgcatgaattcgctaccgggaagttcctattccgaagttcctattctatcagaagtataggaacttcaggtaccgccaccatggaatccgatgagtctggcctgcccgccatggaaatcgagtgcagaatcaccggcaccctgaacggcgtggaatttgagctcgtgggcggaggcgagggcacacctgaacagggcagaatgaccaacaagatgaagtccaccaagggggccctgaccttcagcccctacctgctgtctcacgtgatgggctacggcttctaccacttcggcacctaccccagcggctacgagaaccctttcctgcacgccatcaacaacggcggctacaccaacacccggatcgagaagtacgaggacggcggcgtgctgcacgtgtccttcagctacagatacgaggccggcagagtgatcggcgacttcaaagtgatgggcaccggattccccgaggacagcgtgatcttcaccgacaagatcatccggtccaacgccaccgtggaacatctgcaccccatgggcgacaacgacctggacggcagcttcaccagaaccttctccctgcgggatggcggctactacagcagcgtggtggacagccacatgcacttcaagagcgccatccaccccagcatcctccagaacggcggacccatgttcgccttcagacgggtggaagaggaccacagcaacaccgagctgggcatcgtggaataccagcacgccttcaagacccccgatgccgatgccggcgaggaatgagtcgagtctagacgaagttcctattccgaagttcctattcttataggagtataggaacttcctcgagctgggcctcatgggccttccgctcactgcccgctttccagtcgggaaacctgtcgtgccagctgcattaacatggtcatagctgtttccttgcgtattgggcgctctccgcttcctcgctcactgactcgctgcgctcggtcgttcgggtaaagcctggggtgcctaatgagcaaaaggccagcaaaaggccaggaaccgtaaaaaggccgcgttgctggcgtttttccataggctccgcccccctgacgagcatcacaaaaatcgacgctcaagtcagaggtggcgaaacccgacaggactataaagataccaggcgtttccccctggaagctccctcgtgcgctctcctgttccgaccctgccgcttaccggatacctgtccgcctttctcccttcgggaagcgtggcgctttctcatagctcacgctgtaggtatctcagttcggtgtaggtcgttcgctccaagctgggctgtgtgcacgaaccccccgttcagcccgaccgctgcgccttatccggtaactatcgtcttgagtccaacccggtaagacacgacttatcgccactggcagcagccactggtaacaggattagcagagcgaggtatgtaggcggtgctacagagttcttgaagtggtggcctaactacggctacactagaagaacagtatttggtatctgcgctctgctgaagccagttaccttcggaaaaagagttggtagctcttgatccggcaaacaaaccaccgctggtagcggtggtttttttgtttgcaagcagcagattacgcgcagaaaaaaaggatctcaagaagatcctttgatcttttctacggggtctgacgctcagtggaacgaaaactcacgttaagggattttggtcatgagattatcaaaaaggatcttcacctagatccttttaaattaaaaatgaagttttaaatcaatctaaagtatatatgagtaaacttggtctgacagttaccaatgcttaatcagtgaggcacctatctcagcgatctgtctatttcgttcatccatagttgcctgactccccgtcgtgtagataactacgatacgggagggcttaccatctggccccagtgctgcaatgataccgcgagaaccacgctcaccggctccagatttatcagcaataaaccagccagccggaagggccgagcgcagaagtggtcctgcaactttatccgcctccatccagtctattaattgttgccgggaagctagagtaagtagttcgccagttaatagtttgcgcaacgttgttgccattgctacaggcatcgtggtgtcacgctcgtcgtttggtatggcttcattcagctccggttcccaacgatcaaggcgagttacatgatcccccatgttgtgcaaaaaagcggttagctccttcggtcctccgatcgttgtcagaagtaagttggccgcagtgttatcactcatggttatggcagcactgcataattctcttactgtcatgccatccgtaagatgcttttctgtgactggtgagtactcaaccaagtcattctgagaatagtgtatgcggcgaccgagttgctcttgcccggcgtcaatacgggataataccgcgccacatagcagaactttaaaagtgctcatcattggaaaacgttcttcggggcgaaaactctcaaggatcttaccgctgttgagatccagttcgatgtaacccactcgtgcacccaactgatcttcagcatcttttactttcaccagcgtttctgggtgagcaaaaacaggaaggcaaaatgccgcaaaaaagggaataagggcgacacggaaatgttgaatactcatactcttcctttttcaatattattgaagcatttatcagggttattgtctcatgagcggatacatatttgaatgtatttagaaaaataaacaaataggggttccgcgcacatttccccgaaaagtgccac

SEQ ID NO: 28 - DNA, 4542 bp, Artificial Sequence
  CMVpro-Flp-sv40pA-V2 vector V4.I.8
ctaaattgtaagcgttaatattttgttaaaattcgcgttaaatttttgttaaatcagctcattttttaaccaataggccgaaatcggcaaaatcccttataaatcaaaagaatagaccgagatagggttgagtggccgctacagggcgctcccattcgccattcaggctgcgcaactgttgggaagggcgtttcggtgcgggcctcttcgctattacgccagctggcgaaagggggatgtgctgcaaggcgattaagttgggtaacgccagggttttcccagtcacgacgttgtaaaacgacggccagtgagcgcgacgtaatacgactcactatagggcgaattggcggaaggccgtcaaggccgcatgaattcgctaccggtatagtaatcaattacggggtcattagttcatagcccatatatggagttccgcgttacataacttacggtaaatggcccgcctggctgaccgcccaacgacccccgcccattgacgtcaataatgacgtatgttcccatagtaacgccaatagggactttccattgacgtcaatgggtggagtatttacggtaaactgcccacttggcagtacatcaagtgtatcatatgccaagtacgccccctattgacgtcaatgacggtaaatggcccgcctggcattatgcccagtacatgaccttatgggactttcctacttggcagtacatctacgtattagtcatcgctattaccatggtgatgcggttttggcagtacatcaatgggcgtggatagcggtttgactcacggggatttccaagtctccaccccattgacgtcaatgggagtttgttttggcaccaaaatcaacgggactttccaaaatgtcgtaacaactccgccccattgacgcaaatgggcggtaggcgtgtacggtgggaggtctatataagcagagctggtttagtgaaccgtcagatcaggtaccatggcccccaagaaaaagcggaaagtgggcatccacggcgtgccagctgcaggcggctctatgagccagttcgacatcctgtgcaagaccccacctaaggtgctcgtgcggcagttcgtggaaagattcgagaggcctagcggcgagaagatcgcctcttgtgctgccgagctgacctacctgtgctggatgatcacccacaacggcaccgccatcaagcgggccaccttcatgagctacaataccatcatcagcaacagcctgagcttcgacatcgtgaacaagagcctgcagttcaagtacaagacccagaaggccaccatcctggaagccagcctgaagaaactgatccccgcctgggagtttaccatcatcccatacaatggccagaaacatcagagcgacattaccgatatcgtgtccagcctccagctgcagttcgagagtagcgaagaagccgacaagggcaacagccacagcaagaagatgctgaaggccctgctgagcgagggcgagagcatctgggagatcacagagaagatcctgaacagcttcgagtacaccagccggttcaccaagaccaagaccctgtaccagttcctgttcctggccacctttatcaactgcggccggttctccgacatcaagaacgtggaccccaagagcttcaagctggtgcagaacaagtacctgggcgtgatcattcagtgcctcgtgaccgagacaaagaccagcgtgtcccggcacatctactttttcagcgccagaggccggatcgaccccctggtgtacctggacgagttcctgagaaacagcgagcccgtgctgaagagagtgaaccggaccggcaacagcagctccaacaagcaggaataccagctgctgaaggacaacctcgtgcggtcctacaacaaggccctgaagaaaaacgccccctaccccatcttcgccattaagaacggccccaagtcccacatcggccggcacctgatgaccagctttctgagcatgaagggcctgacagagctgaccaacgtcgtgggcaattggagcgacaagagggcctctgccgtggccagaaccacctacacccaccagatcacagccatccccgaccactacttcgccctggtgtctcggtactacgcctacgaccccatcagcaaagagatgatcgccctgaaggacgagacaaaccccatcgaggaatggcagcacatcgagcagctgaagggcagcgccgagggcagcatcagataccctgcctggaacggcatcatctcccaggaagtgctggactacctgagcagctacatcaaccggcggatctgatctagacctgatcataatcaagccatatcacatctgtagaggtttacttgctttaaaaaacctccacacctccccctgaacctgaaacataaaatgaatgcaattgttgttgttaacttgtttattgcagcttataatggttacaaataaagcaatagcatcacaaatttcacaaataaagcatttttttcactgcattctagttgtggtttgtccaaactcatcaatgtatcttatcatgtctggatctgcggatccaatctcgagctgggcctcatgggccttccgctcactgcccgctttccagtcgggaaacctgtcgtgccagctgcattaacatggtcatagctgtttccttgcgtattgggcgctctccgcttcctcgctcactgactcgctgcgctcggtcgttcgggtaaagcctggggtgcctaatgagcaaaaggccagcaaaaggccaggaaccgtaaaaaggccgcgttgctggcgtttttccataggctccgcccccctgacgagcatcacaaaaatcgacgctcaagtcagaggtggcgaaacccgacaggactataaagataccaggcgtttccccctggaagctccctcgtgcgctctcctgttccgaccctgccgcttaccggatacctgtccgcctttctcccttcgggaagcgtggcgctttctcatagctcacgctgtaggtatctcagttcggtgtaggtcgttcgctccaagctgggctgtgtgcacgaaccccccgttcagcccgaccgctgcgccttatccggtaactatcgtcttgagtccaacccggtaagacacgacttatcgccactggcagcagccactggtaacaggattagcagagcgaggtatgtaggcggtgctacagagttcttgaagtggtggcctaactacggctacactagaagaacagtatttggtatctgcgctctgctgaagccagttaccttcggaaaaagagttggtagctcttgatccggcaaacaaaccaccgctggtagcggtggtttttttgtttgcaagcagcagattacgcgcagaaaaaaaggatctcaagaagatcctttgatcttttctacggggtctgacgctcagtggaacgaaaactcacgttaagggattttggtcatgagattatcaaaaaggatcttcacctagatccttttaaattaaaaatgaagttttaaatcaatctaaagtatatatgagtaaacttggtctgacagttaccaatgcttaatcagtgaggcacctatctcagcgatctgtctatttcgttcatccatagttgcctgactccccgtcgtgtagataactacgatacgggagggcttaccatctggccccagtgctgcaatgataccgcgagaaccacgctcaccggctccagatttatcagcaataaaccagccagccggaagggccgagcgcagaagtggtcctgcaactttatccgcctccatccagtctattaattgttgccgggaagctagagtaagtagttcgccagttaatagtttgcgcaacgttgttgccattgctacaggcatcgtggtgtcacgctcgtcgtttggtatggcttcattcagctccggttcccaacgatcaaggcgagttacatgatcccccatgttgtgcaaaaaagcggttagctccttcggtcctccgatcgttgtcagaagtaagttggccgcagtgttatcactcatggttatggcagcactgcataattctcttactgtcatgccatccgtaagatgcttttctgtgactggtgagtactcaaccaagtcattctgagaatagtgtatgcggcgaccgagttgctcttgcccggcgtcaatacgggataataccgcgccacatagcagaactttaaaagtgctcatcattggaaaacgttcttcggggcgaaaactctcaaggatcttaccgctgttgagatccagttcgatgtaacccactcgtgcacccaactgatcttcagcatcttttactttcaccagcgtttctgggtgagcaaaaacaggaaggcaaaatgccgcaaaaaagggaataagggcgacacggaaatgttgaatactcatactcttcctttttcaatattattgaagcatttatcagggttattgtctcatgagcggatacatatttgaatgtatttagaaaaataaacaaataggggttccgcgcacatttccccgaaaagtgccac

SEQ ID NO: 29 - DNA, 3291 bp, Artificial Sequence
  pMA-F14-TCR-JG9-alpha-F15 vector V7.A.3
acgaagttcctattccgaagttcctattcttataggagtataggaacttcctcgagctgggcctcatgggccttccgctcactgcccgctttccagtcgggaaacctgtcgtgccagctgcattaacatggtcatagctgtttccttgcgtattgggcgctctccgcttcctcgctcactgactcgctgcgctcggtcgttcgggtaaagcctggggtgcctaatgagcaaaaggccagcaaaaggccaggaaccgtaaaaaggccgcgttgctggcgtttttccataggctccgcccccctgacgagcatcacaaaaatcgacgctcaagtcagaggtggcgaaacccgacaggactataaagataccaggcgtttccccctggaagctccctcgtgcgctctcctgttccgaccctgccgcttaccggatacctgtccgcctttctcccttcgggaagcgtggcgctttctcatagctcacgctgtaggtatctcagttcggtgtaggtcgttcgctccaagctgggctgtgtgcacgaaccccccgttcagcccgaccgctgcgccttatccggtaactatcgtcttgagtccaacccggtaagacacgacttatcgccactggcagcagccactggtaacaggattagcagagcgaggtatgtaggcggtgctacagagttcttgaagtggtggcctaactacggctacactagaagaacagtatttggtatctgcgctctgctgaagccagttaccttcggaaaaagagttggtagctcttgatccggcaaacaaaccaccgctggtagcggtggtttttttgtttgcaagcagcagattacgcgcagaaaaaaaggatctcaagaagatcctttgatcttttctacggggtctgacgctcagtggaacgaaaactcacgttaagggattttggtcatgagattatcaaaaaggatcttcacctagatccttttaaattaaaaatgaagttttaaatcaatctaaagtatatatgagtaaacttggtctgacagttaccaatgcttaatcagtgaggcacctatctcagcgatctgtctatttcgttcatccatagttgcctgactccccgtcgtgtagataactacgatacgggagggcttaccatctggccccagtgctgcaatgataccgcgagaaccacgctcaccggctccagatttatcagcaataaaccagccagccggaagggccgagcgcagaagtggtcctgcaactttatccgcctccatccagtctattaattgttgccgggaagctagagtaagtagttcgccagttaatagtttgcgcaacgttgttgccattgctacaggcatcgtggtgtcacgctcgtcgtttggtatggcttcattcagctccggttcccaacgatcaaggcgagttacatgatcccccatgttgtgcaaaaaagcggttagctccttcggtcctccgatcgttgtcagaagtaagttggccgcagtgttatcactcatggttatggcagcactgcataattctcttactgtcatgccatccgtaagatgcttttctgtgactggtgagtactcaaccaagtcattctgagaatagtgtatgcggcgaccgagttgctcttgcccggcgtcaatacgggataataccgcgccacatagcagaactttaaaagtgctcatcattggaaaacgttcttcggggcgaaaactctcaaggatcttaccgctgttgagatccagttcgatgtaacccactcgtgcacccaactgatcttcagcatcttttactttcaccagcgtttctgggtgagcaaaaacaggaaggcaaaatgccgcaaaaaagggaataagggcgacacggaaatgttgaatactcatactcttcctttttcaatattattgaagcatttatcagggttattgtctcatgagcggatacatatttgaatgtatttagaaaaataaacaaataggggttccgcgcacatttccccgaaaagtgccacctaaattgtaagcgttaatattttgttaaaattcgcgttaaatttttgttaaatcagctcattttttaaccaataggccgaaatcggcaaaatcccttataaatcaaaagaatagaccgagatagggttgagtggccgctacagggcgctcccattcgccattcaggctgcgcaactgttgggaagggcgtttcggtgcgggcctcttcgctattacgccagctggcgaaagggggatgtgctgcaaggcgattaagttgggtaacgccagggttttcccagtcacgacgttgtaaaacgacggccagtgagcgcgacgtaatacgactcactatagggcgaattggcggaaggccgtcaaggccgcatgaattcgctaccgggaagttcctattccgaagttcctattctatcagaagtataggaacttcaggtacgccaccatgctccttgaacatttattaataatcttgtggatgcagctgacatgggtcagtggtcaacagctgaatcagagtcctcaatctatgtttatccaggaaggagaagatgtctccatgaactgcacttcttcaagcatatttaacacctggctatggtacaagcaggaacctggggaaggtcctgtcctcttgatagccttatataaggctggtgaattgacctcaaatggaaggctgactgctcagtttggtataaccagaaaggacagcttcctgaatatctcagcatccatacctagtgatgtaggcatctacttctgcgctggacccatgaaaacctcctacgacaaggtgatatttgggccagggacaagcttatcagtcattccaaatatccagaaccctgaccctgccgtgtaccagctgagagactctaaatccagtgacaagtctgtctgcctattcaccgattttgattctcaaacaaatgtgtcacaaagtaaggattctgatgtgtatatcacagacaaaactgtgctagacatgaggtctatggacttcaagagcaacagtgctgtggcctggagcaacaaatctgactttgcatgtgcaaacgccttcaacaacagcattattccagaggacaccttcttccccagcccagaaagttcctgtgatgtcaagctggtcgagaaaagctttgaaacagatacgaacctaaactttcaaaacctgtcagtgattgggttccgaatcctcctcctgaaagtggccgggtttaatctgctcatgacgctgcggctgtggtccagctgactag

SEQ ID NO: 30 - DNA, 3408 bp, Artificial Sequence
  pMA-FRT-TCR-JG9-beta-F3 vector V7.A.4
ctaaattgtaagcgttaatattttgttaaaattcgcgttaaatttttgttaaatcagctcattttttaaccaataggccgaaatcggcaaaatcccttataaatcaaaagaatagaccgagatagggttgagtggccgctacagggcgctcccattcgccattcaggctgcgcaactgttgggaagggcgtttcggtgcgggcctcttcgctattacgccagctggcgaaagggggatgtgctgcaaggcgattaagttgggtaacgccagggttttcccagtcacgacgttgtaaaacgacggccagtgagcgcgacgtaatacgactcactatagggcgaattggcggaaggccgtcaaggccgcatgaattcgctaccgggaagttcctattccgaagttcctattctctagaaagtataggaacttcaggtacgccaccatggactcctggaccctctgctgtgtgtccctttgcatcctggtagcaaagcacacagatgctggagttatccagtcaccccggcacgaggtgacagagatgggacaagaagtgactctgagatgtaaaccaatttcaggacacgactaccttttctggtacagacagaccatgatgcggggactggagttgctcatttactttaacaacaacgttccgatagatgattcagggatgcccgaggatcgattctcagctaagatgcctaatgcatcattctccactctgaagatccagccctcagaacccagggactcagctgtgtacttttgcgccagcagttccgcaaactatggctacacctttggttcggggaccaggttaaccgttgtagaggacctgaacaaggtgttcccacccgaggtcgctgtgtttgagccatcagaagcagagatctcccacacccaaaaggccacactggtatgcctggccacaggcttctaccccgaccacgtggagctgagctggtgggtgaatgggaaggaggtgcacagtggggtcagcacagacccgcagcccctcaaggagcagcccgccctcaatgactccagatactgcctgagcagccgcctgagggtgtcggccaccttctggcagaacccccgcaaccacttccgctgtcaagtccagttctacgggctctcggagaatgacgagtggacccaggatagggccaaacccgtcacccagatcgtcagcgccgaggcctggggtagagcagactgtggcttcacctccgagtcttaccagcaaggggtcctgtctgccaccatcctctatgagatcttgctagggaaggccaccttgtatgccgtgctggtcagtgccctcgtgctgatggccatggtcaagagaaaggattccagaggctagctagacgaagttcctattccgaagttcctattcttcaaatagtataggaacttcctcgagctgggcctcatgggccttccgctcactgcccgctttccagtcgggaaacctgtcgtgccagctgcattaacatggtcatagctgtttccttgcgtattgggcgctctccgcttcctcgctcactgactcgctgcgctcggtcgttcgggtaaagcctggggtgcctaatgagcaaaaggccagcaaaaggccaggaaccgtaaaaaggccgcgttgctggcgtttttccataggctccgcccccctgacgagcatcacaaaaatcgacgctcaagtcagaggtggcgaaacccgacaggactataaagataccaggcgtttccccctggaagctccctcgtgcgctctcctgttccgaccctgccgcttaccggatacctgtccgcctttctcccttcgggaagcgtggcgctttctcatagctcacgctgtaggtatctcagttcggtgtaggtcgttcgctccaagctgggctgtgtgcacgaaccccccgttcagcccgaccgctgcgccttatccggtaactatcgtcttgagtccaacccggtaagacacgacttatcgccactggcagcagccactggtaacaggattagcagagcgaggtatgtaggcggtgctacagagttcttgaagtggtggcctaactacggctacactagaagaacagtatttggtatctgcgctctgctgaagccagttaccttcggaaaaagagttggtagctcttgatccggcaaacaaaccaccgctggtagcggtggtttttttgtttgcaagcagcagattacgcgcagaaaaaaaggatctcaagaagatcctttgatcttttctacggggtctgacgctcagtggaacgaaaactcacgttaagggattttggtcatgagattatcaaaaaggatcttcacctagatccttttaaattaaaaatgaagttttaaatcaatctaaagtatatatgagtaaacttggtctgacagttaccaatgcttaatcagtgaggcacctatctcagcgatctgtctatttcgttcatccatagttgcctgactccccgtcgtgtagataactacgatacgggagggcttaccatctggccccagtgctgcaatgataccgcgagaaccacgctcaccggctccagatttatcagcaataaaccagccagccggaagggccgagcgcagaagtggtcctgcaactttatccgcctccatccagtctattaattgttgccgggaagctagagtaagtagttcgccagttaatagtttgcgcaacgttgttgccattgctacaggcatcgtggtgtcacgctcgtcgtttggtatggcttcattcagctccggttcccaacgatcaaggcgagttacatgatcccccatgttgtgcaaaaaagcggttagctccttcggtcctccgatcgttgtcagaagtaagttggccgcagtgttatcactcatggttatggcagcactgcataattctcttactgtcatgccatccgtaagatgcttttctgtgactggtgagtactcaaccaagtcattctgagaatagtgtatgcggcgaccgagttgctcttgcccggcgtcaatacgggataataccgcgccacatagcagaactttaaaagtgctcatcattggaaaacgttcttcggggcgaaaactctcaaggatcttaccgctgttgagatccagttcgatgtaacccactcgtgcacccaactgatcttcagcatcttttactttcaccagcgtttctgggtgagcaaaaacaggaaggcaaaatgccgcaaaaaagggaataagggcgacacggaaatgttgaatactcatactcttcctttttcaatattattgaagcatttatcagggttattgtctcatgagcggatacatatttgaatgtatttagaaaaataaacaaataggggttccgcgcacatttccccgaaaagtgccac

SEQ ID NO: 31 - DNA, 3291 bp, Artificial Sequence
  F14-TCRaF15 CDR3degen.64mix vector V8.F.8
  variation 2803: /replace="n"= "a", "g", "c", or "t"
  variation 2808: /replace="n"= "a", "g", "c", or "t"
  variation 2814: /replace="n"= "a", "g", "c", or "t"
acgaagttcctattccgaagttcctattcttataggagtataggaacttcctcgagctgggcctcatgggccttccgctcactgcccgctttccagtcgggaaacctgtcgtgccagctgcattaacatggtcatagctgtttccttgcgtattgggcgctctccgcttcctcgctcactgactcgctgcgctcggtcgttcgggtaaagcctggggtgcctaatgagcaaaaggccagcaaaaggccaggaaccgtaaaaaggccgcgttgctggcgtttttccataggctccgcccccctgacgagcatcacaaaaatcgacgctcaagtcagaggtggcgaaacccgacaggactataaagataccaggcgtttccccctggaagctccctcgtgcgctctcctgttccgaccctgccgcttaccggatacctgtccgcctttctcccttcgggaagcgtggcgctttctcatagctcacgctgtaggtatctcagttcggtgtaggtcgttcgctccaagctgggctgtgtgcacgaaccccccgttcagcccgaccgctgcgccttatccggtaactatcgtcttgagtccaacccggtaagacacgacttatcgccactggcagcagccactggtaacaggattagcagagcgaggtatgtaggcggtgctacagagttcttgaagtggtggcctaactacggctacactagaagaacagtatttggtatctgcgctctgctgaagccagttaccttcggaaaaagagttggtagctcttgatccggcaaacaaaccaccgctggtagcggtggtttttttgtttgcaagcagcagattacgcgcagaaaaaaaggatctcaagaagatcctttgatcttttctacggggtctgacgctcagtggaacgaaaactcacgttaagggattttggtcatgagattatcaaaaaggatcttcacctagatccttttaaattaaaaatgaagttttaaatcaatctaaagtatatatgagtaaacttggtctgacagttaccaatgcttaatcagtgaggcacctatctcagcgatctgtctatttcgttcatccatagttgcctgactccccgtcgtgtagataactacgatacgggagggcttaccatctggccccagtgctgcaatgataccgcgagaaccacgctcaccggctccagatttatcagcaataaaccagccagccggaagggccgagcgcagaagtggtcctgcaactttatccgcctccatccagtctattaattgttgccgggaagctagagtaagtagttcgccagttaatagtttgcgcaacgttgttgccattgctacaggcatcgtggtgtcacgctcgtcgtttggtatggcttcattcagctccggttcccaacgatcaaggcgagttacatgatcccccatgttgtgcaaaaaagcggttagctccttcggtcctccgatcgttgtcagaagtaagttggccgcagtgttatcactcatggttatggcagcactgcataattctcttactgtcatgccatccgtaagatgcttttctgtgactggtgagtactcaaccaagtcattctgagaatagtgtatgcggcgaccgagttgctcttgcccggcgtcaatacgggataataccgcgccacatagcagaactttaaaagtgctcatcattggaaaacgttcttcggggcgaaaactctcaaggatcttaccgctgttgagatccagttcgatgtaacccactcgtgcacccaactgatcttcagcatcttttactttcaccagcgtttctgggtgagcaaaaacaggaaggcaaaatgccgcaaaaaagggaataagggcgacacggaaatgttgaatactcatactcttcctttttcaatattattgaagcatttatcagggttattgtctcatgagcggatacatatttgaatgtatttagaaaaataaacaaataggggttccgcgcacatttccccgaaaagtgccacctaaattgtaagcgttaatattttgttaaaattcgcgttaaatttttgttaaatcagctcattttttaaccaataggccgaaatcggcaaaatcccttataaatcaaaagaatagaccgagatagggttgagtggccgctacagggcgctcccattcgccattcaggctgcgcaactgttgggaagggcgtttcggtgcgggcctcttcgctattacgccagctggcgaaagggggatgtgctgcaaggcgattaagttgggtaacgccagggttttcccagtcacgacgttgtaaaacgacggccagtgagcgcgacgtaatacgactcactatagggcgaattggcggaaggccgtcaaggccgcatgaattcgctaccgggaagttcctattccgaagttcctattctatcagaagtataggaacttcaggtacgccaccatgctccttgaacatttattaataatcttgtggatgcagctgacatgggtcagtggtcaacagctgaatcagagtcctcaatctatgtttatccaggaaggagaagatgtctccatgaactgcacttcttcaagcatatttaacacctggctatggtacaagcaggaacctggggaaggtcctgtcctcttgatagccttatataaggctggtgaattgacctcaaatggaaggctgactgctcagtttggtataaccagaaaggacagcttcctgaatatctcagcatccatacctagtgatgtaggcatctacttctgcgctggacccangaaancctccnacgacaaggtgatatttgggccagggacaagcttatcagtcattccaaatatccagaaccctgaccctgccgtgtaccagctgagagactctaaatccagtgacaagtctgtctgcctattcaccgattttgattctcaaacaaatgtgtcacaaagtaaggattctgatgtgtatatcacagacaaaactgtgctagacatgaggtctatggacttcaagagcaacagtgctgtggcctggagcaacaaatctgactttgcatgtgcaaacgccttcaacaacagcattattccagaggacaccttcttccccagcccagaaagttcctgtgatgtcaagctggtcgagaaaagctttgaaacagatacgaacctaaactttcaaaacctgtcagtgattgggttccgaatcctcctcctgaaagtggccgggtttaatctgctcatgacgctgcggctgtggtccagctgactag

SEQ ID NO: 32 - DNA, 4030 bp, Artificial Sequence
  JG9-TRA CDR3 64 variants vectors backbone VP.7751.RC1-A1 to H8
cggggtctgacgctcagtggaacgaaaactcacgttaagggattttggtcatgagattatcaaaaaggatcttcacctagatccttttaaattaaaaatgaagttttaaatcaatctaaagtatatatgagtaaacttggtctgacagttaccaatgcttaatcagtgaggcacctatctcagcgatctgtctatttcgttcatccatagttgcctgactccccgtcgtgtagataactacgatacgggagggcttaccatctggccccagtgctgcaatgataccgcgagaaccacgctcaccggctccagatttatcagcaataaaccagccagccggaagggccgagcgcagaagtggtcctgcaactttatccgcctccatccagtctattaattgttgccgggaagctagagtaagtagttcgccagttaatagtttgcgcaacgttgttgccattgctacaggcatcgtggtgtcacgctcgtcgtttggtatggcttcattcagctccggttcccaacgatcaaggcgagttacatgatcccccatgttgtgcaaaaaagcggttagctccttcggtcctccgatcgttgtcagaagtaagttggccgcagtgttatcactcatggttatggcagcactgcataattctcttactgtcatgccatccgtaagatgcttttctgtgactggtgagtactcaaccaagtcattctgagaatagtgtatgcggcgaccgagttgctcttgcccggcgtcaatacgggataataccgcgccacatagcagaactttaaaagtgctcatcattggaaaacgttcttcggggcgaaaactctcaaggatcttaccgctgttgagatccagttcgatgtaacccactcgtgcacccaactgatcttcagcatcttttactttcaccagcgtttctgggtgagcaaaaacaggaaggcaaaatgccgcaaaaaagggaataagggcgacacggaaatgttgaatactcatactcttcctttttcaatattattgaagcatttatcagggttattgtctcatgagcggatacatatttgaatgtatttagaaaaataaacaaataggggttccgcgcacatttccccgaaaagtgccacctaaattgtaagcgttaatattttgttaaaattcgcgttaaatttttgttaaatcagctcattttttaaccaataggccgaaatcggcaaaatcccttataaatcaaaagaatagaccgagatagggttgagtggccgctacagggcgctcccattcgccattcaggctgcgcaactgttgggaagggcgtttcggtgcgggcctcttcgctattacgccagctggcgaaagggggatgtgctgcaaggcgattaagttgggtaacgccagggttttcccagtcacgacgttgtaaaacgacggccagtgagcgcgacgtaatacgactcactatagggcgaattggcggaaggccgtcaaggccgcatgaattcgctaccggtatagtaatcaattacggggtcattagttcatagcccatatatggagttccgcgttacataacttacggtaaatggcccgcctggctgaccgcccaacgacccccgcccattgacgtcaataatgacgtatgttcccatagtaacgccaatagggactttccattgacgtcaatgggtggagtatttacggtaaactgcccacttggcagtacatcaagtgtatcatatgccaagtacgccccctattgacgtcaatgacggtaaatggcccgcctggcattatgcccagtacatgaccttatgggactttcctacttggcagtacatctacgtattagtcatcgctattaccatggtgatgcggttttggcagtacatcaatgggcgtggatagcggtttgactcacggggatttccaagtctccaccccattgacgtcaatgggagtttgttttggcaccaaaatcaacgggactttccaaaatgtcgtaacaactccgccccattgacgcaaatgggcggtaggcgtgtacggtgggaggtctatataagcagagctggtttagtgaaccgtcagatcaggtacgccaccatgctccttgaacatttattaataatcttgtggatgcagctgacatgggtcagtggtcaacagctgaatcagagtcctcaatctatgtttatccaggaaggagaagatgtctccatgaactgcacttcttcaagcatatttaacacctggctatggtacaagcaggaacctggggaaggtcctgtcctcttgatagccttatataaggctggtgaattgacctcaaatggaaggctgactgctcagtttggtataaccagaaaggacagcttcctgaatatctcagcatccatacctagtgatgtaggcatctacttctgcgctggacccatgaaaacctcctacgacaaggtgatatttgggccagggacaagcttatcagtcattccaaatatccagaaccctgaccctgccgtgtaccagctgagagactctaaatccagtgacaagtctgtctgcctattcaccgattttgattctcaaacaaatgtgtcacaaagtaaggattctgatgtgtatatcacagacaaaactgtgctagacatgaggtctatggacttcaagagcaacagtgctgtggcctggagcaacaaatctgactttgcatgtgcaaacgccttcaacaacagcattattccagaggacaccttcttccccagcccagaaagttcctgtgatgtcaagctggtcgagaaaagctttgaaacagatacgaacctaaactttcaaaacctgtcagtgattgggttccgaatcctcctcctgaaagtggccgggtttaatctgctcatgacgctgcggctgtggtccagctgactagacctgatcataatcaagccatatcacatctgtagaggtttacttgctttaaaaaacctccacacctccccctgaacctgaaacataaaatgaatgcaattgttgttgttaacttgtttattgcagcttataatggttacaaataaagcaatagcatcacaaatttcacaaataaagcatttttttcactgcattctagttgtggtttgtccaaactcatcaatgtatcttatcatgtctggatctgcggatccaatctcgagctgggcctcatgggccttccgctcactgcccgctttccagtcgggaaacctgtcgtgccagctgcattaacatggtcatagctgtttccttgcgtattgggcgctctccgcttcctcgctcactgactcgctgcgctcggtcgttcgggtaaagcctggggtgcctaatgagcaaaaggccagcaaaaggccaggaaccgtaaaaaggccgcgttgctggcgtttttccataggctccgcccccctgacgagcatcacaaaaatcgacgctcaagtcagaggtggcgaaacccgacaggactataaagataccaggcgtttccccctggaagctccctcgtgcgctctcctgttccgaccctgccgcttaccggatacctgtccgcctttctcccttcgggaagcgtggcgctttctcatagctcacgctgtaggtatctcagttcggtgtaggtcgttcgctccaagctgggctgtgtgcacgaaccccccgttcagcccgaccgctgcgccttatccggtaactatcgtcttgagtccaacccggtaagacacgacttatcgccactggcagcagccactggtaacaggattagcagagcgaggtatgtaggcggtgctacagagttcttgaagtggtggcctaactacggctacactagaagaacagtatttggtatctgcgctctgctgaagccagttaccttcggaaaaagagttggtagctcttgatccggcaaacaaaccaccgctggtagcggtggtttttttgtttgcaagcagcagattacgcgcagaaaaaaaggatctcaagaagatcctttgatcttttcta

SEQ ID NO: 33 - DNA, 42 bp, Artificial Sequence
  CDR3 sequence of a JG9-TRA 64 variant VP.7751.RC1_A1
tgcgctggacccaagaaaacctccaacgacaaggtgatattt

SEQ ID NO: 34 - DNA, 42 bp, Artificial Sequence
  CDR3 sequence of a JG9-TRA 64 variant VP.7751.RC1_A2
tgcgctggacccaagaaaacctcccacgacaaggtgatattt

SEQ ID NO: 35 - DNA, 42 bp, Artificial Sequence
  CDR3 sequence of a JG9-TRA 64 variant VP.7751.RC1_A3
tgcgctggacccaagaaaacctccgacgacaaggtgatattt

SEQ ID NO: 36 - DNA, 42 bp, Artificial Sequence
  CDR3 sequence of a JG9-TRA 64 variant VP.7751.RC1_A4
tgcgctggacccaagaaaacctcctacgacaaggtgatattt

SEQ ID NO: 37 - DNA, 42 bp, Artificial Sequence
  CDR3 sequence of a JG9-TRA 64 variant VP.7751.RC1_A5
tgcgctggacccaagaaaccctccaacgacaaggtgatattt

SEQ ID NO: 38 - DNA, 42 bp, Artificial Sequence
  CDR3 sequence of a JG9-TRA 64 variant VP.7751.RC1_A6
tgcgctggacccaagaaaccctcccacgacaaggtgatattt

SEQ ID NO: 39 - DNA, 42 bp, Artificial Sequence
  CDR3 sequence of a JG9-TRA 64 variant VP.7751.RC1_A7
tgcgctggacccaagaaaccctccgacgacaaggtgatattt

SEQ ID NO: 40 - DNA, 42 bp, Artificial Sequence
  CDR3 sequence of a JG9-TRA 64 variant VP.7751.RC1_A8
tgcgctggacccaagaaaccctcctacgacaaggtgatattt

SEQ ID NO: 41 - DNA, 42 bp, Artificial Sequence
  CDR3 sequence of a JG9-TRA 64 variant VP.7751.RC1_B1
tgcgctggacccaagaaagcctccaacgacaaggtgatattt

SEQ ID NO: 42 - DNA, 42 bp, Artificial Sequence
  CDR3 sequence of a JG9-TRA 64 variant VP.7751.RC1_B2
tgcgctggacccaagaaagcctcccacgacaaggtgatattt

SEQ ID NO: 43 - DNA, 42 bp, Artificial Sequence
  CDR3 sequence of a JG9-TRA 64 variant VP.7751.RC1_B3
tgcgctggacccaagaaagcctccgacgacaaggtgatattt

SEQ ID NO: 44 - DNA, 42 bp, Artificial Sequence
  CDR3 sequence of a JG9-TRA 64 variant VP.7751.RC1_B4
tgcgctggacccaagaaagcctcctacgacaaggtgatattt

SEQ ID NO: 45 - DNA, 42 bp, Artificial Sequence
  CDR3 sequence of a JG9-TRA 64 variant VP.7751.RC1_B5
tgcgctggacccaagaaatcctccaacgacaaggtgatattt

SEQ ID NO: 46 - DNA, 42 bp, Artificial Sequence
  CDR3 sequence of a JG9-TRA 64 variant VP.7751.RC1_B6
tgcgctggacccaagaaatcctcccacgacaaggtgatattt

SEQ ID NO: 47 - DNA, 42 bp, Artificial Sequence
  CDR3 sequence of a JG9-TRA 64 variant VP.7751.RC1_B7
tgcgctggacccaagaaatcctccgacgacaaggtgatattt

SEQ ID NO: 48 - DNA, 42 bp, Artificial Sequence
  CDR3 sequence of a JG9-TRA 64 variant VP.7751.RC1_B8
tgcgctggacccaagaaatcctcctacgacaaggtgatattt

SEQ ID NO: 49 - DNA, 42 bp, Artificial Sequence
  CDR3 sequence of a JG9-TRA 64 variant VP.7751.RC1_C1
tgcgctggacccacgaaaacctccaacgacaaggtgatattt

SEQ ID NO: 50 - DNA, 42 bp, Artificial Sequence
  CDR3 sequence of a JG9-TRA 64 variant VP.7751.RC1_C2
tgcgctggacccacgaaaacctcccacgacaaggtgatattt

SEQ ID NO: 51 - DNA, 42 bp, Artificial Sequence
  CDR3 sequence of a JG9-TRA 64 variant VP.7751.RC1_C3
tgcgctggacccacgaaaacctccgacgacaaggtgatattt

SEQ ID NO: 52 - DNA, 42 bp, Artificial Sequence
  CDR3 sequence of a JG9-TRA 64 variant VP.7751.RC1_C4
tgcgctggacccacgaaaacctcctacgacaaggtgatattt

SEQ ID NO: 53 - DNA, 42 bp, Artificial Sequence
  CDR3 sequence of a JG9-TRA 64 variant VP.7751.RC1_C5
tgcgctggacccacgaaaccctccaacgacaaggtgatattt

SEQ ID NO: 54 - DNA, 42 bp, Artificial Sequence
  CDR3 sequence of a JG9-TRA 64 variant VP.7751.RC1_C6
tgcgctggacccacgaaaccctcccacgacaaggtgatattt

SEQ ID NO: 55 - DNA, 42 bp, Artificial Sequence
  CDR3 sequence of a JG9-TRA 64 variant VP.7751.RC1_C7
tgcgctggacccacgaaaccctcctacgacaaggtgatattt

SEQ ID NO: 56 - DNA, 42 bp, Artificial Sequence
  CDR3 sequence of a JG9-TRA 64 variant VP.7751.RC1_D1
tgcgctggacccacgaaagcctccaacgacaaggtgatattt

SEQ ID NO: 57 - DNA, 42 bp, Artificial Sequence
  CDR3 sequence of a JG9-TRA 64 variant VP.7751.RC1_D2
tgcgctggacccacgaaagcctcccacgacaaggtgatattt

SEQ ID NO: 58 - DNA, 42 bp, Artificial Sequence
  CDR3 sequence of a JG9-TRA 64 variant VP.7751.RC1_D3
tgcgctggacccacgaaagcctccgacgacaaggtgatattt

SEQ ID NO: 59 - DNA, 42 bp, Artificial Sequence
  CDR3 sequence of a JG9-TRA 64 variant VP.7751.RC1_D4
tgcgctggacccacgaaagcctcctacgacaaggtgatattt

SEQ ID NO: 60 - DNA, 42 bp, Artificial Sequence
  CDR3 sequence of a JG9-TRA 64 variant VP.7751.RC1_D5
tgcgctggacccacgaaatcctccaacgacaaggtgatattt

SEQ ID NO: 61 - DNA, 42 bp, Artificial Sequence
  CDR3 sequence of a JG9-TRA 64 variant VP.7751.RC1_D6
tgcgctggacccacgaaatcctcccacgacaaggtgatattt

SEQ ID NO: 62 - DNA, 42 bp, Artificial Sequence
  CDR3 sequence of a JG9-TRA 64 variant VP.7751.RC1_D7
tgcgctggacccacgaaatcctccgacgacaaggtgatattt

SEQ ID NO: 63 - DNA, 42 bp, Artificial Sequence
  CDR3 sequence of a JG9-TRA 64 variant VP.7751.RC1_D8
tgcgctggacccacgaaatcctcctacgacaaggtgatattt

SEQ ID NO: 64 - DNA, 42 bp, Artificial Sequence
  CDR3 sequence of a JG9-TRA 64 variant VP.7751.RC1_E1
tgcgctggacccaggaaaacctccaacgacaaggtgatattt

SEQ ID NO: 65 - DNA, 42 bp, Artificial Sequence
  CDR3 sequence of a JG9-TRA 64 variant VP.7751.RC1_E2
tgcgctggacccaggaaaacctcccacgacaaggtgatattt

SEQ ID NO: 66 - DNA, 42 bp, Artificial Sequence
  CDR3 sequence of a JG9-TRA 64 variant VP.7751.RC1_E3
tgcgctggacccaggaaaacctccgacgacaaggtgatattt

SEQ ID NO: 67 - DNA, 42 bp, Artificial Sequence
  CDR3 sequence of a JG9-TRA 64 variant VP.7751.RC1_E4
tgcgctggacccaggaaaacctcctacgacaaggtgatattt

SEQ ID NO: 68 - DNA, 42 bp, Artificial Sequence
  CDR3 sequence of a JG9-TRA 64 variant VP.7751.RC1_E5
tgcgctggacccaggaaaccctccaacgacaaggtgatattt

SEQ ID NO: 69 - DNA, 42 bp, Artificial Sequence
  CDR3 sequence of a JG9-TRA 64 variant VP.7751.RC1_E6
tgcgctggacccaggaaaccctcccacgacaaggtgatattt

SEQ ID NO: 70 - DNA, 42 bp, Artificial Sequence
  CDR3 sequence of a JG9-TRA 64 variant VP.7751.RC1_E7
tgcgctggacccaggaaaccctccgacgacaaggtgatattt

SEQ ID NO: 71 - protein, 42 aa, Artificial Sequence
  CDR3 sequence of a JG9-TRA 64 variant VP.7751.RC1_E8
TGCGCTGGACCCAGGAAACCCTCCTACGACAAGGTGATATTT

SEQ ID NO: 72 - DNA, 42 bp, Artificial Sequence
  CDR3 sequence of a JG9-TRA 64 variant VP.7751.RC1_F1
tgcgctggacccaggaaagcctccaacgacaaggtgatattt

SEQ ID NO: 73 - DNA, 42 bp, Artificial Sequence
  CDR3 sequence of a JG9-TRA 64 variant VP.7751.RC1_F2
tgcgctggacccaggaaagcctcccacgacaaggtgatattt

SEQ ID NO: 74 - DNA, 42 bp, Artificial Sequence
  CDR3 sequence of a JG9-TRA 64 variant VP.7751.RC1_F3
tgcgctggacccaggaaagcctccgacgacaaggtgatattt

SEQ ID NO: 75 - DNA, 42 bp, Artificial Sequence
  CDR3 sequence of a JG9-TRA 64 variant VP.7751.RC1_F4
tgcgctggacccaggaaagcctcctacgacaaggtgatattt

SEQ ID NO: 76 - DNA, 42 bp, Artificial Sequence
  CDR3 sequence of a JG9-TRA 64 variant VP.7751.RC1_F5
tgcgctggacccaggaaatcctccaacgacaaggtgatattt

SEQ ID NO: 77 - DNA, 42 bp, Artificial Sequence
  CDR3 sequence of a JG9-TRA 64 variant VP.7751.RC1_F6
tgcgctggacccaggaaatcctcccacgacaaggtgatattt

SEQ ID NO: 78 - DNA, 42 bp, Artificial Sequence
  CDR3 sequence of a JG9-TRA 64 variant VP.7751.RC1_F7
tgcgctggacccaggaaatcctccgacgacaaggtgatattt

SEQ ID NO: 79 - DNA, 42 bp, Artificial Sequence
  CDR3 sequence of a JG9-TRA 64 variant VP.7751.RC1_F8
tgcgctggacccaggaaatcctcctacgacaaggtgatattt

SEQ ID NO: 80 - DNA, 42 bp, Artificial Sequence
  CDR3 sequence of a JG9-TRA 64 variant VP.7751.RC1_G1
tgcgctggacccatgaaaacctccaacgacaaggtgatattt

SEQ ID NO: 81 - DNA, 42 bp, Artificial Sequence
  CDR3 sequence of a JG9-TRA 64 variant VP.7751.RC1_G2
tgcgctggacccatgaaaacctcccacgacaaggtgatattt

SEQ ID NO: 82 - DNA, 42 bp, Artificial Sequence
  CDR3 sequence of a JG9-TRA 64 variant VP.7751.RC1_G3
tgcgctggacccatgaaaacctccgacgacaaggtgatattt

SEQ ID NO: 83 - DNA, 42 bp, Artificial Sequence
  CDR3 sequence of a JG9-TRA 64 variant VP.7751.RC1_G4
tgcgctggacccatgaaaacctcctacgacaaggtgatattt

SEQ ID NO: 84 - DNA, 42 bp, Artificial Sequence
  CDR3 sequence of a JG9-TRA 64 variant VP.7751.RC1_G5
tgcgctggacccatgaaaccctccaacgacaaggtgatattt

SEQ ID NO: 85 - DNA, 42 bp, Artificial Sequence
  CDR3 sequence of a JG9-TRA 64 variant VP.7751.RC1_G6
tgcgctggacccatgaaaccctcccacgacaaggtgatattt

SEQ ID NO: 86 - DNA, 42 bp, Artificial Sequence
  CDR3 sequence of a JG9-TRA 64 variant VP.7751.RC1_G7
tgcgctggacccatgaaaccctccgacgacaaggtgatattt

SEQ ID NO: 87 - DNA, 42 bp, Artificial Sequence
  CDR3 sequence of a JG9-TRA 64 variant VP.7751.RC1_G8
tgcgctggacccatgaaaccctcctacgacaaggtgatattt

SEQ ID NO: 88 - DNA, 42 bp, Artificial Sequence
  CDR3 sequence of a JG9-TRA 64 variant VP.7751.RC1_H1
tgcgctggacccatgaaagcctccaacgacaaggtgatattt

SEQ ID NO: 89 - DNA, 42 bp, Artificial Sequence
  CDR3 sequence of a JG9-TRA 64 variant VP.7751.RC1_H2
tgcgctggacccatgaaagcctcccacgacaaggtgatattt

SEQ ID NO: 90 - DNA, 42 bp, Artificial Sequence
  CDR3 sequence of a JG9-TRA 64 variant VP.7751.RC1_H3
tgcgctggacccatgaaagcctccgacgacaaggtgatattt

SEQ ID NO: 91 - DNA, 42 bp, Artificial Sequence
  CDR3 sequence of a JG9-TRA 64 variant VP.7751.RC1_H4
tgcgctggacccatgaaagcctcctacgacaaggtgatattt

SEQ ID NO: 92 - DNA, 42 bp, Artificial Sequence
  CDR3 sequence of a JG9-TRA 64 variant VP.7751.RC1_H5
tgcgctggacccatgaaatcctccaacgacaaggtgatattt

SEQ ID NO: 93 - DNA, 42 bp, Artificial Sequence
  CDR3 sequence of a JG9-TRA 64 variant VP.7751.RC1_H6
tgcgctggacccatgaaatcctcccacgacaaggtgatattt

SEQ ID NO: 94 - DNA, 42 bp, Artificial Sequence
  CDR3 sequence of a JG9-TRA 64 variant VP.7751.RC1_H7
tgcgctggacccatgaaatcctccgacgacaaggtgatattt

SEQ ID NO: 95 - DNA, 42 bp, Artificial Sequence
  CDR3 sequence of a JG9-TRA 64 variant VP.7751.RC1_H8
tgcgctggacccatgaaatcctcctacgacaaggtgatattt

SEQ ID NO: 96 - DNA, 25 bp, Artificial Sequence
  pMA-sv40_OE_F1primer 1.C.2
cctgatcataatcaagccatatcac

SEQ ID NO: 97 - DNA, 25 bp, Artificial Sequence
  pMA-sv40_OE_R1 primer 1.C.3
gtgatatggcttgattatgatcagg

SEQ ID NO: 98 - DNA, 21 bp, Artificial Sequence
  pMA-CMV_OE_R1 primer 1.C.5
gtacctgatctgacggttcac

SEQ ID NO: 99 - DNA, 20 bp, Artificial Sequence
  HLA-A-GT-Rg3 primer 4.A.3
tcccgttctccaggtatctg

SEQ ID NO: 100 - DNA, 20 bp, Artificial Sequence
  HLA-A-GT-Fg2 primer 4.A.4
gtgtcgggtttccagagaag

SEQ ID NO: 101 - DNA, 20 bp, Artificial Sequence
  HLA-B-GT-Fg2 primer 4.A.7
gggtcccagttctaaagtcc

SEQ ID NO: 102 - DNA, 20 bp, Artificial Sequence
  HLA-B-GT-Rg2 primer 4.B.1
ggggattttggcctcaactg

SEQ ID NO: 103 - DNA, 21 bp, Artificial Sequence
  HLA-C-GT-Fg2 primer 4.B.5
tcttcctgaatactcatgacg

SEQ ID NO: 104 - DNA, 20 bp, Artificial Sequence
  HLA-A-02_GT_Rg4 primer 4.I.9
ggagatctacaggcgatcag

SEQ ID NO: 105 - DNA, 28 bp, Artificial Sequence
  HLA-A-Exon3_HA-RE-BglII_F1 primer 6.I.9
ggttagatctgggaaggagacgctgcag

SEQ ID NO: 106 - DNA, 20 bp, Artificial Sequence
  HLA-C-04-GT-Rg1 primer 8.A.1
gatcccattttcctcccctc

SEQ ID NO: 107 - DNA, 27 bp, Artificial Sequence
  CMV-pA-HLA-Ex3_Probe_F1 primer 8.B.2
atgtctggatctgcggatcagcgcacg

SEQ ID NO: 108 - DNA, 21 bp, Artificial Sequence
  CMV-pro_GT_R1 primer 9.C.3
atgggctatgaactaatgacc

SEQ ID NO: 109 - DNA, 21 bp, Artificial Sequence
  sv40pA_GT_F1 primer 9.C.4
cattctagttgtggtttgtcc

SEQ ID NO: 110 - DNA, 20 bp, Artificial Sequence
  AAVS1_GT_F1 primer 9.C.5
cttacctctctagtctgtgc

SEQ ID NO: 111 - DNA, 19 bp, Artificial Sequence
  AAVS1_GT_F3 primer 9.C.7
ccattgtcactttgcgctg

SEQ ID NO: 112 - DNA, 20 bp, Artificial Sequence
  AAVS1_GT_F4 primer 9.C.8
tcctggactttgtctccttc

SEQ ID NO: 113 - DNA, 20 bp, Artificial Sequence
  AAVS1_GT_R2 primer 9.C.10
agagatggctccaggaaatg

SEQ ID NO: 114 - DNA, 20 bp, Artificial Sequence
  AAVS1_GT_R3 promer 9.D.1
aagagaaagggagtagaggc

SEQ ID NO: 115 - DNA, 18 bp, Artificial Sequence
  AAVS1_GT_R4 primer 9.D.2
cccgaagagtgagtttgc

SEQ ID NO: 116 - DNA, 20 bp, Artificial Sequence
  HLA-A-intron4_GT_R1 primer 9.D.6
gctaaaggtcagagaggctc

SEQ ID NO: 117 - DNA, 23 bp, Artificial Sequence
  sv40pA-GT-F2 primer 9.D.7
ctgcattctagttgtggtttgtc

SEQ ID NO: 118 - DNA, 24 bp, Artificial Sequence
  sv40pA-AAVS1-probe-FAM-F1 primer 9.J.2
tgcggatcaggattggtgacagaa

SEQ ID NO: 119 - DNA, 26 bp, Artificial Sequence
  TRAC_TCRA-ex1_R1 primer 10.A.9
gacttgtcactggatttagagtctct

SEQ ID NO: 120 - DNA, 23 bp, Artificial Sequence
  TRAC_TCRA-promoter_F1 primer 10.A.10
ctgatcctcttgtcccacagata

SEQ ID NO: 121 - DNA, 22 bp, Artificial Sequence
  TRAC_probe (HEX) primer 10.B.6
atccagaaccctgaccctgccg

SEQ ID NO: 122 - DNA, 19 bp, Artificial Sequence
  TRAC-GT-F1 primer 1.F.7
atgtgcaaacgccttcaac

SEQ ID NO: 123 - DNA, 24 bp, Artificial Sequence
  sv40pA GT-R1 primer 15.H.2
cctctacagatgtgatatggcttg

SEQ ID NO: 124 - DNA, 21 bp, Artificial Sequence
  TRBC2-GT-F1 primer 1.F.9
gctgtcaagtccagttctacg

SEQ ID NO: 125 - DNA, 20 bp, Artificial Sequence
  tGFP-Cterm-Out_SQ_F1 primer 3.J.5
gaagaggaccacagcaacac

SEQ ID NO: 126 - DNA, 19 bp, Artificial Sequence
  TRAC-GT-F1 ddPCR primer/probe
atgtgcaaacgccttcaac

SEQ ID NO: 127 - DNA, 20 bp, Artificial Sequence
  TRAC-GT-R1 ddPCR primer/probe 1.F.8
ttcggaacccaatcactgac

SEQ ID NO: 128 - DNA, 26 bp, Artificial Sequence
  TRAC-probe-FAM ddPCR primer/probe
tttctcgaccagcttgacatcacagg

SEQ ID NO: 129 - DNA, 21 bp, Artificial Sequence
  TRBC2-GT-F1 ddPCR primer/probe 1.F.9
gctgtcaagtccagttctacg

SEQ ID NO: 130 - DNA, 20 bp, Artificial Sequence
  TRBC2-GT-R1 ddPCR primer/probe 1.F.10
cttgctggtaagactcggag

SEQ ID NO: 131 - DNA, 23 bp, Artificial Sequence
  TRBC2-probe-FAM ddPCR primer/probe 1.G.2
caaacccgtcacccagatcgtca

SEQ ID NO: 132 - DNA, 23 bp, Artificial Sequence
  TRAC-TCRA-ex1-F1 ddPCR primer/probe 10.A.9
ctgatcctcttgtcccacagata

SEQ ID NO: 133 - DNA, 26 bp, Artificial Sequence
  TRAC-TCRA-ex1-F1 ddPCR primer/probe 10.A.10
gacttgtcactggatttagagtctct

SEQ ID NO: 134 - DNA, 22 bp, Artificial Sequence
  TRAC-probe(HEX) ddPCR primer/probe 10.B.6
atccagaaccctgaccctgccg